European Patent Application EP 4 786 487 A1, published August 5, 2026. Title: Peptides. Applicant: PeptiDream Inc. The sequence listing filed with the application follows.

SEQUENCE LISTING (368 sequences)

SEQ ID NO: 1 - protein, 15 aa, synthetic construct
  MUTAGEN 5: note = X stands for (2S)-2-(methylamino)-3-phenyl-propanoic acid
  MUTAGEN 7: note = X stands for 2-(methylamino)-acetic acid
  MUTAGEN 11: note = X stands for (2S)-2-(methylamino)-3-phenyl-propanoic acid
  MUTAGEN 13: note = X stands for (2S)-2-(methylamino)-propanoic acid
  MUTAGEN 14: note = X stands for (2S)-2-(methylamino)-3-phenyl-propanoic acid
ARWYXIXYYRXLXXC

SEQ ID NO: 2 - skipped

SEQ ID NO: 3 - protein, 15 aa, synthetic construct
  MUTAGEN 1: note = X stands for 4-((carboxymethyl)amino)-butanoic acid
  MUTAGEN 5: note = X stands for (2S)-2-(methylamino)-3-phenyl-propanoic acid
  MUTAGEN 7: note = X stands for 2-(methylamino)-acetic acid
  MUTAGEN 9: note = X stands for (S)-4-(2-amino-2-carboxyethyl)-benzoic acid
  MUTAGEN 11: note = X stands for (2S)-2-(methylamino)-3-phenyl-propanoic acid
  MUTAGEN 13: note = X stands for (2S)-2-(methylamino)-propanoic acid
  MUTAGEN 14: note = X stands for (2S)-2-(methylamino)-3-phenyl-propanoic acid
  MUTAGEN 15: note = X stands for D-cysteine
XAWYXIXYXRXLXXX

SEQ ID NO: 4 - protein, 19 aa, synthetic construct
  MUTAGEN 1: note = X stands for 4-((carboxymethyl)amino)-butanoic acid
  MUTAGEN 3: note = X stands for (S)-2-amino-3-(1H-pyrrolo[2,3-b]pyridin-3-yl)-propanoic acid
  MUTAGEN 5: note = X stands for (2S)-2-(methylamino)-3-phenyl-propanoic acid
  MUTAGEN 7: note = X stands for 2-(methylamino)-acetic acid
  MUTAGEN 8: note = X stands for (S)-2-amino-3-(pyridin-4-yl)-propanoic acid
  MUTAGEN 9: note = X stands for (S)-4-(2-amino-2-carboxyethyl)-benzoic acid
  MUTAGEN 11: note = X stands for (2S)-2-(methylamino)-3-phenyl-propanoic acid
  MUTAGEN 13: note = X stands for (2S)-2-(methylamino)-propanoic acid
  MUTAGEN 14: note = X stands for (2S)-2-(methylamino)-3-phenyl-propanoic acid
  MUTAGEN 15: note = X stands for D-cysteine
  MUTAGEN 17: note = X stands for D-glutamic acid
  MUTAGEN 19: note = X stands for D-lysine
XAXYXIXXXRXLXXXGXGX

SEQ ID NO: 5 - protein, 15 aa, synthetic construct
  MUTAGEN 1: note = X stands for 4-((carboxymethyl)amino)-butanoic acid
  MUTAGEN 3: note = X stands for (S)-2-amino-3-(1H-pyrrolo[2,3-b]pyridin-3-yl)-propanoic acid
  MUTAGEN 5: note = X stands for (2S)-2-(methylamino)-3-phenyl-propanoic acid
  MUTAGEN 7: note = X stands for 2-(methylamino)-acetic acid
  MUTAGEN 9: note = X stands for (S)-2-amino-3-(pyridin-3-yl)-propanoic acid
  MUTAGEN 11: note = X stands for (2S)-2-(methylamino)-3-phenyl-propanoic acid
  MUTAGEN 13: note = X stands for (2S)-2-(methylamino)-propanoic acid
  MUTAGEN 14: note = X stands for (2S)-2-(methylamino)-3-phenyl-propanoic acid
  MUTAGEN 15: note = X stands for D-cysteine
XAXYXIXFXRXLXXX

SEQ ID NO: 6 - protein, 15 aa, synthetic construct
  MUTAGEN 1: note = X stands for 4-((carboxymethyl)amino)-butanoic acid
  MUTAGEN 3: note = X stands for (S)-2-amino-3-(1H-pyrrolo[2,3-b]pyridin-3-yl)-propanoic acid
  MUTAGEN 5: note = X stands for (2S)-2-(methylamino)-3-phenyl-propanoic acid
  MUTAGEN 7: note = X stands for 2-(methylamino)-acetic acid
  MUTAGEN 9: note = X stands for (S)-2-amino-3-(4-(carboxymethoxy)phenyl)-propanoic acid
  MUTAGEN 11: note = X stands for (2S)-2-(methylamino)-3-phenyl-propanoic acid
  MUTAGEN 13: note = X stands for (2S)-2-(methylamino)-propanoic acid
  MUTAGEN 14: note = X stands for (2S)-2-(methylamino)-3-phenyl-propanoic acid
  MUTAGEN 15: note = X stands for D-cysteine
XAXYXIXFXRXLXXX

SEQ ID NO: 7 - protein, 15 aa, synthetic construct
  MUTAGEN 1: note = X stands for 4-((carboxymethyl)amino)-butanoic acid
  MUTAGEN 3: note = X stands for (S)-2-amino-3-(1H-pyrrolo[2,3-b]pyridin-3-yl)-propanoic acid
  MUTAGEN 5: note = X stands for (2S)-2-(methylamino)-3-phenyl-propanoic acid
  MUTAGEN 7: note = X stands for 2-(methylamino)-acetic acid
  MUTAGEN 9: note = X stands for (S)-2-amino-3-(4-carbamoylphenyl)-propanoic acid
  MUTAGEN 11: note = X stands for (2S)-2-(methylamino)-3-phenyl-propanoic acid
  MUTAGEN 13: note = X stands for (2S)-2-(methylamino)-propanoic acid
  MUTAGEN 14: note = X stands for (2S)-2-(methylamino)-3-phenyl-propanoic acid
  MUTAGEN 15: note = X stands for D-cysteine
XAXYXIXFXRXLXXX

SEQ ID NO: 8 - protein, 15 aa, synthetic construct
  MUTAGEN 1: note = X stands for 4-((carboxymethyl)amino)-butanoic acid
  MUTAGEN 3: note = X stands for (S)-2-amino-3-(1H-pyrrolo[2,3-b]pyridin-3-yl)-propanoic acid
  MUTAGEN 5: note = X stands for (2S)-2-(methylamino)-3-phenyl-propanoic acid
  MUTAGEN 7: note = X stands for 2-(methylamino)-acetic acid
  MUTAGEN 9: note = X stands for (S)-2-amino-3-(3-carbamoylphenyl)-propanoic acid
  MUTAGEN 11: note = X stands for (2S)-2-(methylamino)-3-phenyl-propanoic acid
  MUTAGEN 13: note = X stands for (2S)-2-(methylamino)-propanoic acid
  MUTAGEN 14: note = X stands for (2S)-2-(methylamino)-3-phenyl-propanoic acid
  MUTAGEN 14: note = X stands for D-cysteine
XAXYXIXFXRXLXXX

SEQ ID NO: 9 - protein, 15 aa, synthetic construct
  MUTAGEN 1: note = X stands for 2-[(2-carbamoylethyl)amino]-acetic acid
  MUTAGEN 3: note = X stands for (S)-2-amino-3-(1H-pyrrolo[2,3-b]pyridin-3-yl)-propanoic acid
  MUTAGEN 5: note = X stands for (2S)-2-(methylamino)-3-phenyl-propanoic acid
  MUTAGEN 7: note = X stands for 2-(methylamino)-acetic acid
  MUTAGEN 9: note = X stands for (S)-4-(2-amino-2-carboxyethyl)-benzoic acid
  MUTAGEN 11: note = X stands for (2S)-2-(methylamino)-3-phenyl-propanoic acid
  MUTAGEN 13: note = X stands for (2S)-2-(methylamino)-propanoic acid
  MUTAGEN 14: note = X stands for (2S)-2-(methylamino)-3-phenyl-propanoic acid
  MUTAGEN 15: note = X stands for D-cysteine
XAXYXIXFXRXLXXX

SEQ ID NO: 10 - protein, 15 aa, synthetic construct
  MUTAGEN 1: note = X stands for 4-((carboxymethyl)amino)-butanoic acid
  MUTAGEN 3: note = X stands for (S)-2-amino-3-(1H-pyrrolo[2,3-b]pyridin-3-yl)-propanoic acid
  MUTAGEN 5: note = X stands for (2S)-2-(methylamino)-3-phenyl-propanoic acid
  MUTAGEN 7: note = X stands for 2-(methylamino)-acetic acid
  MUTAGEN 9: note = X stands for (S)-4-(2-amino-2-carboxyethyl)-benzoic acid
  MUTAGEN 11: note = X stands for (2S)-2-(methylamino)-3-phenyl-propanoic acid
  MUTAGEN 13: note = X stands for (2S)-2-(methylamino)-propanoic acid
  MUTAGEN 14: note = X stands for (2S)-2-(methylamino)-3-phenyl-propanoic acid
  MUTAGEN 15: note = X stands for D-cysteine
XAXYXIXFXRXLXXX

SEQ ID NO: 11 - protein, 15 aa, synthetic construct
  MUTAGEN 1: note = X stands for 4-((carboxymethyl)amino)-butanoic acid
  MUTAGEN 3: note = X stands for (S)-2-amino-3-(1H-pyrrolo[2,3-b]pyridin-3-yl)-propanoic acid
  MUTAGEN 5: note = X stands for (2S)-2-(methylamino)-3-phenyl-propanoic acid
  MUTAGEN 7: note = X stands for 2-(methylamino)-acetic acid
  MUTAGEN 8: note = X stands for (S)-2-amino-3-(pyridin-4-yl)-propanoic acid
  MUTAGEN 9: note = X stands for (S)-4-(2-amino-2-carboxyethyl)-benzoic acid
  MUTAGEN 11: note = X stands for (2S)-2-(methylamino)-3-phenyl-propanoic acid
  MUTAGEN 13: note = X stands for (2S)-2-(methylamino)-propanoic acid
  MUTAGEN 14: note = X stands for (2S)-2-(methylamino)-3-phenyl-propanoic acid
  MUTAGEN 15: note = X stands for D-cysteine
XAXYXIXXXRXLXXX

SEQ ID NO: 12 - protein, 15 aa, synthetic construct
  MUTAGEN 1: note = X stands for 4-((carboxymethyl)amino)-butanoic acid
  MUTAGEN 3: note = X stands for (2S)-2-amino-3-[4-(pyridin-4-yl)phenyl]-propanoic acid
  MUTAGEN 5: note = X stands for (2S)-2-(methylamino)-3-phenyl-propanoic acid
  MUTAGEN 7: note = X stands for (2S)-2-(methylamino)-propanoic acid
  MUTAGEN 8: note = X stands for (S)-2-amino-3-(3-(carboxymethoxy)phenyl)-propanoic acid
  MUTAGEN 9: note = X stands for (S)-2-amino-3-(4-(carboxymethoxy)phenyl)-propanoic acid
  MUTAGEN 11: note = X stands for (2S)-2-(methylamino)-3-phenyl-propanoic acid
  MUTAGEN 13: note = X stands for (2S)-2-(methylamino)-propanoic acid
  MUTAGEN 14: note = X stands for (2S)-2-(methylamino)-3-phenyl-propanoic acid
  MUTAGEN 15: note = X stands for D-cysteine
XAXYXIXXXRXLXXX

SEQ ID NO: 13 - protein, 15 aa, synthetic construct
  MUTAGEN 1: note = X stands for 4-((carboxymethyl)amino)-butanoic acid
  MUTAGEN 3: note = X stands for (2S)-2-amino-3-[4-(pyridin-4-yl)phenyl]-propanoic acid
  MUTAGEN 5: note = X stands for (2S)-2-(methylamino)-3-phenyl-propanoic acid
  MUTAGEN 7: note = X stands for 2-(methylamino)-acetic acid
  MUTAGEN 8: note = X stands for (S)-2-amino-3-(3-(carboxymethoxy)phenyl)-propanoic acid
  MUTAGEN 9: note = X stands for (S)-2-amino-3-(4-(carboxymethoxy)phenyl)-propanoic acid
  MUTAGEN 11: note = X stands for (2S)-2-(methylamino)-3-phenyl-propanoic acid
  MUTAGEN 13: note = X stands for (2S)-2-(methylamino)-propanoic acid
  MUTAGEN 14: note = X stands for (2S)-2-(methylamino)-3-phenyl-propanoic acid
  MUTAGEN 15: note = X stands for D-cysteine
XAXYXIXXXRXLXXX

SEQ ID NO: 14 - protein, 15 aa, synthetic construct
  MUTAGEN 1: note = X stands for 4-((carboxymethyl)amino)-butanoic acid
  MUTAGEN 3: note = X stands for (S)-3-([1,1'-biphenyl]-4-yl)-2-amino-propanoic acid
  MUTAGEN 5: note = X stands for (2S)-2-(methylamino)-3-phenyl-propanoic acid
  MUTAGEN 7: note = X stands for (2S)-2-(methylamino)-propanoic acid
  MUTAGEN 8: note = X stands for (S)-2-amino-3-(3-(carboxymethoxy)phenyl)-propanoic acid
  MUTAGEN 9: note = X stands for (S)-2-amino-3-(4-(carboxymethoxy)phenyl)-propanoic acid
  MUTAGEN 11: note = X stands for (2S)-2-(methylamino)-3-phenyl-propanoic acid
  MUTAGEN 13: note = X stands for (2S)-2-(methylamino)-propanoic acid
  MUTAGEN 14: note = X stands for (2S)-2-(methylamino)-3-phenyl-propanoic acid
  MUTAGEN 15: note = X stands for D-cysteine
XAXYXIXXXRXLXXX

SEQ ID NO: 15 - protein, 15 aa, synthetic construct
  MUTAGEN 1: note = note = X stands for 4-((carboxymethyl)amino)-butanoic acid
  MUTAGEN 3: note = X stands for (S)-3-([1,1'-biphenyl]-4-yl)-2-amino-propanoic acid
  MUTAGEN 5: note = X stands for (2S)-2-(methylamino)-3-phenyl-propanoic acid
  MUTAGEN 7: note = X stands for 2-(methylamino)-acetic acid
  MUTAGEN 8: note = X stands for (S)-2-amino-3-(3-(carboxymethoxy)phenyl)-propanoic acid
  MUTAGEN 9: note = X stands for (S)-2-amino-3-(4-(carboxymethoxy)phenyl)-propanoic acid
  MUTAGEN 11: note = X stands for (2S)-2-(methylamino)-3-phenyl-propanoic acid
  MUTAGEN 13: note = X stands for (2S)-2-(methylamino)-propanoic acid
  MUTAGEN 14: note = X stands for (2S)-2-(methylamino)-3-phenyl-propanoic acid
  MUTAGEN 15: note = X stands for D-cysteine
XAXYXIXXXRXLXXX

SEQ ID NO: 16 - protein, 15 aa, synthetic construct
  MUTAGEN 1: note = X stands for 4-((carboxymethyl)amino)-butanoic acid
  MUTAGEN 3: note = X stands for (2S)-2-amino-3-[4-(pyridin-4-yl)phenyl]-propanoic acid
  MUTAGEN 5: note = X stands for (2S)-2-(methylamino)-3-phenyl-propanoic acid
  MUTAGEN 7: note = X stands for (2S)-2-(methylamino)-propanoic acid
  MUTAGEN 8: note = X stands for (S)-2-amino-3-(3-(carboxymethoxy)phenyl)-propanoic acid
  MUTAGEN 9: note = X stands for (S)-2-amino-3-(4-(carboxymethoxy)phenyl)-propanoic acid
  MUTAGEN 11: note = X stands for (2S)-2-(methylamino)-3-phenyl-propanoic acid
  MUTAGEN 13: note = X stands for (2S)-2-(methylamino)-propanoic acid
  MUTAGEN 14: note = X stands for (2S)-2-(methylamino)-3-phenyl-propanoic acid
  MUTAGEN 15: note = X stands for D-cysteine
XGXYXIXXXRXLXXX

SEQ ID NO: 17 - protein, 15 aa, synthetic construct
  MUTAGEN 1: note = X stands for 4-((carboxymethyl)amino)-butanoic acid
  MUTAGEN 3: note = X stands for (2S)-2-amino-3-[4-(pyridin-4-yl)phenyl]-propanoic acid
  MUTAGEN 5: note = X stands for (2S)-2-(methylamino)-3-phenyl-propanoic acid
  MUTAGEN 7: note = X stands for 2-(methylamino)-acetic acid
  MUTAGEN 8: note = X stands for (S)-2-amino-3-(3-(carboxymethoxy)phenyl)-propanoic acid
  MUTAGEN 9: note = X stands for (S)-2-amino-3-(4-(carboxymethoxy)phenyl)-propanoic acid
  MUTAGEN 11: note = X stands for (2S)-2-(methylamino)-3-phenyl-propanoic acid
  MUTAGEN 13: note = X stands for (2S)-2-(methylamino)-propanoic acid
  MUTAGEN 14: note = X stands for (2S)-2-(methylamino)-3-phenyl-propanoic acid
  MUTAGEN 15: note = X stands for D-cysteine
XGXYXIXXXRXLXXX

SEQ ID NO: 18 - protein, 15 aa, synthetic construct
  MUTAGEN 1: note = X standards for (2S)-2-(methylamino)-butanedioic acid
  MUTAGEN 3: note = X stands for (2S)-2-amino-3-[4-(pyridin-4-yl)phenyl]-propanoic acid
  MUTAGEN 5: note = X stands for (2S)-2-(methylamino)-3-phenyl-propanoic acid
  MUTAGEN 7: note = X stands for 2-(methylamino)-acetic acid
  MUTAGEN 8: note = X stands for (S)-2-amino-3-(3-(carboxymethoxy)phenyl)-propanoic acid
  MUTAGEN 9: note = X stands for (S)-2-amino-3-(4-(carboxymethoxy)phenyl)-propanoic acid
  MUTAGEN 11: note = X stands for (2S)-2-(methylamino)-3-phenyl-propanoic acid
  MUTAGEN 13: note = X stands for (2S)-2-(methylamino)-propanoic acid
  MUTAGEN 14: note = X stands for (2S)-2-(methylamino)-3-phenyl-propanoic acid
  MUTAGEN 15: note = X stands for D-cysteine
XAXYXIXXXRXLXXX

SEQ ID NO: 19 - protein, 15 aa, synthetic construct
  MUTAGEN 3: note = X stands for (2S)-2-amino-3-[4-(pyridin-4-yl)phenyl]-propanoic acid
  MUTAGEN 5: note = X stands for (2S)-2-(methylamino)-3-phenyl-propanoic acid
  MUTAGEN 7: note = X stands for 2-(methylamino)-acetic acid
  MUTAGEN 8: note = X stands for (S)-2-amino-3-(3-(carboxymethoxy)phenyl)-propanoic acid
  MUTAGEN 9: note = X stands for (S)-2-amino-3-(4-(carboxymethoxy)phenyl)-propanoic acid
  MUTAGEN 11: note = X stands for (2S)-2-(methylamino)-3-phenyl-propanoic acid
  MUTAGEN 13: note = X stands for (2S)-2-(methylamino)-propanoic acid
  MUTAGEN 14: note = X stands for (2S)-2-(methylamino)-3-phenyl-propanoic acid
  MUTAGEN 15: note = X stands for D-cysteine
AAXYXIXXXRXLXXX

SEQ ID NO: 20 - protein, 15 aa, synthetic construct
  MUTAGEN 3: note = X stands for (S)-3-([1,1'-biphenyl]-4-yl)-2-amino-propanoic acid
  MUTAGEN 5: note = X stands for (2S)-2-(methylamino)-3-phenyl-propanoic acid
  MUTAGEN 7: note = X stands for 2-(methylamino)-acetic acid
  MUTAGEN 8: note = X stands for (S)-2-amino-3-(3-(carboxymethoxy)phenyl)-propanoic acid
  MUTAGEN 9: note = X stands for (S)-2-amino-3-(4-(carboxymethoxy)phenyl)-propanoic acid
  MUTAGEN 11: note = X stands for (2S)-2-(methylamino)-3-phenyl-propanoic acid
  MUTAGEN 13: note = X stands for (2S)-2-(methylamino)-propanoic acid MUTAGEN
  MUTAGEN 14: note = X stands for (2S)-2-(methylamino)-3-phenyl-propanoic acid
  MUTAGEN 15: note = X stands for D-cysteine
AAXYXIXXXRXLXXX

SEQ ID NO: 21 - protein, 15 aa, synthetic construct
  MUTAGEN 3: note = X stands for (S)-3-([1,1'-biphenyl]-4-yl)-2-amino-propanoic acid
  MUTAGEN 5: note = X stands for (2S)-2-(methylamino)-3-phenyl-propanoic acid
  MUTAGEN 7: note = X stands for (2S)-2-(methylamino)-propanoic acid
  MUTAGEN 8: note = X stands for (S)-2-amino-3-(3-(carboxymethoxy)phenyl)-propanoic acid
  MUTAGEN 9: note = X stands for (S)-2-amino-3-(4-(carboxymethoxy)phenyl)-propanoic acid
  MUTAGEN 11: note = X stands for (2S)-2-(methylamino)-3-phenyl-propanoic acid
  MUTAGEN 13: note = X stands for (2S)-2-(methylamino)-propanoic acid
  MUTAGEN 14: note = X stands for (2S)-2-(methylamino)-3-phenyl-propanoic acid
  MUTAGEN 15: note = X stands for D-cysteine
AAXYXIXXXRXLXXX

SEQ ID NO: 22 - protein, 15 aa, synthetic construct
  MUTAGEN 1: note = X stands for 4-((carboxymethyl)amino)-butanoic acid
  MUTAGEN 3: note = X stands for (2S)-2-amino-3-[4-(pyridin-4-yl)phenyl]-propanoic acid
  MUTAGEN 5: note = X stands for (2S)-2-(methylamino)-3-phenyl-propanoic acid
  MUTAGEN 7: note = X stands for 2-(methylamino)-acetic acid
  MUTAGEN 8: note = X stands for (S)-2-amino-3-(3-(carboxymethoxy)phenyl)-propanoic acid
  MUTAGEN 9: note = X stands for (S)-2-amino-3-(4-(carboxymethoxy)phenyl)-propanoic acid
  MUTAGEN 11: note = X stands for (2S)-2-(methylamino)-3-phenyl-propanoic acid
  MUTAGEN 13: note = X stands for (2S)-2-(methylamino)-propanoic acid
  MUTAGEN 14: note = X stands for (2S)-2-(methylamino)-3-phenyl-propanoic acid
  MUTAGEN 15: note = X stands for D-cysteine
XSXYXIXXXRXLXXX

SEQ ID NO: 23 - protein, 15 aa, synthetic construct
  MUTAGEN 1: note = X stands for 4-((carboxymethyl)amino)-butanoic acid
  MUTAGEN 3: note = X stands for (S)-3-([1,1'-biphenyl]-4-yl)-2-amino-propanoic acid
  MUTAGEN 5: note = X stands for (2S)-3-(4-hydroxyphenyl)-2-(methylamino)-propanoic acid
  MUTAGEN 7: note = X stands for 2-(methylamino)-acetic acid
  MUTAGEN 8: note = X stands for (S)-2-amino-3-(3-(carboxymethoxy)phenyl)-propanoic acid
  MUTAGEN 9: note = X stands for (S)-4-(2-amino-2-carboxyethyl)-benzoic acid
  MUTAGEN 11: note = X stands for (2S)-2-(methylamino)-3-phenyl-propanoic acid
  MUTAGEN 12: note = X stands for (S)-2-amino-heptanoic acid
  MUTAGEN 13: note = X stands for (2S)-2-(methylamino)-propanoic acid
  MUTAGEN 14: note = X stands for (2S)-2-(methylamino)-3-phenyl-propanoic acid
  MUTAGEN 15: note = X stands for D-cysteine
XAXYXIXXXRXXXXX

SEQ ID NO: 24 - protein, 15 aa, synthetic construct
  MUTAGEN 1: note = X stands for 4-((carboxymethyl)amino)-butanoic acid
  MUTAGEN 3: note = X stands for (S)-3-([1,1'-biphenyl]-4-yl)-2-amino-propanoic acid
  MUTAGEN 5: note = X stands for (2S)-3-(4-hydroxyphenyl)-2-(methylamino)-propanoic acid
  MUTAGEN 7: note = X stands for 2-(methylamino)-acetic acid
  MUTAGEN 8: note = X stands for (S)-2-amino-3-(3-(carboxymethoxy)phenyl)-propanoic acid
  MUTAGEN 9: note = X stands for (S)-4-(2-amino-2-carboxyethyl)-benzoic acid
  MUTAGEN 11: note = X stands for (2S)-2-(methylamino)-3-phenyl-propanoic acid
  MUTAGEN 12: note = X stands for (S)-2-amino-nonanoic acid
  MUTAGEN 13: note = X stands for (2S)-2-(methylamino)-propanoic acid
  MUTAGEN 14: note = X stands for (2S)-2-(methylamino)-3-phenyl-propanoic acid
  MUTAGEN 15: note = X stands for D-cysteine
XAXYXIXXXRXXXXX

SEQ ID NO: 25 - protein, 15 aa, synthetic construct
  MUTAGEN 1: note = X stands for 4-((carboxymethyl)amino)-butanoic acid
  MUTAGEN 3: note = X stands for (S)-3-([1,1'-biphenyl]-4-yl)-2-amino-propanoic acid
  MUTAGEN 5: note = X stands for (2S)-3-(4-hydroxyphenyl)-2-(methylamino)-propanoic acid
  MUTAGEN 7: note = X stands for (2R)-2-(methylamino)-propanoic acid
  MUTAGEN 8: note = X stands for (S)-2-amino-3-(3-(carboxymethoxy)phenyl)-propanoic acid
  MUTAGEN 9: note = X stands for (S)-4-(2-amino-2-carboxyethyl)-benzoic acid
  MUTAGEN 11: note = X stands for (2S)-2-(methylamino)-3-phenyl-propanoic acid
  MUTAGEN 13: note = X stands for (2S)-2-(methylamino)-propanoic acid
  MUTAGEN 14: note = X stands for (2S)-2-(methylamino)-3-phenyl-propanoic acid
  MUTAGEN 15: note = X stands for D-cysteine
XAXYXIXXXRXLXXX

SEQ ID NO: 26 - protein, 15 aa, synthetic construct
  MUTAGEN 1: note = X stands for 4-((carboxymethyl)amino)-butanoic acid
  MUTAGEN 3: note = X stands for (2S)-2-amino-3-[4-(pyridin-4-yl)phenyl]-propanoic acid
  MUTAGEN 5: note = X stands for (2S)-2-(methylamino)-3-phenyl-propanoic acid
  MUTAGEN 7: note = X stands for (2S)-2-(methylamino)-propanoic acid
  MUTAGEN 8: note = X stands for (S)-2-amino-3-(3-(carboxymethoxy)phenyl)-propanoic acid
  MUTAGEN 9: note = X stands for (S)-2-amino-3-(4-(carboxymethoxy)phenyl)-propanoic acid
  MUTAGEN 11: note = X stands for (2S)-2-(methylamino)-3-phenyl-propanoic acid
  MUTAGEN 13: note = X stands for (2S)-2-(methylamino)-propanoic acid
  MUTAGEN 14: note = X stands for (2S)-2-(methylamino)-3-phenyl-propanoic acid
  MUTAGEN 15: note = X stands for D-cysteine
XAXYXIXXXRXLXXX

SEQ ID NO: 27 - protein, 15 aa, synthetic construct
  MUTAGEN 1: note = X stands for 4-((carboxymethyl)amino)-butanoic acid
  MUTAGEN 5: note = X stands for (2S)-2-(methylamino)-3-phenyl-propanoic acid
  MUTAGEN 7: note = X stands for (2S)-2-(methylamino)-propanoic acid
  MUTAGEN 8: note = X stands for (S)-2-amino-3-(3-(carboxymethoxy)phenyl)-propanoic acid
  MUTAGEN 9: note = X stands for (S)-2-amino-3-(4-(carboxymethoxy)phenyl)-propanoic acid
  MUTAGEN 11: note = X stands for (2S)-2-(methylamino)-3-phenyl-propanoic acid
  MUTAGEN 13: note = X stands for (2S)-2-(methylamino)-propanoic acid
  MUTAGEN 14: note = X stands for (2S)-2-(methylamino)-3-phenyl-propanoic acid
  MUTAGEN 15: note = X stands for D-cysteine
XAWYXIXXXRXLXXX

SEQ ID NO: 28 - protein, 15 aa, synthetic construct
  MUTAGEN 1: note = X stands for 4-((carboxymethyl)amino)-butanoic acid
  MUTAGEN 3: note = X stands for (2S)-2-amino-3-[4-(pyridin-4-yl)phenyl]-propanoic acid
  MUTAGEN 5: note = X stands for (2S)-2-(methylamino)-3-phenyl-propanoic acid
  MUTAGEN 6: note = X stands for (S)-2-amino-2-cyclopentyl-acetic acid
  MUTAGEN 7: note = X stands for (2S)-2-(methylamino)-propanoic acid
  MUTAGEN 8: note = X stands for (S)-2-amino-3-(3-(carboxymethoxy)phenyl)-propanoic acid
  MUTAGEN 9: note = X stands for (S)-2-amino-3-(4-(carboxymethoxy)phenyl)-propanoic acid
  MUTAGEN 11: note = X stands for (2S)-2-(methylamino)-3-phenyl-propanoic acid
  MUTAGEN 13: note = X stands for (2S)-2-(methylamino)-propanoic acid
  MUTAGEN 14: note = X stands for (2S)-2-(methylamino)-3-phenyl-propanoic acid
  MUTAGEN 15: note = X stands for D-cysteine
XAXYXXXXXRXLXXX

SEQ ID NO: 29 - protein, 15 aa, synthetic construct
  MUTAGEN 1: note = X stands for 4-((carboxymethyl)amino)-butanoic acid
  MUTAGEN 5: note = X stands for (2S)-2-(methylamino)-3-phenyl-propanoic acid
  MUTAGEN 7: note = X stands for (2S)-2-(methylamino)-propanoic acid
  MUTAGEN 8: note = X stands for (S)-2-amino-3-(3-(carboxymethoxy)phenyl)-propanoic acid
  MUTAGEN 9: note = X stands for (S)-4-(2-amino-2-carboxyethyl)-benzoic acid
  MUTAGEN 11: note = X stands for (2S)-2-(methylamino)-3-phenyl-propanoic acid
  MUTAGEN 13: note = X stands for (2S)-2-(methylamino)-propanoic acid
  MUTAGEN 14: note = X stands for (2S)-2-(methylamino)-3-phenyl-propanoic acid
  MUTAGEN 15: note = X stands for D-cysteine
XAWYXIXXXRXLXXX

SEQ ID NO: 30 - protein, 15 aa, synthetic construct
  MUTAGEN 1: note = X stands for 4-((carboxymethyl)amino)-butanoic acid
  MUTAGEN 5: note = X stands for (2S)-2-(methylamino)-3-phenyl-propanoic acid
  MUTAGEN 7: note = X stands for (2S)-2-(methylamino)-propanoic acid
  MUTAGEN 8: note = X stands for (S)-2-amino-3-(3-(carboxymethoxy)phenyl)-propanoic acid
  MUTAGEN 9: note = X stands for (S)-4-(2-amino-2-carboxyethyl)-benzoic acid
  MUTAGEN 11: note = X stands for (2S)-2-(methylamino)-3-phenyl-propanoic acid
  MUTAGEN 12: note = X stands for (S)-2-amino-nonanoic acid
  MUTAGEN 13: note = X stands for (2S)-2-(methylamino)-propanoic acid
  MUTAGEN 14: note = X stands for (2S)-2-(methylamino)-3-phenyl-propanoic acid
  MUTAGEN 15: note = X stands for D-cysteine
XAWYXIXXXRXXXXX

SEQ ID NO: 31 - protein, 15 aa, synthetic construct
  MUTAGEN 1: note = X stands for 4-((carboxymethyl)amino)-butanoic acid
  MUTAGEN 3: note = X stands for (S)-2-amino-3-(1H-pyrrolo[2,3-b]pyridin-3-yl)-propanoic acid
  MUTAGEN 5: note = X stands for (2S)-2-(methylamino)-3-phenyl-propanoic acid
  MUTAGEN 7: note = X stands for (2S)-2-(methylamino)-propanoic acid
  MUTAGEN 8: note = X stands for (S)-2-amino-3-(3-(carboxymethoxy)phenyl)-propanoic acid
  MUTAGEN 9: note = X stands for (S)-4-(2-amino-2-carboxyethyl)-benzoic acid
  MUTAGEN 11: note = X stands for (2S)-2-(methylamino)-3-phenyl-propanoic acid
  MUTAGEN 12: note = X stands for (S)-2-amino-nonanoic acid
  MUTAGEN 13: note = X stands for (2S)-2-(methylamino)-propanoic acid
  MUTAGEN 14: note = X stands for (2S)-2-(methylamino)-3-phenyl-propanoic acid
  MUTAGEN 15: note = X stands for D-cysteine
XAXYXIXXXRXXXXX

SEQ ID NO: 32 - protein, 15 aa, synthetic construct
  MUTAGEN 1: note = X stands for 4-((carboxymethyl)amino)-butanoic acid
  MUTAGEN 5: note = X stands for (2S)-2-(methylamino)-3-phenyl-propanoic acid
  MUTAGEN 7: note = X stands for (2S)-2-(methylamino)-propanoic acid
  MUTAGEN 8: note = X stands for (S)-2-amino-3-(3-(carboxymethoxy)phenyl)-propanoic acid
  MUTAGEN 9: note = X stands for (S)-2-amino-3-(4-(carboxymethoxy)phenyl)-propanoic acid
  MUTAGEN 11: note = X stands for (2S)-2-(methylamino)-3-phenyl-propanoic acid
  MUTAGEN 12: note = X stands for (S)-2-amino-nonanoic acid
  MUTAGEN 13: note = X stands for (2S)-2-(methylamino)-propanoic acid
  MUTAGEN 14: note = X stands for (2S)-2-(methylamino)-3-phenyl-propanoic acid
  MUTAGEN 15: note = X stands for D-cysteine
XAWYXIXXXRXXXXX

SEQ ID NO: 33 - protein, 15 aa, synthetic construct
  MUTAGEN 1: note = X stands for 4-((carboxymethyl)amino)-butanoic acid
  MUTAGEN 3: note = X stands for (S)-2-amino-3-(1H-pyrrolo[2,3-b]pyridin-3-yl)-propanoic acid
  MUTAGEN 5: note = X stands for (2S)-2-(methylamino)-3-phenyl-propanoic acid
  MUTAGEN 7: note = X stands for (2S)-2-(methylamino)-propanoic acid
  MUTAGEN 8: note = X stands for (S)-2-amino-3-(3-(carboxymethoxy)phenyl)-propanoic acid
  MUTAGEN 9: note = X stands for (S)-2-amino-3-(4-(carboxymethoxy)phenyl)-propanoic acid
  MUTAGEN 11: note = X stands for (2S)-2-(methylamino)-3-phenyl-propanoic acid
  MUTAGEN 12: note = X stands for (S)-2-amino-nonanoic acid
  MUTAGEN 13: note = X stands for (2S)-2-(methylamino)-propanoic acid
  MUTAGEN 14: note = X stands for (2S)-2-(methylamino)-3-phenyl-propanoic acid
  MUTAGEN 15: note = X stands for D-cysteine
XAXYXIXXXRXXXXX

SEQ ID NO: 34 - protein, 15 aa, synthetic construct
  MUTAGEN 1: note = X stands for 4-((carboxymethyl)amino)-butanoic acid
  MUTAGEN 5: note = X stands for (2S)-2-(methylamino)-3-phenyl-propanoic acid
  MUTAGEN 7: note = X stands for 2-(methylamino)-acetic acid
  MUTAGEN 8: note = X stands for (S)-2-amino-3-(3-(carboxymethoxy)phenyl)-propanoic acid
  MUTAGEN 9: note = X stands for (S)-4-(2-amino-2-carboxyethyl)-benzoic acid
  MUTAGEN 11: note = X stands for (2S)-2-(methylamino)-3-phenyl-propanoic acid
  MUTAGEN 13: note = X stands for (2S)-2-(methylamino)-3-phenyl-propanoic acid
  MUTAGEN 14: note = X stands for (2S)-2-(methylamino)-3-phenyl-propanoic acid
  MUTAGEN 15: note = X stands for D-cysteine
XAWYXIXXXRXLXXX

SEQ ID NO: 35 - protein, 15 aa, synthetic construct
  MUTAGEN 1: note = X stands for 4-((carboxymethyl)amino)-butanoic acid
  MUTAGEN 5: note = X stands for (2S)-2-(methylamino)-3-phenyl-propanoic acid
  MUTAGEN 7: note = X stands for (2S)-2-(methylamino)-propanoic acid
  MUTAGEN 8: note = X stands for (S)-2-amino-3-(3-(carboxymethoxy)phenyl)-propanoic acid
  MUTAGEN 9: note = X stands for (S)-4-(2-amino-2-carboxyethyl)-benzoic acid
  MUTAGEN 11: note = X stands for (2S)-2-(methylamino)-3-phenyl-propanoic acid
  MUTAGEN 13: note = X stands for (2S)-2-(methylamino)-propanoic acid
  MUTAGEN 14: note = X stands for (2S)-2-(methylamino)-3-phenyl-propanoic acid
  MUTAGEN 15: note = X stands for D-cysteine
XSWYXIXXXRXLXXX

SEQ ID NO: 36 - protein, 15 aa, synthetic construct
  MUTAGEN 5: note = X stands for (2S)-2-(methylamino)-3-phenyl-propanoic acid
  MUTAGEN 7: note = X stands for 2-(methylamino)-acetic acid
  MUTAGEN 8: note = X stands for (S)-2-amino-3-(3-(carboxymethoxy)phenyl)-propanoic acid
  MUTAGEN 9: note = X stands for (S)-4-(2-amino-2-carboxyethyl)-benzoic acid
  MUTAGEN 11: note = X stands for (2S)-2-(methylamino)-3-phenyl-propanoic acid
  MUTAGEN 12: note = X stands for (S)-2-amino-nonanoic acid
  MUTAGEN 13: note = X stands for (2S)-2-(methylamino)-propanoic acid
  MUTAGEN 14: note = X stands for (2S)-2-(methylamino)-3-phenyl-propanoic acid
  MUTAGEN 15: note = X stands for D-cysteine
ASWYXIXXXRXXXXX

SEQ ID NO: 37 - protein, 15 aa, synthetic construct
  MUTAGEN 3: note = X stands for (S)-2-amino-3-(1H-pyrrolo[2,3-b]pyridin-3-yl)-propanoic acid
  MUTAGEN 5: note = X stands for (2S)-2-(methylamino)-3-phenyl-propanoic acid
  MUTAGEN 7: note = X stands for 2-(methylamino)-acetic acid
  MUTAGEN 8: note = X stands for (S)-2-amino-3-(3-(carboxymethoxy)phenyl)-propanoic acid
  MUTAGEN 9: note = X stands for (S)-4-(2-amino-2-carboxyethyl)-benzoic acid
  MUTAGEN 11: note = X stands for (2S)-2-(methylamino)-3-phenyl-propanoic acid
  MUTAGEN 12: note = X stands for (S)-2-amino-nonanoic acid
  MUTAGEN 13: note = X stands for (2S)-2-(methylamino)-propanoic acid
  MUTAGEN 14: note = X stands for (2S)-2-(methylamino)-3-phenyl-propanoic acid
  MUTAGEN 15: note = X stands for D-cysteine
ASXYXIXXXRXXXXX

SEQ ID NO: 38 - protein, 15 aa, synthetic construct
  MUTAGEN 1: note = X stands for 4-((carboxymethyl)amino)-butanoic acid
  MUTAGEN 5: note = X stands for (2S)-2-(methylamino)-3-phenyl-propanoic acid
  MUTAGEN 7: note = X stands for 2-(methylamino)-acetic acid
  MUTAGEN 8: note = X stands for (S)-2-amino-3-(3-(carboxymethoxy)phenyl)-propanoic acid
  MUTAGEN 9: note = X stands for (S)-4-(2-amino-2-carboxyethyl)-benzoic acid
  MUTAGEN 11: note = X stands for (2S)-2-(methylamino)-3-phenyl-propanoic acid
  MUTAGEN 12: note = X stands for (S)-2-amino-nonanoic acid
  MUTAGEN 13: note = X stands for (2S)-2-(methylamino)-propanoic acid
  MUTAGEN 14: note = X stands for (2S)-2-(methylamino)-3-phenyl-propanoic acid
  MUTAGEN 15: note = X stands for D-cysteine
XSWYXIXXXRXXXXX

SEQ ID NO: 39 - protein, 15 aa, synthetic construct
  MUTAGEN 1: note = X stands for 4-((carboxymethyl)amino)-butanoic acid
  MUTAGEN 3: note = X stands for (S)-2-amino-3-(1H-pyrrolo[2,3-b]pyridin-3-yl)-propanoic acid
  MUTAGEN 5: note = X stands for (2S)-2-(methylamino)-3-phenyl-propanoic acid
  MUTAGEN 7: note = X stands for 2-(methylamino)-acetic acid
  MUTAGEN 8: note = X stands for (S)-2-amino-3-(3-(carboxymethoxy)phenyl)-propanoic acid
  MUTAGEN 9: note = X stands for (S)-4-(2-amino-2-carboxyethyl)-benzoic acid
  MUTAGEN 11: note = X stands for (2S)-2-(methylamino)-3-phenyl-propanoic acid
  MUTAGEN 12: note = X stands for (S)-2-amino-nonanoic acid
  MUTAGEN 13: note = X stands for (2S)-2-(methylamino)-propanoic acid
  MUTAGEN 14: note = X stands for (2S)-2-(methylamino)-3-phenyl-propanoic acid
  MUTAGEN 15: note = X stands for D-cysteine
XSXYXIXXXRXXXXX

SEQ ID NO: 40 - protein, 15 aa, synthetic construct
  MUTAGEN 1: note = X stands for 4-((carboxymethyl)amino)-butanoic acid
  MUTAGEN 5: note = X stands for (2S)-2-(methylamino)-3-phenyl-propanoic acid
  MUTAGEN 7: note = X stands for (2S)-2-(methylamino)-propanoic acid
  MUTAGEN 8: note = X stands for (S)-2-amino-3-(3-(carboxymethoxy)phenyl)-propanoic acid
  MUTAGEN 9: note = X stands for (S)-4-(2-amino-2-carboxyethyl)-benzoic acid
  MUTAGEN 11: note = X stands for (2S)-2-(methylamino)-3-phenyl-propanoic acid
  MUTAGEN 12: note = X stands for (S)-2-amino-nonanoic acid
  MUTAGEN 13: note = X stands for (2S)-2-(methylamino)-propanoic acid
  MUTAGEN 14: note = X stands for (2S)-2-(methylamino)-3-phenyl-propanoic acid
  MUTAGEN 15: note = X stands for D-cysteine
XSWYXIXXXRXXXXX

SEQ ID NO: 41 - protein, 15 aa, synthetic construct
  MUTAGEN 1: note = X stands for 4-((carboxymethyl)amino)-butanoic acid
  MUTAGEN 3: note = X stands for (S)-2-amino-3-(1H-pyrrolo[2,3-b]pyridin-3-yl)-propanoic acid
  MUTAGEN 5: note = X stands for (2S)-2-(methylamino)-3-phenyl-propanoic acid
  MUTAGEN 7: note = X stands for (2S)-2-(methylamino)-propanoic acid
  MUTAGEN 8: note = X stands for (S)-2-amino-3-(3-(carboxymethoxy)phenyl)-propanoic acid
  MUTAGEN 9: note = X stands for (S)-4-(2-amino-2-carboxyethyl)-benzoic acid
  MUTAGEN 11: note = X stands for (2S)-2-(methylamino)-3-phenyl-propanoic acid
  MUTAGEN 12: note = X stands for (S)-2-amino-nonanoic acid
  MUTAGEN 13: note = X stands for (2S)-2-(methylamino)-propanoic acid
  MUTAGEN 14: note = X stands for (2S)-2-(methylamino)-3-phenyl-propanoic acid
  MUTAGEN 15: note = X stands for D-cysteine
XSXYXIXXXRXXXXX

SEQ ID NO: 42 - protein, 15 aa, synthetic construct
  MUTAGEN 1: note = X stands for 4-((carboxymethyl)amino)-butanoic acid
  MUTAGEN 5: note = X stands for (2S)-2-(methylamino)-3-phenyl-propanoic acid
  MUTAGEN 7: note = X stands for 2-(methylamino)-acetic acid
  MUTAGEN 8: note = X stands for (S)-2-amino-3-(3-(carboxymethoxy)phenyl)-propanoic acid
  MUTAGEN 9: note = X stands for (S)-4-(2-amino-2-carboxyethyl)-benzoic acid
  MUTAGEN 11: note = X stands for (2S)-2-(methylamino)-3-phenyl-propanoic acid
  MUTAGEN 12: note = X stands for (S)-2-amino-nonanoic acid
  MUTAGEN 13: note = X stands for (2S)-2-(methylamino)-propanoic acid
  MUTAGEN 14: note = X stands for (2S)-2-(methylamino)-3-phenyl-propanoic acid
  MUTAGEN 15: note = X stands for D-cysteine
XAWYXIXXXRXXXXX

SEQ ID NO: 43 - protein, 15 aa, synthetic construct
  MUTAGEN 1: note = X stands for 4-((carboxymethyl)amino)-butanoic acid
  MUTAGEN 3: note = X stands for (S)-2-amino-3-(1H-pyrrolo[2,3-b]pyridin-3-yl)-propanoic acid
  MUTAGEN 5: note = X stands for (2S)-2-(methylamino)-3-phenyl-propanoic acid
  MUTAGEN 7: note = X stands for 2-(methylamino)-acetic acid
  MUTAGEN 8: note = X stands for (S)-2-amino-3-(3-(carboxymethoxy)phenyl)-propanoic acid
  MUTAGEN 9: note = X stands for (S)-4-(2-amino-2-carboxyethyl)-benzoic acid
  MUTAGEN 11: note = X stands for (2S)-2-(methylamino)-3-phenyl-propanoic acid
  MUTAGEN 12: note = X stands for (S)-2-amino-nonanoic acid
  MUTAGEN 13: note = X stands for (2S)-2-(methylamino)-propanoic acid
  MUTAGEN 14: note = X stands for (2S)-2-(methylamino)-3-phenyl-propanoic acid
  MUTAGEN 15: note = X stands for D-cysteine
XAXYXIXXXRXXXXX

SEQ ID NO: 44 - protein, 15 aa, synthetic construct
  MUTAGEN 1: note = X stands for 4-((carboxymethyl)amino)-butanoic acid
  MUTAGEN 5: note = X stands for (2S)-2-(methylamino)-3-phenyl-propanoic acid
  MUTAGEN 7: note = X stands for 2-(methylamino)-acetic acid
  MUTAGEN 9: note = X stands for (S)-4-(2-amino-2-carboxyethyl)-benzoic acid
  MUTAGEN 11: note = X stands for (2S)-2-(methylamino)-3-phenyl-propanoic acid
  MUTAGEN 12: note = X stands for (S)-2-amino-nonanoic acid
  MUTAGEN 13: note = X stands for (2S)-2-(methylamino)-propanoic acid
  MUTAGEN 14: note = X stands for (2S)-2-(methylamino)-3-phenyl-propanoic acid
  MUTAGEN 15: note = X stands for D-cysteine
XAWYXIXYXRXXXXX

SEQ ID NO: 45 - protein, 15 aa, synthetic construct
  MUTAGEN 1: note = X stands for 4-((carboxymethyl)amino)-butanoic acid
  MUTAGEN 3: note = X stands for (S)-2-amino-3-(1H-pyrrolo[2,3-b]pyridin-3-yl)-propanoic acid
  MUTAGEN 5: note = X stands for (2S)-2-(methylamino)-3-phenyl-propanoic acid
  MUTAGEN 7: note = X stands for 2-(methylamino)-acetic acid
  MUTAGEN 9: note = X stands for (S)-4-(2-amino-2-carboxyethyl)-benzoic acid
  MUTAGEN 11: note = X stands for (2S)-2-(methylamino)-3-phenyl-propanoic acid
  MUTAGEN 12: note = X stands for (S)-2-amino-nonanoic acid
  MUTAGEN 13: note = X stands for (2S)-2-(methylamino)-propanoic acid
  MUTAGEN 14: note = X stands for (2S)-2-(methylamino)-3-phenyl-propanoic acid
  MUTAGEN 15: note = X stands for D-cysteine
XAXYXIXYXRXXXXX

SEQ ID NO: 46 - protein, 15 aa, synthetic construct
  MUTAGEN 1: note = X stands for 4-((carboxymethyl)amino)-butanoic acid
  MUTAGEN 5: note = X stands for (2S)-2-(methylamino)-3-phenyl-propanoic acid
  MUTAGEN 7: note = X stands for 2-(methylamino)-acetic acid
  MUTAGEN 8: note = X stands for (S)-2-amino-3-(pyridin-4-yl)-propanoic acid
  MUTAGEN 9: note = X stands for (S)-4-(2-amino-2-carboxyethyl)-benzoic acid
  MUTAGEN 11: note = X stands for (2S)-2-(methylamino)-3-phenyl-propanoic acid
  MUTAGEN 12: note = X stands for (S)-2-amino-nonanoic acid
  MUTAGEN 13: note = X stands for (2S)-2-(methylamino)-propanoic acid
  MUTAGEN 14: note = X stands for (2S)-2-(methylamino)-3-phenyl-propanoic acid
  MUTAGEN 15: note = X stands for D-cysteine
XAWYXIXXXRXXXXX

SEQ ID NO: 47 - protein, 15 aa, synthetic construct
  MUTAGEN 1: note = X stands for 4-((carboxymethyl)amino)-butanoic acid
  MUTAGEN 3: note = X stands for (S)-2-amino-3-(1H-pyrrolo[2,3-b]pyridin-3-yl)-propanoic acid
  MUTAGEN 5: note = X stands for (2S)-2-(methylamino)-3-phenyl-propanoic acid
  MUTAGEN 7: note = X stands for 2-(methylamino)-acetic acid
  MUTAGEN 8: note = X stands for (S)-2-amino-3-(pyridin-4-yl)-propanoic acid
  MUTAGEN 9: note = X stands for (S)-4-(2-amino-2-carboxyethyl)-benzoic acid
  MUTAGEN 11: note = X stands for (2S)-2-(methylamino)-3-phenyl-propanoic acid
  MUTAGEN 12: note = X stands for (S)-2-amino-nonanoic acid
  MUTAGEN 13: note = X stands for (2S)-2-(methylamino)-propanoic acid
  MUTAGEN 14: note = X stands for (2S)-2-(methylamino)-3-phenyl-propanoic acid
  MUTAGEN 15: note = X stands for D-cysteine
XAXYXIXXXRXXXXX

SEQ ID NO: 48 - protein, 15 aa, synthetic construct
  MUTAGEN 1: note = X stands for 4-((carboxymethyl)amino)-butanoic acid
  MUTAGEN 5: note = X stands for (2S)-2-(methylamino)-3-phenyl-propanoic acid
  MUTAGEN 7: note = X stands for 2-(methylamino)-acetic acid
  MUTAGEN 9: note = X stands for (S)-4-(2-amino-2-carboxyethyl)-benzoic acid
  MUTAGEN 11: note = X stands for (2S)-2-(methylamino)-3-phenyl-propanoic acid
  MUTAGEN 13: note = X stands for (2S)-2-(methylamino)-propanoic acid
  MUTAGEN 14: note = X stands for (2S)-2-(methylamino)-3-phenyl-propanoic acid
  MUTAGEN 15: note = X stands for D-cysteine
XSWYXIXYXRXLXXX

SEQ ID NO: 49 - protein, 15 aa, synthetic construct
  MUTAGEN 5: note = X stands for (2S)-2-(methylamino)-3-phenyl-propanoic acid
  MUTAGEN 7: note = X stands for 2-(methylamino)-acetic acid
  MUTAGEN 9: note = X stands for (S)-4-(2-amino-2-carboxyethyl)-benzoic acid
  MUTAGEN 11: note = X stands for (2S)-2-(methylamino)-3-phenyl-propanoic acid
  MUTAGEN 13: note = X stands for (2S)-2-(methylamino)-propanoic acid
  MUTAGEN 14: note = X stands for (2S)-2-(methylamino)-3-phenyl-propanoic acid
  MUTAGEN 15: note = X stands for D-cysteine
AAWYXIXYXRXLXXX

SEQ ID NO: 50 - protein, 15 aa, synthetic construct
  MUTAGEN 1: note = X stands for 4-((carboxymethyl)amino)-butanoic acid
  MUTAGEN 5: note = X stands for (2S)-2-(methylamino)-3-phenyl-propanoic acid
  MUTAGEN 7: note = X stands for 2-(methylamino)-acetic acid
  MUTAGEN 9: note = X stands for (S)-4-(2-amino-2-carboxyethyl)-benzoic acid
  MUTAGEN 11: note = X stands for (2S)-2-(methylamino)-3-phenyl-propanoic acid
  MUTAGEN 12: note = X stands for (S)-2-amino-nonanoic acid
  MUTAGEN 13: note = X stands for (2S)-2-(methylamino)-propanoic acid
  MUTAGEN 14: note = X stands for (2S)-2-(methylamino)-3-phenyl-propanoic acid
  MUTAGEN 15: note = X stands for D-cysteine
XSWYXIXYXRXXXXX

SEQ ID NO: 51 - protein, 15 aa, synthetic construct
  MUTAGEN 5: note = X stands for (2S)-2-(methylamino)-3-phenyl-propanoic acid
  MUTAGEN 7: note = X stands for 2-(methylamino)-acetic acid
  MUTAGEN 8: note = X stands for (S)-2-amino-3-(3-(carboxymethoxy)phenyl)-propanoic acid
  MUTAGEN 9: note = X stands for (S)-4-(2-amino-2-carboxyethyl)-benzoic acid
  MUTAGEN 11: note = X stands for (2S)-2-(methylamino)-3-phenyl-propanoic acid
  MUTAGEN 12: note = X stands for (S)-2-amino-nonanoic acid
  MUTAGEN 13: note = X stands for (2S)-2-(methylamino)-propanoic acid
  MUTAGEN 14: note = X stands for (2S)-2-(methylamino)-3-phenyl-propanoic acid
  MUTAGEN 15: note = X stands for D-cysteine
AAWYXIXXXRXXXXX

SEQ ID NO: 52 - protein, 15 aa, synthetic construct
  MUTAGEN 5: note = X stands for (2S)-2-(methylamino)-3-phenyl-propanoic acid
  MUTAGEN 7: note = X stands for 2-(methylamino)-acetic acid
  MUTAGEN 9: note = X stands for (S)-4-(2-amino-2-carboxyethyl)-benzoic acid
  MUTAGEN 11: note = X stands for (2S)-2-(methylamino)-3-phenyl-propanoic acid
  MUTAGEN 13: note = X stands for (2S)-2-(methylamino)-propanoic acid
  MUTAGEN 14: note = X stands for (2S)-2-(methylamino)-3-phenyl-propanoic acid
  MUTAGEN 15: note = X stands for D-cysteine
ASWYXIXYXRXLXXX

SEQ ID NO: 53 - protein, 15 aa, synthetic construct
  MUTAGEN 1: note = X stands for 4-((carboxymethyl)amino)-butanoic acid
  MUTAGEN 3: note = X stands for (S)-3-([1,1'-biphenyl]-4-yl)-2-amino-propanoic acid
  MUTAGEN 5: note = X stands for (2S)-2-(methylamino)-3-phenyl-propanoic acid
  MUTAGEN 7: note = X stands for 2-(methylamino)-acetic acid
  MUTAGEN 9: note = X stands for (S)-4-(2-amino-2-carboxyethyl)-benzoic acid
  MUTAGEN 11: note = X stands for (2S)-2-(methylamino)-3-phenyl-propanoic acid
  MUTAGEN 13: note = X stands for (2S)-2-(methylamino)-propanoic acid
  MUTAGEN 14: note = X stands for (2S)-2-(methylamino)-3-phenyl-propanoic acid
  MUTAGEN 15: note = X stands for D-cysteine
XAXYXIXYXRXLXXX

SEQ ID NO: 54 - protein, 15 aa, synthetic construct
  MUTAGEN 1: note = X stands for 4-((carboxymethyl)amino)-butanoic acid
  MUTAGEN 5: note = X stands for (2S)-2-(methylamino)-3-phenyl-propanoic acid
  MUTAGEN 7: note = X stands for (2S)-2-(methylamino)-propanoic acid
  MUTAGEN 9: note = X stands for (S)-4-(2-amino-2-carboxyethyl)-benzoic acid
  MUTAGEN 11: note = X stands for (2S)-2-(methylamino)-3-phenyl-propanoic acid
  MUTAGEN 13: note = X stands for (2S)-2-(methylamino)-propanoic acid
  MUTAGEN 14: note = X stands for (2S)-2-(methylamino)-3-phenyl-propanoic acid
  MUTAGEN 15: note = X stands for D-cysteine
XAWYXIXYXRXLXXX

SEQ ID NO: 55 - protein, 15 aa, synthetic construct
  MUTAGEN 1: note = X stands for 4-((carboxymethyl)amino)-butanoic acid
  MUTAGEN 3: note = X stands for (S)-3-([1,1'-biphenyl]-4-yl)-2-amino-propanoic acid
  MUTAGEN 5: note = X stands for (2S)-2-(methylamino)-3-phenyl-propanoic acid
  MUTAGEN 7: note = X stands for 2-(methylamino)-acetic acid
  MUTAGEN 9: note = X stands for (S)-4-(2-amino-2-carboxyethyl)-benzoic acid
  MUTAGEN 11: note = X stands for (2S)-2-(methylamino)-3-phenyl-propanoic acid
  MUTAGEN 12: note = X stands for (S)-2-amino-nonanoic acid
  MUTAGEN 13: note = X stands for (2S)-2-(methylamino)-propanoic acid
  MUTAGEN 14: note = X stands for (2S)-2-(methylamino)-3-phenyl-propanoic acid
  MUTAGEN 15: note = X stands for D-cysteine
XAXYXIXYXRXXXXX

SEQ ID NO: 56 - protein, 15 aa, synthetic construct
  MUTAGEN 1: note = X stands for 4-((carboxymethyl)amino)-butanoic acid
  MUTAGEN 5: note = X stands for (2S)-2-(methylamino)-3-phenyl-propanoic acid
  MUTAGEN 7: note = X stands for (2S)-2-(methylamino)-propanoic acid
  MUTAGEN 9: note = X stands for (S)-4-(2-amino-2-carboxyethyl)-benzoic acid
  MUTAGEN 11: note = X stands for (2S)-2-(methylamino)-3-phenyl-propanoic acid
  MUTAGEN 12: note = X stands for (S)-2-amino-nonanoic acid
  MUTAGEN 13: note = X stands for (2S)-2-(methylamino)-propanoic acid
  MUTAGEN 14: note = X stands for (2S)-2-(methylamino)-3-phenyl-propanoic acid
  MUTAGEN 15: note = X stands for D-cysteine
XAWYXIXYXRXXXXX

SEQ ID NO: 57 - protein, 15 aa, synthetic construct
  MUTAGEN 1: note = X stands for 4-((carboxymethyl)amino)-butanoic acid
  MUTAGEN 3: note = X stands for (S)-3-([1,1'-biphenyl]-4-yl)-2-amino-propanoic acid
  MUTAGEN 5: note = X stands for (2S)-2-(methylamino)-3-phenyl-propanoic acid
  MUTAGEN 7: note = X stands for (2S)-2-(methylamino)-propanoic acid
  MUTAGEN 9: note = X stands for (S)-4-(2-amino-2-carboxyethyl)-benzoic acid
  MUTAGEN 11: note = X stands for (2S)-2-(methylamino)-3-phenyl-propanoic acid
  MUTAGEN 13: note = X stands for (2S)-2-(methylamino)-propanoic acid
  MUTAGEN 14: note = X stands for (2S)-2-(methylamino)-3-phenyl-propanoic acid
  MUTAGEN 15: note = X stands for D-cysteine
XAXYXIXYXRXLXXX

SEQ ID NO: 58 - protein, 15 aa, synthetic construct
  MUTAGEN 1: note = X stands for 4-((carboxymethyl)amino)-butanoic acid
  MUTAGEN 3: note = X stands for (S)-3-([1,1'-biphenyl]-4-yl)-2-amino-propanoic acid
  MUTAGEN 5: note = X stands for (2S)-2-(methylamino)-3-phenyl-propanoic acid
  MUTAGEN 7: note = X stands for 2-(methylamino)-acetic acid
  MUTAGEN 8: note = X stands for (S)-2-amino-3-(3-(carboxymethoxy)phenyl)-propanoic acid
  MUTAGEN 9: note = X stands for (S)-4-(2-amino-2-carboxyethyl)-benzoic acid
  MUTAGEN 11: note = X stands for (2S)-2-(methylamino)-3-phenyl-propanoic acid
  MUTAGEN 13: note = X stands for (2S)-2-(methylamino)-propanoic acid
  MUTAGEN 14: note = X stands for (2S)-2-(methylamino)-3-phenyl-propanoic acid
  MUTAGEN 15: note = X stands for D-cysteine
XAXYXIXXXRXLXXX

SEQ ID NO: 59 - protein, 15 aa, synthetic construct
  MUTAGEN 1: note = X stands for 4-((carboxymethyl)amino)-butanoic acid
  MUTAGEN 3: note = X stands for (S)-3-([1,1'-biphenyl]-4-yl)-2-amino-propanoic acid
  MUTAGEN 5: note = X stands for (2S)-2-(methylamino)-3-phenyl-propanoic acid
  MUTAGEN 7: note = X stands for 2-(methylamino)-acetic acid
  MUTAGEN 9: note = X stands for (S)-4-(2-amino-2-carboxyethyl)-benzoic acid
  MUTAGEN 11: note = X stands for (2S)-2-(methylamino)-3-phenyl-propanoic acid
  MUTAGEN 13: note = X stands for (2S)-2-(methylamino)-propanoic acid
  MUTAGEN 14: note = X stands for (2S)-2-(methylamino)-3-phenyl-propanoic acid
  MUTAGEN 15: note = X stands for D-cysteine
XSXYXIXYXRXLXXX

SEQ ID NO: 60 - protein, 15 aa, synthetic construct
  MUTAGEN 1: note = X stands for 4-((carboxymethyl)amino)-butanoic acid
  MUTAGEN 5: note = X stands for (2S)-2-(methylamino)-3-phenyl-propanoic acid
  MUTAGEN 7: note = X stands for (2S)-2-(methylamino)-propanoic acid
  MUTAGEN 9: note = X stands for (S)-4-(2-amino-2-carboxyethyl)-benzoic acid
  MUTAGEN 11: note = X stands for (2S)-2-(methylamino)-3-phenyl-propanoic acid
  MUTAGEN 13: note = X stands for (2S)-2-(methylamino)-propanoic acid
  MUTAGEN 14: note = X stands for (2S)-2-(methylamino)-3-phenyl-propanoic acid
  MUTAGEN 15: note = X stands for D-cysteine
XSWYXIXYXRXLXXX

SEQ ID NO: 61 - protein, 15 aa, synthetic construct
  MUTAGEN 3: note = X stands for (S)-3-([1,1'-biphenyl]-4-yl)-2-amino-propanoic acid
  MUTAGEN 5: note = X stands for (2S)-2-(methylamino)-3-phenyl-propanoic acid
  MUTAGEN 7: note = X stands for 2-(methylamino)-acetic acid
  MUTAGEN 9: note = X stands for (S)-4-(2-amino-2-carboxyethyl)-benzoic acid
  MUTAGEN 11: note = X stands for (2S)-2-(methylamino)-3-phenyl-propanoic acid
  MUTAGEN 13: note = X stands for (2S)-2-(methylamino)-propanoic acid
  MUTAGEN 14: note = X stands for (2S)-2-(methylamino)-3-phenyl-propanoic acid
  MUTAGEN 15: note = X stands for D-cysteine
AAXYXIXYXRXLXXX

SEQ ID NO: 62 - protein, 15 aa, synthetic construct
  MUTAGEN 5: note = X stands for (2S)-2-(methylamino)-3-phenyl-propanoic acid
  MUTAGEN 7: note = X stands for (2S)-2-(methylamino)-propanoic acid
  MUTAGEN 9: note = X stands for (S)-4-(2-amino-2-carboxyethyl)-benzoic acid
  MUTAGEN 11: note = X stands for (2S)-2-(methylamino)-3-phenyl-propanoic acid
  MUTAGEN 13: note = X stands for (2S)-2-(methylamino)-propanoic acid
  MUTAGEN 14: note = X stands for (2S)-2-(methylamino)-3-phenyl-propanoic acid
  MUTAGEN 15: note = X stands for D-cysteine
AAWYXIXYXRXLXXX

SEQ ID NO: 63 - protein, 15 aa, synthetic construct
  MUTAGEN 5: note = X stands for (2S)-2-(methylamino)-3-phenyl-propanoic acid
  MUTAGEN 7: note = X stands for 2-(methylamino)-acetic acid
  MUTAGEN 8: note = X stands for (S)-2-amino-3-(3-(carboxymethoxy)phenyl)-propanoic acid
  MUTAGEN 9: note = X stands for (S)-4-(2-amino-2-carboxyethyl)-benzoic acid
  MUTAGEN 11: note = X stands for (2S)-2-(methylamino)-3-phenyl-propanoic acid
  MUTAGEN 13: note = X stands for (2S)-2-(methylamino)-propanoic acid
  MUTAGEN 14: note = X stands for (2S)-2-(methylamino)-3-phenyl-propanoic acid
  MUTAGEN 15: note = X stands for D-cysteine
AAWYXIXXXRXLXXX

SEQ ID NO: 64 - protein, 15 aa, synthetic construct
  MUTAGEN 5: note = X stands for (2S)-2-(methylamino)-3-phenyl-propanoic acid
  MUTAGEN 7: note = X stands for 2-(methylamino)-acetic acid
  MUTAGEN 9: note = X stands for (S)-4-(2-amino-2-carboxyethyl)-benzoic acid
  MUTAGEN 11: note = X stands for (2S)-2-(methylamino)-3-phenyl-propanoic acid
  MUTAGEN 12: note = X stands for (S)-2-amino-nonanoic acid
  MUTAGEN 13: note = X stands for (2S)-2-(methylamino)-propanoic acid
  MUTAGEN 14: note = X stands for (2S)-2-(methylamino)-3-phenyl-propanoic acid
  MUTAGEN 15: note = X stands for D-cysteine
AAWYXIXYXRXXXXX

SEQ ID NO: 65 - protein, 15 aa, synthetic construct
  MUTAGEN 5: note = X stands for (2S)-2-(methylamino)-3-phenyl-propanoic acid
  MUTAGEN 7: note = X stands for (2S)-2-(methylamino)-propanoic acid
  MUTAGEN 8: note = X stands for (S)-2-amino-3-(3-(carboxymethoxy)phenyl)-propanoic acid
  MUTAGEN 9: note = X stands for (S)-4-(2-amino-2-carboxyethyl)-benzoic acid
  MUTAGEN 11: note = X stands for (2S)-2-(methylamino)-3-phenyl-propanoic acid
  MUTAGEN 12: note = X stands for (S)-2-amino-nonanoic acid
  MUTAGEN 13: note = X stands for (2S)-2-(methylamino)-propanoic acid
  MUTAGEN 14: note = X stands for (2S)-2-(methylamino)-3-phenyl-propanoic acid
  MUTAGEN 15: note = X stands for D-cysteine
AAWYXIXXXRXXXXX

SEQ ID NO: 66 - protein, 15 aa, synthetic construct
  MUTAGEN 1: note = X stands for (2S)-2-(methylamino)-propanoic acid
  MUTAGEN 5: note = X stands for (2S)-2-(methylamino)-3-phenyl-propanoic acid
  MUTAGEN 7: note = X stands for (2S)-2-(methylamino)-propanoic acid
  MUTAGEN 8: note = X stands for (S)-2-amino-3-(3-(carboxymethoxy)phenyl)-propanoic acid
  MUTAGEN 9: note = X stands for (S)-4-(2-amino-2-carboxyethyl)-benzoic acid
  MUTAGEN 11: note = X stands for (2S)-2-(methylamino)-3-phenyl-propanoic acid
  MUTAGEN 12: note = X stands for (S)-2-amino-nonanoic acid
  MUTAGEN 13: note = X stands for (2S)-2-(methylamino)-propanoic acid
  MUTAGEN 14: note = X stands for (2S)-2-(methylamino)-3-phenyl-propanoic acid
  MUTAGEN 15: note = X stands for D-cysteine
XAWYXIXXXRXXXXX

SEQ ID NO: 67 - protein, 15 aa, synthetic construct
  MUTAGEN 1: note = X stands for 4-((carboxymethyl)amino)-butanoic acid
  MUTAGEN 5: note = X stands for (2S)-2-(methylamino)-3-phenyl-propanoic acid
  MUTAGEN 7: note = X stands for (2S)-2-(methylamino)-propanoic acid
  MUTAGEN 8: note = X stands for (S)-2-amino-3-(3-(carboxymethoxy)phenyl)-propanoic acid
  MUTAGEN 9: note = X stands for (S)-4-(2-amino-2-carboxyethyl)-benzoic acid
  MUTAGEN 11: note = X stands for (2S)-2-(methylamino)-3-phenyl-propanoic acid
  MUTAGEN 12: note = X stands for (S)-2-amino-nonanoic acid
  MUTAGEN 13: note = X stands for (2S)-2-(methylamino)-propanoic acid
  MUTAGEN 14: note = X stands for (2S)-2-(methylamino)-3-phenyl-propanoic acid
  MUTAGEN 15: note = X stands for D-cysteine
XAWYXIXXXRXXXXX

SEQ ID NO: 68 - protein, 15 aa, synthetic construct
  MUTAGEN 5: note = X stands for (2S)-2-(methylamino)-3-phenyl-propanoic acid
  MUTAGEN 7: note = X stands for (2S)-2-(methylamino)-propanoic acid
  MUTAGEN 8: note = X stands for (S)-2-amino-3-(3-(carboxymethoxy)phenyl)-propanoic acid
  MUTAGEN 9: note = X stands for (S)-4-(2-amino-2-carboxyethyl)-benzoic acid
  MUTAGEN 11: note = X stands for (2S)-2-(methylamino)-3-phenyl-propanoic acid
  MUTAGEN 12: note = X stands for (S)-2-amino-nonanoic acid
  MUTAGEN 13: note = X stands for (2S)-2-(methylamino)-propanoic acid
  MUTAGEN 14: note = X stands for (2S)-2-(methylamino)-3-phenyl-propanoic acid
  MUTAGEN 15: note = X stands for D-cysteine
ASWYXIXXXRXXXXX

SEQ ID NO: 69 - protein, 15 aa, synthetic construct
  MUTAGEN 1: note = X stands for 4-((carboxymethyl)amino)-butanoic acid
  MUTAGEN 5: note = X stands for (2S)-2-(methylamino)-3-phenyl-propanoic acid
  MUTAGEN 7: note = X stands for (2S)-2-(methylamino)-propanoic acid
  MUTAGEN 8: note = X stands for (S)-2-amino-3-(3-(carboxymethoxy)phenyl)-propanoic acid
  MUTAGEN 9: note = X stands for (S)-4-(2-amino-2-carboxyethyl)-benzoic acid
  MUTAGEN 11: note = X stands for (2S)-2-(methylamino)-3-phenyl-propanoic acid
  MUTAGEN 12: note = X stands for (S)-2-amino-dodecanoic acid
  MUTAGEN 13: note = X stands for (2S)-2-(methylamino)-propanoic acid
  MUTAGEN 14: note = X stands for (2S)-2-(methylamino)-3-phenyl-propanoic acid
  MUTAGEN 15: note = X stands for D-cysteine
XAWYXIXXXRXXXXX

SEQ ID NO: 70 - protein, 15 aa, synthetic construct
  MUTAGEN 1: note = X stands for 4-((carboxymethyl)amino)-butanoic acid
  MUTAGEN 5: note = X stands for (2S)-2-(methylamino)-3-phenyl-propanoic acid
  MUTAGEN 7: note = X stands for (2S)-2-(methylamino)-propanoic acid
  MUTAGEN 8: note = X stands for (S)-2-amino-3-(3-(carboxymethoxy)phenyl)-propanoic acid
  MUTAGEN 9: note = X stands for (S)-4-(2-amino-2-carboxyethyl)-benzoic acid
  MUTAGEN 11: note = X stands for (2S)-2-(methylamino)-3-phenyl-propanoic acid
  MUTAGEN 12: note = X stands for (S)-2-amino-decanoic acid
  MUTAGEN 13: note = X stands for (2S)-2-(methylamino)-propanoic acid
  MUTAGEN 14: note = X stands for (2S)-2-(methylamino)-3-phenyl-propanoic acid
  MUTAGEN 15: note = X stands for D-cysteine
XAWYXIXXXRXXXXX

SEQ ID NO: 71 - protein, 15 aa, synthetic construct
  MUTAGEN 1: note = X stands for 4-((carboxymethyl)amino)-butanoic acid
  MUTAGEN 5: note = X stands for (2S)-2-(methylamino)-3-phenyl-propanoic acid
  MUTAGEN 7: note = X stands for 2-(methylamino)-acetic acid
  MUTAGEN 8: note = X stands for (S)-2-amino-3-(3-(carboxymethoxy)phenyl)-propanoic acid
  MUTAGEN 9: note = X stands for (S)-4-(2-amino-2-carboxyethyl)-benzoic acid
  MUTAGEN 11: note = X stands for (2S)-2-(methylamino)-3-phenyl-propanoic acid
  MUTAGEN 12: note = X stands for (S)-2-amino-decanoic acid
  MUTAGEN 13: note = X stands for (2S)-2-(methylamino)-propanoic acid
  MUTAGEN 14: note = X stands for (2S)-2-(methylamino)-3-phenyl-propanoic acid
  MUTAGEN 15: note = X stands for D-cysteine
XAWYXIXXXRXXXXX

SEQ ID NO: 72 - protein, 15 aa, synthetic construct
  MUTAGEN 5: note = X stands for (2S)-2-(methylamino)-3-phenyl-propanoic acid
  MUTAGEN 7: note = X stands for 2-(methylamino)-acetic acid
  MUTAGEN 8: note = X stands for (S)-2-amino-3-(3-(carboxymethoxy)phenyl)-propanoic acid
  MUTAGEN 9: note = X stands for (S)-4-(2-amino-2-carboxyethyl)-benzoic acid
  MUTAGEN 11: note = X stands for (2S)-2-(methylamino)-3-phenyl-propanoic acid
  MUTAGEN 12: note = X stands for (S)-2-amino-heptanoic acid
  MUTAGEN 13: note = X stands for (2S)-2-(methylamino)-propanoic acid
  MUTAGEN 14: note = X stands for (2S)-2-(methylamino)-3-phenyl-propanoic acid
  MUTAGEN 15: note = X stands for D-cysteine
AAWYXIXXXRXXXXX

SEQ ID NO: 73 - protein, 15 aa, synthetic construct
  MUTAGEN 5: note = X stands for (2S)-2-(methylamino)-3-phenyl-propanoic acid
  MUTAGEN 7: note = X stands for 2-(methylamino)-acetic acid
  MUTAGEN 8: note = X stands for (S)-2-amino-3-(3-(carboxymethoxy)phenyl)-propanoic acid
  MUTAGEN 9: note = X stands for (S)-4-(2-amino-2-carboxyethyl)-benzoic acid
  MUTAGEN 11: note = X stands for (2S)-2-(methylamino)-3-phenyl-propanoic acid
  MUTAGEN 12: note = X stands for (S)-2-amino-octanoic acid
  MUTAGEN 13: note = X stands for (2S)-2-(methylamino)-propanoic acid
  MUTAGEN 14: note = X stands for (2S)-2-(methylamino)-3-phenyl-propanoic acid
  MUTAGEN 15: note = X stands for D-cysteine
AAWYXIXXXRXXXXX

SEQ ID NO: 74 - protein, 15 aa, synthetic construct
  MUTAGEN 7: note = X stands for 2-(methylamino)-acetic acid
  MUTAGEN 8: note = X stands for (S)-2-amino-3-(3-(carboxymethoxy)phenyl)-propanoic acid
  MUTAGEN 9: note = X stands for (S)-4-(2-amino-2-carboxyethyl)-benzoic acid
  MUTAGEN 11: note = X stands for (2S)-2-(methylamino)-3-phenyl-propanoic acid
  MUTAGEN 12: note = X stands for (S)-2-amino-nonanoic acid
  MUTAGEN 13: note = X stands for (2S)-2-(methylamino)-propanoic acid
  MUTAGEN 14: note = X stands for (2S)-2-(methylamino)-3-phenyl-propanoic acid
  MUTAGEN 15: note = X stands for D-cysteine
AAWYFIXXXRXXXXX

SEQ ID NO: 75 - protein, 15 aa, synthetic construct
  MUTAGEN 5: note = X stands for (2S)-2-(methylamino)-3-phenyl-propanoic acid
  MUTAGEN 7: note = X stands for 2-(methylamino)-acetic acid
  MUTAGEN 8: note = X stands for (S)-2-amino-3-(3-(carboxymethoxy)phenyl)-propanoic acid
  MUTAGEN 9: note = X stands for (S)-4-(2-amino-2-carboxyethyl)-benzoic acid
  MUTAGEN 11: note = X stands for (S)-2-(methylamino)-3-(pyridin-3-yl)-propanoic acid
  MUTAGEN 12: note = X stands for (S)-2-amino-nonanoic acid
  MUTAGEN 13: note = X stands for (2S)-2-(methylamino)-propanoic acid
  MUTAGEN 14: note = X stands for (2S)-2-(methylamino)-3-phenyl-propanoic acid
  MUTAGEN 15: note = X stands for D-cysteine
AAWYXIXXXRXXXXX

SEQ ID NO: 76 - protein, 15 aa, synthetic construct
  MUTAGEN 5: note = X stands for (2S)-2-(methylamino)-3-phenyl-propanoic acid
  MUTAGEN 7: note = X stands for 2-(methylamino)-acetic acid
  MUTAGEN 8: note = X stands for (S)-2-amino-3-(3-(carboxymethoxy)phenyl)-propanoic acid
  MUTAGEN 9: note = X stands for (S)-4-(2-amino-2-carboxyethyl)-benzoic acid
  MUTAGEN 12: note = X stands for (S)-2-amino-nonanoic acid
  MUTAGEN 13: note = X stands for (2S)-2-(methylamino)-propanoic acid
  MUTAGEN 14: note = X stands for (2S)-2-(methylamino)-3-phenyl-propanoic acid
  MUTAGEN 15: note = X stands for D-cysteine
AAWYXIXXXRFXXXX

SEQ ID NO: 77 - protein, 15 aa, synthetic construct
  MUTAGEN 5: note = X stands for (2S)-2-(methylamino)-3-phenyl-propanoic acid
  MUTAGEN 7: note = X stands for 2-(methylamino)-acetic acid
  MUTAGEN 8: note = X stands for (S)-2-amino-3-(3-(carboxymethoxy)phenyl)-propanoic acid
  MUTAGEN 9: note = X stands for (S)-4-(2-amino-2-carboxyethyl)-benzoic acid
  MUTAGEN 11: note = X stands for (2S)-2-(methylamino)-3-phenyl-propanoic acid
  MUTAGEN 12: note = X stands for (S)-2-amino-nonanoic acid
  MUTAGEN 13: note = X stands for (2S)-2-(methylamino)-propanoic acid
  MUTAGEN 14: note = X stands for (S)-2-(methylamino)-3-(pyridin-3-yl)-propanoic acid
  MUTAGEN 15: note = X stands for D-cysteine
AAWYXIXXXRXXXXX

SEQ ID NO: 78 - protein, 15 aa, synthetic construct
  MUTAGEN 5: note = X stands for (2S)-2-(methylamino)-3-phenyl-propanoic acid
  MUTAGEN 7: note = X stands for 2-(methylamino)-acetic acid
  MUTAGEN 8: note = X stands for (S)-2-amino-3-(3-(carboxymethoxy)phenyl)-propanoic acid
  MUTAGEN 9: note = X stands for (S)-4-(2-amino-2-carboxyethyl)-benzoic acid
  MUTAGEN 11: note = X stands for (2S)-2-(methylamino)-3-phenyl-propanoic acid
  MUTAGEN 12: note = X stands for (S)-2-amino-nonanoic acid
  MUTAGEN 13: note = X stands for (2S)-2-(methylamino)-propanoic acid
  MUTAGEN 14: note = X stands for (2S)-2-(methylamino)-3-phenyl-propanoic acid
AAWYXIXXXRXXXXC

SEQ ID NO: 79 - protein, 15 aa, synthetic construct
  MUTAGEN 5: note = X stands for (2S)-2-(methylamino)-3-phenyl-propanoic acid
  MUTAGEN 7: note = X stands for 2-(methylamino)-acetic acid
  MUTAGEN 8: note = X stands for (S)-2-amino-3-(3-(carboxymethoxy)phenyl)-propanoic acid
  MUTAGEN 9: note = X stands for (S)-4-(2-amino-2-carboxyethyl)-benzoic acid
  MUTAGEN 11: note = X stands for (2S)-2-(methylamino)-3-phenyl-propanoic acid
  MUTAGEN 12: note = X stands for (S)-2-amino-nonanoic acid
  MUTAGEN 13: note = X stands for (2S)-2-(methylamino)-propanoic acid
  MUTAGEN 14: note = X stands for (2S)-2-(methylamino)-3-phenyl-propanoic acid
  MUTAGEN 15: note = X stands for D-cysteine
NAWYXIXXXRXXXXX

SEQ ID NO: 80 - protein, 15 aa, synthetic construct
  MUTAGEN 2: note = X stands for D-glutamic acid
  MUTAGEN 3: note = X stands for (S)-2-amino-3-(1H-pyrrolo[2,3-b]pyridin-3-yl)-propanoic acid
  MUTAGEN 5: note = X stands for (2S)-2-(methylamino)-3-phenyl-propanoic acid
  MUTAGEN 7: note = X stands for 2-(methylamino)-acetic acid
  MUTAGEN 8: note = X stands for (S)-2-amino-3-(3-(carboxymethoxy)phenyl)-propanoic acid
  MUTAGEN 11: note = X stands for (2S)-2-(methylamino)-3-phenyl-propanoic acid
  MUTAGEN 12: note = X stands for (S)-2-amino-nonanoic acid
  MUTAGEN 13: note = X stands for (2S)-2-(methylamino)-propanoic acid
  MUTAGEN 14: note = X stands for (2S)-2-(methylamino)-3-phenyl-propanoic acid
  MUTAGEN 15: note = X stands for D-cysteine
AXXYXIXXYRXXXXX

SEQ ID NO: 81 - protein, 15 aa, synthetic construct
  MUTAGEN 1: note = X stands for 4-((carboxymethyl)amino)-butanoic acid
  MUTAGEN 5: note = X stands for (2S)-2-(methylamino)-3-phenyl-propanoic acid
  MUTAGEN 7: note = X stands for 2-(methylamino)-acetic acid
  MUTAGEN 8: note = X stands for (S)-2-amino-3-(pyridin-4-yl)-propanoic acid
  MUTAGEN 9: note = X stands for (S)-4-(2-amino-2-carboxyethyl)-benzoic acid
  MUTAGEN 11: note = X stands for (2S)-2-(methylamino)-3-phenyl-propanoic acid
  MUTAGEN 12: note = X stands for (2S)-2-amino-3-(pentyloxy)-propanoic acid
  MUTAGEN 13: note = X stands for (2S)-2-(methylamino)-propanoic acid
  MUTAGEN 14: note = X stands for (2S)-2-(methylamino)-3-phenyl-propanoic acid
  MUTAGEN 15: note = X stands for D-cysteine
XAWYXIXXXRXXXXX

SEQ ID NO: 82 - protein, 15 aa, synthetic construct
  MUTAGEN 1: note = X stands for 4-((carboxymethyl)amino)-butanoic acid
  MUTAGEN 5: note = X stands for (2S)-2-(methylamino)-3-phenyl-propanoic acid
  MUTAGEN 7: note = X stands for 2-(methylamino)-acetic acid
  MUTAGEN 8: note = X stands for (S)-2-amino-3-(pyridin-4-yl)-propanoic acid
  MUTAGEN 9: note = X stands for (S)-4-(2-amino-2-carboxyethyl)-benzoic acid
  MUTAGEN 11: note = X stands for (2S)-2-(methylamino)-3-phenyl-propanoic acid
  MUTAGEN 12: note = X stands for (2S)-2-amino-4-butoxy-butanoic acid
  MUTAGEN 13: note = X stands for (2S)-2-(methylamino)-propanoic acid
  MUTAGEN 14: note = X stands for (2S)-2-(methylamino)-3-phenyl-propanoic acid
  MUTAGEN 15: note = X stands for D-cysteine
XAWYXIXXXRXXXXX

SEQ ID NO: 83 - protein, 15 aa, synthetic construct
  MUTAGEN 1: note = X stands for 4-((carboxymethyl)amino)-butanoic acid
  MUTAGEN 5: note = X stands for (2S)-2-(methylamino)-3-phenyl-propanoic acid
  MUTAGEN 7: note = X stands for 2-(methylamino)-acetic acid
  MUTAGEN 8: note = X stands for (S)-2-amino-3-(pyridin-4-yl)-propanoic acid
  MUTAGEN 9: note = X stands for (S)-4-(2-amino-2-carboxyethyl)-benzoic acid
  MUTAGEN 11: note = X stands for (2S)-2-(methylamino)-3-phenyl-propanoic acid
  MUTAGEN 12: note = X stands for (2S)-2-amino-4-propoxy-butanoic acid
  MUTAGEN 13: note = X stands for (2S)-2-(methylamino)-propanoic acid
  MUTAGEN 14: note = X stands for (2S)-2-(methylamino)-3-phenyl-propanoic acid
  MUTAGEN 15: note = X stands for D-cysteine
XAWYXIXXXRXXXXX

SEQ ID NO: 84 - protein, 16 aa, synthetic construct
  MUTAGEN 2: note = X stands for D-glutamic acid
  MUTAGEN 5: note = X stands for (S)-3-cyclohexyl-2-(methylamino)-propanoic acid
  MUTAGEN 7: note = X stands for D-proline
  MUTAGEN 8: note = X stands for (2S)-2-amino-6-{[4-(carboxymethyl)piperazine-1-carbonyl]amino} hexanoic acid
  MUTAGEN 9: note = X stands for (S)-4-(2-amino-2-carboxyethyl)-benzoic acid
  MUTAGEN 11: note = X stands for (S)-2-amino-3-cyclohexyl-propanoic acid
  MUTAGEN 12: note = X stands for (S)-2-amino-nonanoic acid
  MUTAGEN 13: note = X stands for (2S)-2-(methylamino)-propanoic acid
  MUTAGEN 14: note = X stands for (2S)-2-(methylamino)-3-phenyl-propanoic acid
  MUTAGEN 15: note = X stands for D-cysteine
  MUTAGEN 16: note = X stands for 2-(piperazin-1-yl)-acetic acid
AXWYXIXXXRXXXXXX

SEQ ID NO: 85 - protein, 16 aa, synthetic construct
  MUTAGEN 2: note = X stands for D-glutamic acid
  MUTAGEN 5: note = X stands for (S)-3-cyclohexyl-2-(methylamino)-propanoic acid
  MUTAGEN 7: note = X stands for D-proline
  MUTAGEN 8: note = X stands for (2S)-2-amino-6-{[4-(carboxymethyl)piperazine-1-carbonyl]amino} hexanoic acid
  MUTAGEN 9: note = X stands for (S)-4-(2-amino-2-carboxyethyl)-benzoic acid
  MUTAGEN 11: note = X stands for (S)-3-cyclohexyl-2-(methylamino)-propanoic acid
  MUTAGEN 12: note = X stands for (S)-2-amino-nonanoic acid
  MUTAGEN 13: note = X stands for (2S)-2-(methylamino)-propanoic acid
  MUTAGEN 14: note = X stands for (2S)-2-(methylamino)-3-phenyl-propanoic acid
  MUTAGEN 15: note = X stands for D-cysteine
  MUTAGEN 16: note = X stands for 2-(piperazin-1-yl)-acetic acid
AXWYXIXXXRXXXXXX

SEQ ID NO: 86 - protein, 16 aa, synthetic construct
  MUTAGEN 2: note = X stands for D-glutamic acid
  MUTAGEN 5: note = X stands for (S)-3-cyclohexyl-2-(methylamino)-propanoic acid
  MUTAGEN 7: note = X stands for 2-(methylamino)-acetic acid
  MUTAGEN 8: note = X stands for (2S)-2-amino-6-{[4-(carboxymethyl)piperazine-1-carbonyl]amino} hexanoic acid
  MUTAGEN 9: note = X stands for (S)-4-(2-amino-2-carboxyethyl)-benzoic acid
  MUTAGEN 11: note = X stands for (S)-2-amino-3-cyclohexyl-propanoic acid
  MUTAGEN 12: note = X stands for (S)-2-amino-nonanoic acid
  MUTAGEN 13: note = X stands for (2S)-2-(methylamino)-propanoic acid
  MUTAGEN 14: note = X stands for (2S)-2-(methylamino)-3-phenyl-propanoic acid
  MUTAGEN 15: note = X stands for D-cysteine
  MUTAGEN 16: note = X stands for 2-(piperazin-1-yl)-acetic acid
AXWYXIXXXRXXXXXX

SEQ ID NO: 87 - protein, 16 aa, synthetic construct
  MUTAGEN 2: note = X stands for D-glutamic acid
  MUTAGEN 5: note = X stands for (S)-3-cyclohexyl-2-(methylamino)-propanoic acid
  MUTAGEN 7: note = X stands for D-proline
  MUTAGEN 8: note = X stands for (S)-2-amino-3-(3-(carboxymethoxy)phenyl)-propanoic acid
  MUTAGEN 9: note = X stands for (S)-4-(2-amino-2-carboxyethyl)-benzoic acid
  MUTAGEN 11: note = X stands for (2S)-2-(methylamino)-3-phenyl-propanoic acid
  MUTAGEN 12: note = X stands for (S)-2-amino-nonanoic acid
  MUTAGEN 13: note = X stands for (2S)-2-(methylamino)-propanoic acid
  MUTAGEN 14: note = X stands for (2S)-2-(methylamino)-3-phenyl-propanoic acid
  MUTAGEN 15: note = X stands for D-cysteine
  MUTAGEN 16: note = X stands for 2-(piperazin-1-yl)-acetic acid
AXWYXIXXXRXXXXXX

SEQ ID NO: 88 - protein, 16 aa, synthetic construct
  MUTAGEN 2: note = X stands for D-glutamic acid
  MUTAGEN 5: note = X stands for (2S)-2-(methylamino)-3-phenyl-propanoic acid
  MUTAGEN 7: note = X stands for D-proline
  MUTAGEN 8: note = X stands for (S)-2-amino-3-(3-(carboxymethoxy)phenyl)-propanoic acid
  MUTAGEN 9: note = X stands for (S)-4-(2-amino-2-carboxyethyl)-benzoic acid
  MUTAGEN 11: note = X stands for (2S)-2-(methylamino)-3-phenyl-propanoic acid
  MUTAGEN 12: note = X stands for (S)-2-amino-nonanoic acid
  MUTAGEN 14: note = X stands for (S)-2-amino-nonanoic acid
  MUTAGEN 13: note = X stands for (2S)-2-(methylamino)-propanoic acid
  MUTAGEN 15: note = X stands for D-cysteine
  MUTAGEN 16: note = X stands for 2-(piperazin-1-yl)-acetic acid
AXWYXIXXXRXXXXXX

SEQ ID NO: 89 - protein, 16 aa, synthetic construct
  MUTAGEN 2: note = X stands for D-glutamic acid
  MUTAGEN 5: note = X stands for (S)-3-cyclohexyl-2-(methylamino)-propanoic acid
  MUTAGEN 7: note = X stands for 2-(methylamino)-acetic acid
  MUTAGEN 8: note = X stands for (S)-2-amino-3-(3-(carboxymethoxy)phenyl)-propanoic acid
  MUTAGEN 9: note = X stands for (S)-4-(2-amino-2-carboxyethyl)-benzoic acid
  MUTAGEN 11: note = X stands for (2S)-2-(methylamino)-3-phenyl-propanoic acid
  MUTAGEN 12: note = X stands for (S)-2-amino-nonanoic acid
  MUTAGEN 13: note = X stands for (2S)-2-(methylamino)-propanoic acid
  MUTAGEN 14: note = X stands for (2S)-2-(methylamino)-3-phenyl-propanoic acid
  MUTAGEN 15: note = X stands for D-cysteine
  MUTAGEN 16: note = X stands for 2-(piperazin-1-yl)-acetic acid
AXWYXIXXXRXXXXXX

SEQ ID NO: 90 - protein, 16 aa, synthetic construct
  MUTAGEN 5: note = X stands for (2S)-2-(methylamino)-3-phenyl-propanoic acid
  MUTAGEN 7: note = X stands for 2-(methylamino)-acetic acid
  MUTAGEN 8: note = X stands for (S)-2-amino-3-(3-(carboxymethoxy)phenyl)-propanoic acid
  MUTAGEN 9: note = X stands for (S)-4-(2-amino-2-carboxyethyl)-benzoic acid
  MUTAGEN 11: note = X stands for (2S)-2-(methylamino)-3-phenyl-propanoic acid
  MUTAGEN 12: note = X stands for (S)-2-amino-nonanoic acid
  MUTAGEN 13: note = X stands for (2S)-2-(methylamino)-propanoic acid
  MUTAGEN 14: note = X stands for (2S)-2-(methylamino)-3-phenyl-propanoic acid
  MUTAGEN 15: note = X stands for D-cysteine
  MUTAGEN 16: note = X stands for 2-(piperazin-1-yl)-acetic acid
AAWYXIXXXRXXXXXX

SEQ ID NO: 91 - protein, 16 aa, synthetic construct
  MUTAGEN 5: note = X stands for (2S)-2-(methylamino)-3-phenyl-propanoic acid
  MUTAGEN 7: note = X stands for 2-(methylamino)-acetic acid
  MUTAGEN 8: note = X stands for (S)-2-amino-3-(3-(carboxymethoxy)phenyl)-propanoic acid
  MUTAGEN 9: note = X stands for (S)-4-(2-amino-2-carboxyethyl)-benzoic acid
  MUTAGEN 11: note = X stands for (S)-2-amino-3-cyclohexyl-propanoic acid
  MUTAGEN 12: note = X stands for (S)-2-amino-dodecanoic acid
  MUTAGEN 13: note = X stands for (2S)-2-(methylamino)-pentanedioic acid
  MUTAGEN 14: note = X stands for (2S)-2-(methylamino)-3-phenyl-propanoic acid
  MUTAGEN 15: note = X stands for D-cysteine
  MUTAGEN 16: note = X stands for 2-(piperazin-1-yl)-acetic acid
AAWYXIXXXRXXXXXX

SEQ ID NO: 92 - protein, 16 aa, synthetic construct
  MUTAGEN 5: note = X stands for (2S)-2-(methylamino)-3-phenyl-propanoic acid
  MUTAGEN 7: note = X stands for 2-(methylamino)-acetic acid
  MUTAGEN 8: note = X stands for (S)-2-amino-3-(3-(carboxymethoxy)phenyl)-propanoic acid
  MUTAGEN 9: note = X stands for (S)-4-(2-amino-2-carboxyethyl)-benzoic acid
  MUTAGEN 11: note = X stands for (2S)-2-(methylamino)-3-phenyl-propanoic acid
  MUTAGEN 12: note = X stands for (S)-2-amino-dodecanoic acid
  MUTAGEN 13: note = X stands for (2S)-2-(methylamino)-pentanedioic acid
  MUTAGEN 14: note = X stands for (2S)-2-(methylamino)-3-phenyl-propanoic acid
  MUTAGEN 15: note = X stands for D-cysteine
  MUTAGEN 16: note = X stands for 2-(piperazin-1-yl)-acetic acid
AAWYXIXXXRXXXXXX

SEQ ID NO: 93 - protein, 16 aa, synthetic construct
  MUTAGEN 4: note = X stands for (S)-2-amino-3-(4-(benzyloxy)phenyl)-propanoic acid
  MUTAGEN 5: note = X stands for (2S)-2-(methylamino)-3-phenyl-propanoic acid
  MUTAGEN 7: note = X stands for 2-(methylamino)-acetic acid
  MUTAGEN 8: note = X stands for (S)-2-amino-3-(3-(carboxymethoxy)phenyl)-propanoic acid
  MUTAGEN 9: note = X stands for (S)-4-(2-amino-2-carboxyethyl)-benzoic acid
  MUTAGEN 11: note = X stands for (2S)-2-(methylamino)-3-phenyl-propanoic acid
  MUTAGEN 12: note = X stands for (S)-2-amino-nonanoic acid
  MUTAGEN 13: note = X stands for (2S)-2-(methylamino)-propanoic acid
  MUTAGEN 14: note = X stands for (2S)-2-(methylamino)-3-phenyl-propanoic acid
  MUTAGEN 15: note = X stands for D-cysteine
  MUTAGEN 16: note = X stands for 2-(piperazin-1-yl)-acetic acid
AAWXXIXXXRXXXXXX

SEQ ID NO: 94 - protein, 16 aa, synthetic construct
  MUTAGEN 5: note = X stands for (2S)-2-(methylamino)-3-phenyl-propanoic acid
  MUTAGEN 7: note = X stands for D-proline
  MUTAGEN 8: note = X stands for (S)-2-amino-3-(3-(carboxymethoxy)phenyl)-propanoic acid
  MUTAGEN 9: note = X stands for (S)-4-(2-amino-2-carboxyethyl)-benzoic acid
  MUTAGEN 11: note = X stands for (2S)-2-(methylamino)-3-phenyl-propanoic acid
  MUTAGEN 12: note = X stands for (S)-2-amino-dodecanoic acid
  MUTAGEN 13: note = X stands for (2S)-2-(methylamino)-pentanedioic acid
  MUTAGEN 14: note = X stands for (2S)-2-(methylamino)-3-phenyl-propanoic acid
  MUTAGEN 15: note = X stands for D-cysteine
  MUTAGEN 16: note = X stands for 2-(piperazin-1-yl)-acetic acid
AAWYXIXXXRXXXXXX

SEQ ID NO: 95 - protein, 16 aa, synthetic construct
  MUTAGEN 5: note = X stands for (2S)-2-(methylamino)-3-phenyl-propanoic acid
  MUTAGEN 7: note = X stands for 2-(methylamino)-acetic acid
  MUTAGEN 8: note = X stands for (S)-2-amino-3-(3-(carboxymethoxy)phenyl)-propanoic acid
  MUTAGEN 9: note = X stands for (S)-4-(2-amino-2-carboxyethyl)-benzoic acid
  MUTAGEN 11: note = X stands for (2S)-2-(methylamino)-3-phenyl-propanoic acid
  MUTAGEN 12: note = X stands for (S)-2-amino-nonanoic acid
  MUTAGEN 13: note = X stands for (2S)-2-(methylamino)-pentanedioic acid
  MUTAGEN 14: note = X stands for (2S)-2-(methylamino)-3-phenyl-propanoic acid
  MUTAGEN 15: note = X stands for D-cysteine
  MUTAGEN 16: note = X stands for 2-(piperidine-4-yl)-acetic acid
AAWYXIXXXRXXXXXX

SEQ ID NO: 96 - protein, 16 aa, synthetic construct
  MUTAGEN 5: note = X stands for (2S)-2-(methylamino)-3-phenyl-propanoic acid
  MUTAGEN 7: note = X stands for 2-(methylamino)-acetic acid
  MUTAGEN 8: note = X stands for (S)-2-amino-3-(3-(carboxymethoxy)phenyl)-propanoic acid
  MUTAGEN 9: note = X stands for (S)-4-(2-amino-2-carboxyethyl)-benzoic acid
  MUTAGEN 11: note = X stands for (2S)-2-(methylamino)-3-phenyl-propanoic acid
  MUTAGEN 12: note = X stands for (S)-2-amino-nonanoic acid
  MUTAGEN 13: note = X stands for (2S)-2-(methylamino)-pentanedioic acid
  MUTAGEN 14: note = X stands for (2S)-2-(methylamino)-3-phenyl-propanoic acid
  MUTAGEN 15: note = X stands for D-cysteine
  MUTAGEN 16: note = X stands for 3-(piperidine-4-yl)-propanoic acid
AAWYXIXXXRXXXXXX

SEQ ID NO: 97 - protein, 16 aa, synthetic construct
  MUTAGEN 5: note = X stands for (2S)-2-(methylamino)-3-phenyl-propanoic acid
  MUTAGEN 7: note = X stands for D-proline
  MUTAGEN 8: note = X stands for (S)-2-amino-3-(3-(carboxymethoxy)phenyl)-propanoic acid
  MUTAGEN 9: note = X stands for (S)-4-(2-amino-2-carboxyethyl)-benzoic acid
  MUTAGEN 11: note = X stands for (2S)-2-(methylamino)-3-phenyl-propanoic acid
  MUTAGEN 12: note = X stands for (S)-2-amino-dodecanoic acid
  MUTAGEN 13: note = X stands for (2S)-2-(methylamino)-pentanedioic acid
  MUTAGEN 14: note = X stands for (2S)-2-(methylamino)-3-phenyl-propanoic acid
  MUTAGEN 15: note = X stands for D-cysteine
  MUTAGEN 16: note = X stands for 2-(piperidine-4-yl)-acetic acid
AAWYXIXXXRXXXXXX

SEQ ID NO: 98 - protein, 16 aa, synthetic construct
  MUTAGEN 3: note = X stands for (S)-2-amino-3-(1H-pyrrolo[2,3-c]pyridin-3-yl)-propanoic acid
  MUTAGEN 5: note = X stands for (2S)-2-(methylamino)-3-phenyl-propanoic acid
  MUTAGEN 7: note = X stands for D-proline
  MUTAGEN 8: note = X stands for (S)-2-amino-3-(3-(carboxymethoxy)phenyl)-propanoic acid
  MUTAGEN 9: note = X stands for (S)-4-(2-amino-2-carboxyethyl)-benzoic acid
  MUTAGEN 11: note = X stands for (2S)-2-(methylamino)-3-phenyl-propanoic acid
  MUTAGEN 12: note = X stands for (S)-2-amino-dodecanoic acid
  MUTAGEN 13: note = X stands for (2S)-2-(methylamino)-pentanedioic acid
  MUTAGEN 14: note = X stands for (2S)-2-(methylamino)-3-phenyl-propanoic acid
  MUTAGEN 15: note = X stands for D-cysteine
  MUTAGEN 16: note = X stands for 2-(piperidine-4-yl)-acetic acid
AAXYXIXXXRXXXXXX

SEQ ID NO: 99 - protein, 16 aa, synthetic construct
  MUTAGEN 3: note = X stands for (S)-2-amino-3-(1H-pyrrolo[2,3-c]pyridin-3-yl)-propanoic acid
  MUTAGEN 5: note = X stands for (2S)-2-(methylamino)-3-phenyl-propanoic acid
  MUTAGEN 7: note = X stands for 2-(ethylamino)-acetic acid
  MUTAGEN 8: note = X stands for (S)-2-amino-3-(3-(carboxymethoxy)phenyl)-propanoic acid
  MUTAGEN 9: note = X stands for (S)-4-(2-amino-2-carboxyethyl)-benzoic acid
  MUTAGEN 11: note = X stands for (2S)-2-(methylamino)-3-phenyl-propanoic acid
  MUTAGEN 12: note = X stands for (S)-2-amino-dodecanoic acid
  MUTAGEN 13: note = X stands for (2S)-2-(methylamino)-pentanedioic acid
  MUTAGEN 14: note = X stands for (2S)-2-(methylamino)-3-phenyl-propanoic acid
  MUTAGEN 15: note = X stands for D-cysteine
  MUTAGEN 16: note = X stands for 2-(piperidine-4-yl)-acetic acid
AAXYXIXXXRXXXXXX

SEQ ID NO: 100 - protein, 16 aa, synthetic construct
  MUTAGEN 3: note = X stands for (S)-2-amino-3-(1H-pyrrolo[2,3-c]pyridin-3-yl)-propanoic acid
  MUTAGEN 5: note = X stands for (2S)-2-(methylamino)-3-phenyl-propanoic acid
  MUTAGEN 6: note = X stands for (2S, 3R)-2-amino-3-methoxy-butanoic acid
  MUTAGEN 7: note = X stands for 2-(methylamino)-acetic acid
  MUTAGEN 8: note = X stands for (S)-2-amino-3-(3-(carboxymethoxy)phenyl)-propanoic acid
  MUTAGEN 9: note = X stands for (S)-4-(2-amino-2-carboxyethyl)-benzoic acid
  MUTAGEN 11: note = X stands for (2S)-2-(methylamino)-3-phenyl-propanoic acid
  MUTAGEN 12: note = X stands for (S)-2-amino-dodecanoic acid
  MUTAGEN 13: note = X stands for (2S)-2-(methylamino)-pentanedioic acid
  MUTAGEN 14: note = X stands for (2S)-2-(methylamino)-3-phenyl-propanoic acid
  MUTAGEN 15: note = X stands for D-cysteine
  MUTAGEN 16: note = X stands for 2-(piperidine-4-yl)-acetic acid
AAXYXXXXXRXXXXXX

SEQ ID NO: 101 - protein, 16 aa, synthetic construct
  MUTAGEN 5: note = X stands for (2S)-2-(methylamino)-3-phenyl-propanoic acid
  MUTAGEN 7: note = X stands for D-proline
  MUTAGEN 8: note = X stands for (S)-2-amino-3-(3-(carboxymethoxy)phenyl)-propanoic acid
  MUTAGEN 9: note = X stands for (S)-4-(2-amino-2-carboxyethyl)-benzoic acid
  MUTAGEN 11: note = X stands for (2S)-2-(methylamino)-3-phenyl-propanoic acid
  MUTAGEN 12: note = X stands for (S)-2-amino-dodecanoic acid
  MUTAGEN 13: note = X stands for (2S)-2-(methylamino)-pentanedioic acid
  MUTAGEN 14: note = X stands for (2S)-2-(methylamino)-3-phenyl-propanoic acid
  MUTAGEN 15: note = X stands for D-cysteine
  MUTAGEN 16: note = X stands for 3-(piperidine-4-yl)-propanoic acid
AAWYXIXXXRXXXXXX

SEQ ID NO: 102 - protein, 16 aa, synthetic construct
  MUTAGEN 5: note = X stands for (2S)-2-(methylamino)-3-phenyl-propanoic acid
  MUTAGEN 7: note = X stands for 2-(methylamino)-acetic acid
  MUTAGEN 8: note = X stands for (S)-2-amino-3-(3-(carboxymethoxy)phenyl)-propanoic acid
  MUTAGEN 9: note = X stands for (S)-4-(2-amino-2-carboxyethyl)-benzoic acid
  MUTAGEN 11: note = X stands for (2S)-2-(methylamino)-3-phenyl-propanoic acid
  MUTAGEN 12: note = X stands for (S)-2-amino-dodecanoic acid
  MUTAGEN 13: note = X stands for (2S)-2-(methylamino)-pentanedioic acid
  MUTAGEN 14: note = X stands for (2S)-2-(methylamino)-3-phenyl-propanoic acid
  MUTAGEN 15: note = X stands for D-cysteine
  MUTAGEN 16: note = X stands for 3-(piperidine-4-yl)-propanoic acid
AAWYXIXXXRXXXXXX

SEQ ID NO: 103 - protein, 16 aa, synthetic construct
  MUTAGEN 3: note = X stands for (S)-2-amino-3-(4'-(methylsulfonyl)-[1,1'-biphenyl]-4-yl)-propanoic acid
  MUTAGEN 5: note = X stands for (2S)-2-(methylamino)-3-phenyl-propanoic acid
  MUTAGEN 7: note = X stands for D-proline
  MUTAGEN 8: note = X stands for (S)-2-amino-3-(3-(carboxymethoxy)phenyl)-propanoic acid
  MUTAGEN 9: note = X stands for (S)-4-(2-amino-2-carboxyethyl)-benzoic acid
  MUTAGEN 11: note = X stands for (2S)-2-(methylamino)-3-phenyl-propanoic acid
  MUTAGEN 12: note = X stands for (S)-2-amino-dodecanoic acid
  MUTAGEN 13: note = X stands for (2S)-2-(methylamino)-pentanedioic acid
  MUTAGEN 14: note = X stands for (2S)-2-(methylamino)-3-phenyl-propanoic acid
  MUTAGEN 15: note = X stands for D-cysteine
  MUTAGEN 16: note = X stands for 2-(piperazin-1-yl)-acetic acid
AAXYXIXXXRXXXXXX

SEQ ID NO: 104 - protein, 15 aa, synthetic construct
  MUTAGEN 1: note = X stands for 4-((carboxymethyl)amino)-butanoic acid
  MUTAGEN 3: note = X stands for 4-{3-[(2S)-2-amino-2-carboxyethyl]-1H-indole-1-yl}-benzoic acid
  MUTAGEN 5: note = X stands for (2S)-2-(methylamino)-3-phenyl-propanoic acid
  MUTAGEN 7: note = X stands for (2S)-2-(methylamino)-propanoic acid
  MUTAGEN 8: note = X stands for (S)-2-amino-3-(3-(carboxymethoxy)phenyl)-propanoic acid
  MUTAGEN 9: note = X stands for (S)-4-(2-amino-2-carboxyethyl)-benzoic acid
  MUTAGEN 11: note = X stands for (2S)-2-(methylamino)-3-phenyl-propanoic acid
  MUTAGEN 12: note = X stands for (S)-2-amino-nonanoic acid
  MUTAGEN 13: note = X stands for (2S)-2-(methylamino)-propanoic acid
  MUTAGEN 14: note = X stands for (2S)-2-(methylamino)-3-phenyl-propanoic acid
  MUTAGEN 15: note = X stands for D-cysteine
XAXYXIXXXRXXXXX

SEQ ID NO: 105 - protein, 16 aa, synthetic construct
  MUTAGEN 3: note = X stands for (S)-2-amino-3-(6-hydroxy-1H-indol-3-yl)-propanoic acid
  MUTAGEN 5: note = X stands for (2S)-2-(methylamino)-3-phenyl-propanoic acid
  MUTAGEN 7: note = X stands for (2S)-2-(methylamino)-propanoic acid
  MUTAGEN 8: note = X stands for (S)-2-amino-3-(3-(carboxymethoxy)phenyl)-propanoic acid
  MUTAGEN 9: note = X stands for (S)-4-(2-amino-2-carboxyethyl)-benzoic acid
  MUTAGEN 11: note = X stands for (2S)-2-(methylamino)-3-phenyl-propanoic acid
  MUTAGEN 12: note = X stands for (S)-2-amino-dodecanoic acid
  MUTAGEN 13: note = X stands for (2S)-2-(methylamino)-pentanedioic acid
  MUTAGEN 14: note = X stands for (2S)-2-(methylamino)-3-phenyl-propanoic acid
  MUTAGEN 15: note = X stands for D-cysteine
  MUTAGEN 16: note = X stands for 3-(piperidine-4-yl)-propanoic acid
AAXYXIXXXRXXXXXX

SEQ ID NO: 106 - protein, 16 aa, synthetic construct
  MUTAGEN 3: note = X stands for (S)-2-amino-3-(6-hydroxy-1H-indol-3-yl)-propanoic acid
  MUTAGEN 5: note = X stands for (2S)-2-(methylamino)-3-phenyl-propanoic acid
  MUTAGEN 7: note = X stands for D-proline
  MUTAGEN 8: note = X stands for (S)-2-amino-3-(3-(carboxymethoxy)phenyl)-propanoic acid
  MUTAGEN 9: note = X stands for (S)-4-(2-amino-2-carboxyethyl)-benzoic acid
  MUTAGEN 11: note = X stands for (2S)-2-(methylamino)-3-phenyl-propanoic acid
  MUTAGEN 12: note = X stands for (S)-2-amino-dodecanoic acid
  MUTAGEN 13: note = X stands for (2S)-2-(methylamino)-pentanedioic acid
  MUTAGEN 14: note = X stands for (2S)-2-(methylamino)-3-phenyl-propanoic acid
  MUTAGEN 15: note = X stands for D-cysteine
  MUTAGEN 16: note = X stands for 3-(piperidine-4-yl)-propanoic acid
AAXYXIXXXRXXXXXX

SEQ ID NO: 107 - protein, 16 aa, synthetic construct
  MUTAGEN 3: note = X stands for (S)-2-amino-3-(6-hydroxy-1H-indol-3-yl)-propanoic acid
  MUTAGEN 5: note = X stands for (2S)-2-(methylamino)-3-phenyl-propanoic acid
  MUTAGEN 7: note = X stands for 2-(ethylamino)-acetic acid
  MUTAGEN 8: note = X stands for (S)-2-amino-3-(3-(carboxymethoxy)phenyl)-propanoic acid
  MUTAGEN 9: note = X stands for (S)-4-(2-amino-2-carboxyethyl)-benzoic acid
  MUTAGEN 11: note = X stands for (2S)-2-(methylamino)-3-phenyl-propanoic acid
  MUTAGEN 12: note = X stands for (S)-2-amino-dodecanoic acid
  MUTAGEN 13: note = X stands for (2S)-2-(methylamino)-pentanedioic acid
  MUTAGEN 14: note = X stands for (2S)-2-(methylamino)-3-phenyl-propanoic acid
  MUTAGEN 15: note = X stands for D-cysteine
  MUTAGEN 16: note = X stands for 3-(piperidine-4-yl)-propanoic acid
AAXYXIXXXRXXXXXX

SEQ ID NO: 108 - protein, 16 aa, synthetic construct
  MUTAGEN 3: note = X stands for (S)-2-amino-3-(6-hydroxy-1H-indol-3-yl)-propanoic acid
  MUTAGEN 5: note = X stands for (2S)-2-(methylamino)-3-phenyl-propanoic acid
  MUTAGEN 7: note = X stands for D-proline
  MUTAGEN 8: note = X stands for (S)-2-amino-3-(3-(carboxymethoxy)phenyl)-propanoic acid
  MUTAGEN 9: note = X stands for (S)-4-(2-amino-2-carboxyethyl)-benzoic acid
  MUTAGEN 11: note = X stands for (2S)-2-(methylamino)-3-phenyl-propanoic acid
  MUTAGEN 12: note = X stands for (S)-2-amino-dodecanoic acid
  MUTAGEN 13: note = X stands for (2S)-2-(methylamino)-pentanedioic acid
  MUTAGEN 14: note = X stands for (2S)-2-(methylamino)-3-phenyl-propanoic acid
  MUTAGEN 15: note = X stands for D-cysteine
  MUTAGEN 16: note = X stands for 2-(piperazin-1-yl)-acetic acid
AAXYXIXXXRXXXXXX

SEQ ID NO: 109 - protein, 16 aa, synthetic construct
  MUTAGEN 3: note = X stands for (S)-2-amino-3-(6-hydroxy-1H-indol-3-yl)-propanoic acid
  MUTAGEN 5: note = X stands for (2S)-2-(methylamino)-3-phenyl-propanoic acid
  MUTAGEN 7: note = X stands for 2-(ethylamino)-acetic acid
  MUTAGEN 8: note = X stands for (S)-2-amino-3-(3-(carboxymethoxy)phenyl)-propanoic acid
  MUTAGEN 9: note = X stands for (S)-4-(2-amino-2-carboxyethyl)-benzoic acid
  MUTAGEN 11: note = X stands for (2S)-2-(methylamino)-3-phenyl-propanoic acid
  MUTAGEN 12: note = X stands for (S)-2-amino-dodecanoic acid
  MUTAGEN 13: note = X stands for (2S)-2-(methylamino)-pentanedioic acid
  MUTAGEN 14: note = X stands for (2S)-2-(methylamino)-3-phenyl-propanoic acid
  MUTAGEN 15: note = X stands for D-cysteine
  MUTAGEN 16: note = X stands for 2-(piperazin-1-yl)-acetic acid
AAXYXIXXXRXXXXXX

SEQ ID NO: 110 - protein, 15 aa, synthetic construct
  MUTAGEN 5: note = X stands for (2S)-2-(methylamino)-3-phenyl-propanoic acid
  MUTAGEN 7: note = X stands for 2-(methylamino)-acetic acid
  MUTAGEN 11: note = X stands for (2S)-2-(methylamino)-3-phenyl-propanoic acid
  MUTAGEN 13: note = X stands for (2S)-2-(methylamino)-propanoic acid
  MUTAGEN 14: note = X stands for (2S)-2-(methylamino)-3-phenyl-propanoic acid
ARWYXIXYYRXLXXC

SEQ ID NO: 111 - protein, 15 aa, synthetic construct
  MUTAGEN 1: note = X stands for (2S)-2-(methylamino)-propanoic acid
  MUTAGEN 5: note = X stands for (2S)-2-(methylamino)-3-phenyl-propanoic acid
  MUTAGEN 7: note = X stands for 2-(methylamino)-acetic acid
  MUTAGEN 11: note = X stands for (2S)-2-(methylamino)-3-phenyl-propanoic acid
  MUTAGEN 13: note = X stands for (2S)-2-(methylamino)-propanoic acid
  MUTAGEN 14: note = X stands for (2S)-2-(methylamino)-3-phenyl-propanoic acid
XRWYXIXYYRXLXXC

SEQ ID NO: 112 - protein, 15 aa, synthetic construct
  MUTAGEN 5: note = X stands for (2S)-2-(methylamino)-3-phenyl-propanoic acid
  MUTAGEN 7: note = X stands for 2-(methylamino)-acetic acid
  MUTAGEN 11: note = X stands for (2S)-2-(methylamino)-3-phenyl-propanoic acid
  MUTAGEN 13: note = X stands for (2S)-2-(methylamino)-propanoic acid
  MUTAGEN 14: note = X stands for (2S)-2-(methylamino)-3-phenyl-propanoic acid
  MUTAGEN 15: note = X stands for (2R)-2-(methylamino)-3-sulfanyl-propanoic acid
ARWYXIXYYRXLXXX

SEQ ID NO: 113 - protein, 15 aa, synthetic construct
  MUTAGEN 5: note = X stands for (2S)-2-(methylamino)-3-phenyl-propanoic acid
  MUTAGEN 7: note = X stands for 2-(methylamino)-acetic acid
  MUTAGEN 11: note = X stands for (2S)-2-(methylamino)-3-phenyl-propanoic acid
  MUTAGEN 13: note = X stands for (2S)-2-(methylamino)-propanoic acid
  MUTAGEN 14: note = X stands for (2S)-2-(methylamino)-3-phenyl-propanoic acid
  MUTAGEN 15: note = X stands for D-cysteine
ARWYXIXYYRXLXXX

SEQ ID NO: 114 - protein, 16 aa, synthetic construct
  MUTAGEN 5: note = X stands for (2S)-2-(methylamino)-3-phenyl-propanoic acid
  MUTAGEN 7: note = X stands for 2-(methylamino)-acetic acid
  MUTAGEN 11: note = X stands for (2S)-2-(methylamino)-3-phenyl-propanoic acid
  MUTAGEN 13: note = X stands for (2S)-2-(methylamino)-propanoic acid
  MUTAGEN 14: note = X stands for (2S)-2-(methylamino)-3-phenyl-propanoic acid
  MUTAGEN 16: note = X stands for (2S)-2,3-diamino-propionic acid
ARWYXIXYYRXLXXCX

SEQ ID NO: 115 - protein, 15 aa, synthetic construct
  MUTAGEN 2: note = X stands for (2S)-2,3-diamino-propionic acid
  MUTAGEN 5: note = X stands for (2S)-2-(methylamino)-3-phenyl-propanoic acid
  MUTAGEN 7: note = X stands for 2-(methylamino)-acetic acid
  MUTAGEN 11: note = X stands for (2S)-2-(methylamino)-3-phenyl-propanoic acid
  MUTAGEN 13: note = X stands for (2S)-2-(methylamino)-propanoic acid
  MUTAGEN 14: note = X stands for (2S)-2-(methylamino)-3-phenyl-propanoic acid
AXWYXIXYYRXLXXC

SEQ ID NO: 116 - protein, 16 aa, synthetic construct
  MUTAGEN 5: note = X stands for (2S)-2-(methylamino)-3-phenyl-propanoic acid
  MUTAGEN 7: note = X stands for 2-(methylamino)-acetic acid
  MUTAGEN 11: note = X stands for (2S)-2-(methylamino)-3-phenyl-propanoic acid
  MUTAGEN 13: note = X stands for (2S)-2-(methylamino)-propanoic acid
  MUTAGEN 14: note = X stands for (2S)-2-(methylamino)-3-phenyl-propanoic acid
  MUTAGEN 16: note = X stands for D-glutamic acid
ARWYXIXYYRXLXXCX

SEQ ID NO: 117 - protein, 15 aa, synthetic construct
  MUTAGEN 5: note = X stands for (2S)-2-(methylamino)-3-phenyl-propanoic acid
  MUTAGEN 7: note = X stands for 2-(methylamino)-acetic acid
  MUTAGEN 11: note = X stands for (2S)-2-(methylamino)-3-phenyl-propanoic acid
  MUTAGEN 13: note = X stands for (2S)-2-(methylamino)-propanoic acid
  MUTAGEN 14: note = X stands for (2S)-2-(methylamino)-3-phenyl-propanoic acid
AKWYXIXYYRXLXXC

SEQ ID NO: 118 - protein, 15 aa, synthetic construct
  MUTAGEN 5: note = X stands for (2S)-2-(methylamino)-3-phenyl-propanoic acid
  MUTAGEN 7: note = X stands for 2-(methylamino)-acetic acid
  MUTAGEN 11: note = X stands for (2S)-2-(methylamino)-3-phenyl-propanoic acid
  MUTAGEN 13: note = X stands for (2S)-2-(methylamino)-propanoic acid
  MUTAGEN 14: note = X stands for (2S)-2-(methylamino)-3-phenyl-propanoic acid
AEWYXIXYYRXLXXC

SEQ ID NO: 119 - protein, 15 aa, synthetic construct
  MUTAGEN 1: note = X stands for (2S)-2,3-diamino-propionic acid
  MUTAGEN 5: note = X stands for (2S)-2-(methylamino)-3-phenyl-propanoic acid
  MUTAGEN 7: note = X stands for 2-(methylamino)-acetic acid
  MUTAGEN 11: note = X stands for (2S)-2-(methylamino)-3-phenyl-propanoic acid
  MUTAGEN 13: note = X stands for (2S)-2-(methylamino)-propanoic acid
  MUTAGEN 14: note = X stands for (2S)-2-(methylamino)-3-phenyl-propanoic acid
XRWYXIXYYRXLXXC

SEQ ID NO: 120 - protein, 15 aa, synthetic construct
  MUTAGEN 1: note = X standards for 2-[(3-aminopropyl)amino]-acetic acid
  MUTAGEN 5: note = X stands for (2S)-2-(methylamino)-3-phenyl-propanoic acid
  MUTAGEN 7: note = X stands for 2-(methylamino)-acetic acid
  MUTAGEN 11: note = X stands for (2S)-2-(methylamino)-3-phenyl-propanoic acid
  MUTAGEN 13: note = X stands for (2S)-2-(methylamino)-propanoic acid
  MUTAGEN 14: note = X stands for (2S)-2-(methylamino)-3-phenyl-propanoic acid
XRWYXIXYYRXLXXC

SEQ ID NO: 121 - protein, 15 aa, synthetic construct
  MUTAGEN 5: note = X stands for (2S)-2-(methylamino)-3-phenyl-propanoic acid
  MUTAGEN 7: note = X stands for 2-(methylamino)-acetic acid
  MUTAGEN 11: note = X stands for (2S)-2-(methylamino)-3-phenyl-propanoic acid
  MUTAGEN 13: note = X stands for (2S)-2-(methylamino)-propanoic acid
  MUTAGEN 14: note = X stands for (2S)-2-(methylamino)-3-phenyl-propanoic acid
AAWYXIXYYRXLXXC

SEQ ID NO: 122 - protein, 15 aa, synthetic construct
  MUTAGEN 2: note = X stands for D-alanine
  MUTAGEN 5: note = X stands for (2S)-2-(methylamino)-3-phenyl-propanoic acid
  MUTAGEN 7: note = X stands for 2-(methylamino)-acetic acid
  MUTAGEN 11: note = X stands for (2S)-2-(methylamino)-3-phenyl-propanoic acid
  MUTAGEN 13: note = X stands for (2S)-2-(methylamino)-propanoic acid
  MUTAGEN 14: note = X stands for (2S)-2-(methylamino)-3-phenyl-propanoic acid
  MUTAGEN 15: note = X stands for D-cysteine
AXWYXIXYYRXLXXX

SEQ ID NO: 123 - protein, 15 aa, synthetic construct
  MUTAGEN 1: note = X stands for 4-((carboxymethyl)amino)-butanoic acid
  MUTAGEN 5: note = X stands for (2S)-2-(methylamino)-3-phenyl-propanoic acid
  MUTAGEN 7: note = X stands for 2-(methylamino)-acetic acid
  MUTAGEN 8: note = X stands for (S)-4-(2-amino-2-carboxyethyl)-benzoic acid
  MUTAGEN 11: note = X stands for (2S)-2-(methylamino)-3-phenyl-propanoic acid
  MUTAGEN 13: note = X stands for (2S)-2-(methylamino)-propanoic acid
  MUTAGEN 14: note = X stands for (2S)-2-(methylamino)-3-phenyl-propanoic acid
  MUTAGEN 15: note = X stands for D-cysteine
XAWYXIXXYRXLXXX

SEQ ID NO: 124 - protein, 16 aa, synthetic construct
  MUTAGEN 2: note = X stands for (2S)-2,3-diamino-propioic acid
  MUTAGEN 5: note = X stands for (2S)-2-(methylamino)-3-phenyl-propanoic acid
  MUTAGEN 7: note = X stands for 2-(methylamino)-acetic acid
  MUTAGEN 11: note = X stands for (2S)-2-(methylamino)-3-phenyl-propanoic acid
  MUTAGEN 13: note = X stands for (2S)-2-(methylamino)-propanoic acid
  MUTAGEN 14: note = X stands for (2S)-2-(methylamino)-3-phenyl-propanoic acid
  MUTAGEN 15: note = X stands for D-cysteine
  MUTAGEN 16: note = X stands for (2S)-2,3-diamino-propionic acid
AXWYXIXYYRXLXXXX

SEQ ID NO: 125 - protein, 16 aa, synthetic construct
  MUTAGEN 1: note = X standards for 2-[(3-aminopropyl)amino]-acetic acid
  MUTAGEN 5: note = X stands for (2S)-2-(methylamino)-3-phenyl-propanoic acid
  MUTAGEN 7: note = X stands for 2-(methylamino)-acetic acid
  MUTAGEN 11: note = X stands for (2S)-2-(methylamino)-3-phenyl-propanoic acid
  MUTAGEN 13: note = X stands for (2S)-2-(methylamino)-propanoic acid
  MUTAGEN 14: note = X stands for (2S)-2-(methylamino)-3-phenyl-propanoic acid
  MUTAGEN 15: note = X stands for D-cysteine
  MUTAGEN 16: note = X stands for (2S)-2,3-diamino-propionic acid
XAWYXIXYYRXLXXXX

SEQ ID NO: 126 - protein, 17 aa, synthetic construct
  MUTAGEN 2: note = X stands for (2S)-2,3-diamino-propionic acid
  MUTAGEN 5: note = X stands for (2S)-2-(methylamino)-3-phenyl-propanoic acid
  MUTAGEN 7: note = X stands for 2-(methylamino)-acetic acid
  MUTAGEN 11: note = X stands for (2S)-2-(methylamino)-3-phenyl-propanoic acid
  MUTAGEN 13: note = X stands for (2S)-2-(methylamino)-propanoic acid
  MUTAGEN 14: note = X stands for (2S)-2-(methylamino)-3-phenyl-propanoic acid
  MUTAGEN 15: note = X stands for D-cysteine
  MUTAGEN 16: note = X stands for (2S)-2,3-diamino-propionic acid
  MUTAGEN 17: note = X stands for (2S)-2,3-diamino-propionic acid
AXWYXIXYYRXLXXXXX

SEQ ID NO: 127 - protein, 16 aa, synthetic construct
  MUTAGEN 5: note = X stands for (2S)-2-(methylamino)-3-phenyl-propanoic acid
  MUTAGEN 7: note = X stands for 2-(methylamino)-acetic acid
  MUTAGEN 11: note = X stands for (2S)-2-(methylamino)-3-phenyl-propanoic acid
  MUTAGEN 13: note = X stands for (2S)-2-(methylamino)-propanoic acid
  MUTAGEN 14: note = X stands for (2S)-2-(methylamino)-3-phenyl-propanoic acid
  MUTAGEN 15: note = X stands for D-cysteine
  MUTAGEN 16: note = X stands for (2S)-2,3-diamino-propionic acid
AAWYXIXKYRXLXXXX

SEQ ID NO: 128 - protein, 15 aa, synthetic construct
  MUTAGEN 1: note = X standards for 2-[(3-aminopropyl)amino]-acetic acid
  MUTAGEN 2: note = X stands for (2S)-2,3-diamino-propionic acid
  MUTAGEN 5: note = X stands for (2S)-2-(methylamino)-3-phenyl-propanoic acid
  MUTAGEN 7: note = X stands for 2-(methylamino)-acetic acid
  MUTAGEN 11: note = X stands for (2S)-2-(methylamino)-3-phenyl-propanoic acid
  MUTAGEN 13: note = X stands for (2S)-2-(methylamino)-propanoic acid
  MUTAGEN 14: note = X stands for (2S)-2-(methylamino)-3-phenyl-propanoic acid
  MUTAGEN 15: note = X stands for D-cysteine
XXWYXIXYYRXLXXX

SEQ ID NO: 129 - protein, 15 aa, synthetic construct
  MUTAGEN 1: note = X stands for 4-((carboxymethyl)amino)-butanoic acid
  MUTAGEN 3: note = X stands for (S)-2-amino-3-(1H-pyrrolo[2,3-b]pyridin-3-yl)-propanoic acid
  MUTAGEN 5: note = X stands for (2S)-2-(methylamino)-3-phenyl-propanoic acid
  MUTAGEN 7: note = X stands for 2-(methylamino)-acetic acid
  MUTAGEN 9: note = X stands for (S)-4-(2-amino-2-carboxyethyl)-benzoic acid
  MUTAGEN 11: note = X stands for (2S)-2-(methylamino)-3-phenyl-propanoic acid
  MUTAGEN 13: note = X stands for (2S)-2-(methylamino)-propanoic acid
  MUTAGEN 14: note = X stands for (2S)-2-(methylamino)-3-phenyl-propanoic acid
  MUTAGEN 15: note = X stands for D-cysteine
XAXYXIXYXRXLXXX

SEQ ID NO: 130 - protein, 15 aa, synthetic construct
  MUTAGEN 1: note = X stands for 4-((carboxymethyl)amino)-butanoic acid
  MUTAGEN 5: note = X stands for (2S)-2-(methylamino)-3-phenyl-propanoic acid
  MUTAGEN 7: note = X stands for (2S)-2-(methylamino)-propanoic acid
  MUTAGEN 9: note = X stands for (S)-4-(2-amino-2-carboxyethyl)-benzoic acid
  MUTAGEN 11: note = X stands for (2S)-2-(methylamino)-3-phenyl-propanoic acid
  MUTAGEN 13: note = X stands for (2S)-2-(methylamino)-propanoic acid
  MUTAGEN 14: note = X stands for (2S)-2-(methylamino)-3-phenyl-propanoic acid
  MUTAGEN 15: note = X stands for D-cysteine
XAWYXIXYXRXLXXX

SEQ ID NO: 131 - protein, 15 aa, synthetic construct
  MUTAGEN 1: note = X stands for 4-((carboxymethyl)amino)-butanoic acid
  MUTAGEN 5: note = X stands for (2S)-2-(methylamino)-3-phenyl-propanoic acid
  MUTAGEN 7: note = X stands for 2-(methylamino)-acetic acid
  MUTAGEN 9: note = X stands for (S)-2-amino-3-(pyridin-3-yl)-propanoic acid
  MUTAGEN 11: note = X stands for (2S)-2-(methylamino)-3-phenyl-propanoic acid
  MUTAGEN 13: note = X stands for (2S)-2-(methylamino)-propanoic acid
  MUTAGEN 14: note = X stands for (2S)-2-(methylamino)-3-phenyl-propanoic acid
  MUTAGEN 15: note = X stands for D-cysteine
XAWYXIXYXRXLXXX

SEQ ID NO: 132 - protein, 15 aa, synthetic construct
  MUTAGEN 1: note = X stands for 4-((carboxymethyl)amino)-butanoic acid
  MUTAGEN 5: note = X stands for (2S)-2-(methylamino)-3-phenyl-propanoic acid
  MUTAGEN 7: note = X stands for 2-(methylamino)-acetic acid
  MUTAGEN 9: note = X stands for (S)-2-amino-3-(pyridin-4-yl)-propanoic acid
  MUTAGEN 11: note = X stands for (2S)-2-(methylamino)-3-phenyl-propanoic acid
  MUTAGEN 13: note = X stands for (2S)-2-(methylamino)-propanoic acid
  MUTAGEN 14: note = X stands for (2S)-2-(methylamino)-3-phenyl-propanoic acid
  MUTAGEN 15: note = X stands for D-cysteine
XAWYXIXYXRXLXXX

SEQ ID NO: 133 - protein, 15 aa, synthetic construct
  MUTAGEN 1: note = X stands for 4-((carboxymethyl)amino)-butanoic acid
  MUTAGEN 5: note = X stands for (2S)-2-(methylamino)-3-phenyl-propanoic acid
  MUTAGEN 7: note = X stands for 2-(methylamino)-acetic acid
  MUTAGEN 8: note = X stands for (S)-2-amino-3-(pyridin-4-yl)-propanoic acid
  MUTAGEN 9: note = X stands for (S)-4-(2-amino-2-carboxyethyl)-benzoic acid
  MUTAGEN 11: note = X stands for (2S)-2-(methylamino)-3-phenyl-propanoic acid
  MUTAGEN 13: note = X stands for (2S)-2-(methylamino)-propanoic acid
  MUTAGEN 14: note = X stands for (2S)-2-(methylamino)-3-phenyl-propanoic acid
  MUTAGEN 15: note = X stands for D-cysteine
XAWYXIXXXRXLXXX

SEQ ID NO: 134 - protein, 15 aa, synthetic construct
  MUTAGEN 1: note = X stands for 4-((carboxymethyl)amino)-butanoic acid
  MUTAGEN 3: note = X stands for (S)-2-amino-3-(1H-pyrrolo[2,3-b]pyridin-3-yl)-propanoic acid
  MUTAGEN 5: note = X stands for (2S)-2-(methylamino)-3-phenyl-propanoic acid
  MUTAGEN 7: note = X stands for 2-(methylamino)-acetic acid
  MUTAGEN 9: note = X stands for (S)-4-(2-amino-2-carboxyethyl)-benzoic acid
  MUTAGEN 11: note = X stands for (2S)-2-(methylamino)-3-phenyl-propanoic acid
  MUTAGEN 13: note = X stands for (2S)-2-(methylamino)-propanoic acid
  MUTAGEN 14: note = X stands for (2S)-2-(methylamino)-3-phenyl-propanoic acid
  MUTAGEN 15: note = X stands for D-cysteine
XAXYXIXFXRXLXXX

SEQ ID NO: 135 - protein, 15 aa, synthetic construct
  MUTAGEN 1: note = X stands for 4-((carboxymethyl)amino)-butanoic acid
  MUTAGEN 3: note = X stands for (S)-2-amino-3-(1H-pyrrolo[2,3-b]pyridin-3-yl)-propanoic acid
  MUTAGEN 5: note = X stands for (2S)-2-(methylamino)-3-phenyl-propanoic acid
  MUTAGEN 7: note = X stands for 2-(methylamino)-acetic acid
  MUTAGEN 8: note = X stands for (S)-2-amino-3-(pyridin-4-yl)-propanoic acid
  MUTAGEN 9: note = X stands for (S)-4-(2-amino-2-carboxyethyl)-benzoic acid
  MUTAGEN 11: note = X stands for (2S)-2-(methylamino)-3-phenyl-propanoic acid
  MUTAGEN 13: note = X stands for (2S)-2-(methylamino)-propanoic acid
  MUTAGEN 14: note = X stands for (2S)-2-(methylamino)-3-phenyl-propanoic acid
  MUTAGEN 15: note = X stands for D-cysteine
XAXYXIXFXRXLXXX

SEQ ID NO: 136 - protein, 15 aa, synthetic construct
  MUTAGEN 1: note = X stands for 4-((carboxymethyl)amino)-butanoic acid
  MUTAGEN 3: note = X stands for (S)-2-amino-3-(1H-pyrrolo[2,3-b]pyridin-3-yl)-propanoic acid
  MUTAGEN 5: note = X stands for (2S)-2-(methylamino)-3-phenyl-propanoic acid
  MUTAGEN 7: note = X stands for 2-(methylamino)-acetic acid
  MUTAGEN 9: note = X stands for (S)-2-amino-3-(pyridin-3-yl)-propanoic acid
  MUTAGEN 11: note = X stands for (2S)-2-(methylamino)-3-phenyl-propanoic acid
  MUTAGEN 13: note = X stands for (2S)-2-(methylamino)-propanoic acid
  MUTAGEN 14: note = X stands for (2S)-2-(methylamino)-3-phenyl-propanoic acid
  MUTAGEN 15: note = X stands for D-cysteine
XAXYXIXFXRXLXXX

SEQ ID NO: 137 - protein, 15 aa, synthetic construct
  MUTAGEN 1: note = X stands for 4-((carboxymethyl)amino)-butanoic acid
  MUTAGEN 5: note = X stands for (2S)-2-(methylamino)-3-phenyl-propanoic acid
  MUTAGEN 7: note = X stands for 2-(methylamino)-acetic acid
  MUTAGEN 8: note = X stands for (S)-2-amino-3-(pyridin-4-yl)-propanoic acid
  MUTAGEN 9: note = X stands for (S)-2-amino-3-(pyridin-3-yl)-propanoic acid
  MUTAGEN 11: note = X stands for (2S)-2-(methylamino)-3-phenyl-propanoic acid
  MUTAGEN 13: note = X stands for (2S)-2-(methylamino)-propanoic acid
  MUTAGEN 14: note = X stands for (2S)-2-(methylamino)-3-phenyl-propanoic acid
  MUTAGEN 15: note = X stands for D-cysteine
XAWYXIXXXRXLXXX

SEQ ID NO: 138 - protein, 15 aa, synthetic construct
  MUTAGEN 1: note = X stands for 4-((carboxymethyl)amino)-butanoic acid
  MUTAGEN 3: note = X stands for (S)-2-amino-3-(1H-pyrrolo[2,3-b]pyridin-3-yl)-propanoic acid
  MUTAGEN 4: note = X stands for (S)-2-amino-3-(6-aminopyridin-3-yl)-propanoic acid
  MUTAGEN 5: note = X stands for (2S)-2-(methylamino)-3-phenyl-propanoic acid
  MUTAGEN 7: note = X stands for 2-(methylamino)-acetic acid
  MUTAGEN 9: note = X stands for (S)-4-(2-amino-2-carboxyethyl)-benzoic acid
  MUTAGEN 11: note = X stands for (2S)-2-(methylamino)-3-phenyl-propanoic acid
  MUTAGEN 13: note = X stands for (2S)-2-(methylamino)-propanoic acid
  MUTAGEN 14: note = X stands for (2S)-2-(methylamino)-3-phenyl-propanoic acid
  MUTAGEN 15: note = X stands for D-cysteine
XAXXXIXFXRXLXXX

SEQ ID NO: 139 - protein, 15 aa, synthetic construct
  MUTAGEN 1: note = X stands for 4-((carboxymethyl)amino)-butanoic acid
  MUTAGEN 4: note = X stands for (S)-2-amino-3-(6-aminopyridin-3-yl)-propanoic acid
  MUTAGEN 5: note = X stands for (2S)-2-(methylamino)-3-phenyl-propanoic acid
  MUTAGEN 7: note = X stands for 2-(methylamino)-acetic acid
  MUTAGEN 8: note = X stands for (S)-2-amino-3-(pyridin-4-yl)-propanoic acid
  MUTAGEN 9: note = X stands for (S)-4-(2-amino-2-carboxyethyl)-benzoic acid
  MUTAGEN 11: note = X stands for (2S)-2-(methylamino)-3-phenyl-propanoic acid
  MUTAGEN 13: note = X stands for (2S)-2-(methylamino)-propanoic acid
  MUTAGEN 14: note = X stands for (2S)-2-(methylamino)-3-phenyl-propanoic acid
  MUTAGEN 15: note = X stands for D-cysteine
XAWXXIXXXRXLXXX

SEQ ID NO: 140 - protein, 15 aa, synthetic construct
  MUTAGEN 1: note = X stands for 4-((carboxymethyl)amino)-butanoic acid
  MUTAGEN 4: note = X stands for (S)-2-amino-3-(6-aminopyridin-3-yl)-propanoic acid
  MUTAGEN 5: note = X stands for (2S)-2-(methylamino)-3-phenyl-propanoic acid
  MUTAGEN 7: note = X stands for 2-(methylamino)-acetic acid
  MUTAGEN 9: note = X stands for (S)-2-amino-3-(pyridin-3-yl)-propanoic acid
  MUTAGEN 11: note = X stands for (2S)-2-(methylamino)-3-phenyl-propanoic acid
  MUTAGEN 13: note = X stands for (2S)-2-(methylamino)-propanoic acid
  MUTAGEN 14: note = X stands for (2S)-2-(methylamino)-3-phenyl-propanoic acid
  MUTAGEN 15: note = X stands for D-cysteine
XAWXXIXFXRXLXXX

SEQ ID NO: 141 - protein, 19 aa, synthetic construct
  MUTAGEN 1: note = X stands for 4-((carboxymethyl)amino)-butanoic acid
  MUTAGEN 5: note = X stands for (2S)-2-(methylamino)-3-phenyl-propanoic acid
  MUTAGEN 7: note = X stands for 2-(methylamino)-acetic acid
  MUTAGEN 9: note = X stands for (S)-4-(2-amino-2-carboxyethyl)-benzoic acid
  MUTAGEN 11: note = X stands for (2S)-2-(methylamino)-3-phenyl-propanoic acid
  MUTAGEN 13: note = X stands for (2S)-2-(methylamino)-propanoic acid
  MUTAGEN 14: note = X stands for (2S)-2-(methylamino)-3-phenyl-propanoic acid
  MUTAGEN 15: note = X stands for D-cysteine
  MUTAGEN 17: note = X stands for D-glutamic acid
  MUTAGEN 19: note = X stands for D-lysine
XAWYXIXYXRXLXXXGXGX

SEQ ID NO: 142 - protein, 19 aa, synthetic construct
  MUTAGEN 3: note = X stands for (S)-2-amino-3-(1H-pyrrolo[2,3-b]pyridin-3-yl)-propanoic acid
  MUTAGEN 5: note = X stands for (2S)-2-(methylamino)-3-phenyl-propanoic acid
  MUTAGEN 7: note = X stands for 2-(methylamino)-acetic acid
  MUTAGEN 9: note = X stands for (S)-4-(2-amino-2-carboxyethyl)-benzoic acid
  MUTAGEN 11: note = X stands for (2S)-2-(methylamino)-3-phenyl-propanoic acid
  MUTAGEN 13: note = X stands for (2S)-2-(methylamino)-propanoic acid
  MUTAGEN 14: note = X stands for (2S)-2-(methylamino)-3-phenyl-propanoic acid
  MUTAGEN 15: note = X stands for D-cysteine
  MUTAGEN 17: note = X stands for D-glutamic acid
  MUTAGEN 19: note = X stands for D-lysine
AAXYXIXFXRXLXXXGXGX

SEQ ID NO: 143 - protein, 19 aa, synthetic construct
  MUTAGEN 3: note = X stands for (S)-2-amino-3-(1H-pyrrolo[2,3-b]pyridin-3-yl)-propanoic acid
  MUTAGEN 5: note = X stands for (2S)-2-(methylamino)-3-phenyl-propanoic acid
  MUTAGEN 7: note = X stands for 2-(methylamino)-acetic acid
  MUTAGEN 8: note = X stands for (S)-2-amino-3-(pyridin-4-yl)-propanoic acid
  MUTAGEN 9: note = X stands for (S)-4-(2-amino-2-carboxyethyl)-benzoic acid
  MUTAGEN 11: note = X stands for (2S)-2-(methylamino)-3-phenyl-propanoic acid
  MUTAGEN 13: note = X stands for (2S)-2-(methylamino)-propanoic acid
  MUTAGEN 14: note = X stands for (2S)-2-(methylamino)-3-phenyl-propanoic acid
  MUTAGEN 15: note = X stands for D-cysteine
  MUTAGEN 17: note = X stands for D-glutamic acid
  MUTAGEN 19: note = X stands for D-lysine
AAXYXIXXXRXLXXXGXGX

SEQ ID NO: 144 - protein, 19 aa, synthetic construct
  MUTAGEN 1: note = X stands for 4-((carboxymethyl)amino)-butanoic acid
  MUTAGEN 3: note = X stands for (S)-2-amino-3-(1H-pyrrolo[2,3-b]pyridin-3-yl)-propanoic acid
  MUTAGEN 5: note = X stands for (2S)-2-(methylamino)-3-phenyl-propanoic acid
  MUTAGEN 7: note = X stands for 2-(methylamino)-acetic acid
  MUTAGEN 9: note = X stands for (S)-4-(2-amino-2-carboxyethyl)-benzoic acid
  MUTAGEN 11: note = X stands for (2S)-2-(methylamino)-3-phenyl-propanoic acid
  MUTAGEN 13: note = X stands for (2S)-2-(methylamino)-propanoic acid
  MUTAGEN 14: note = X stands for (2S)-2-(methylamino)-3-phenyl-propanoic acid
  MUTAGEN 15: note = X stands for D-cysteine
  MUTAGEN 17: note = X stands for D-glutamic acid
  MUTAGEN 19: note = X stands for D-lysine
XAXYXIXFXRXLXXXGXGX

SEQ ID NO: 145 - protein, 19 aa, synthetic construct
  MUTAGEN 1: note = X stands for 4-((carboxymethyl)amino)-butanoic acid
  MUTAGEN 5: note = X stands for (2S)-2-(methylamino)-3-phenyl-propanoic acid
  MUTAGEN 7: note = X stands for 2-(methylamino)-acetic acid
  MUTAGEN 9: note = X stands for (S)-4-(2-amino-2-carboxyethyl)-benzoic acid
  MUTAGEN 11: note = X stands for (2S)-2-(methylamino)-3-phenyl-propanoic acid
  MUTAGEN 13: note = X stands for (2S)-2-(methylamino)-propanoic acid
  MUTAGEN 14: note = X stands for (2S)-2-(methylamino)-3-phenyl-propanoic acid
  MUTAGEN 15: note = X stands for D-cysteine
  MUTAGEN 16: note = X stands for D-serine
  MUTAGEN 17: note = X stands for D-serine
  MUTAGEN 18: note = X stands for D-serine
  MUTAGEN 19: note = X stands for D-lysine
XAWYXIXYXRXLXXXXXXX

SEQ ID NO: 146 - protein, 19 aa, synthetic construct
  MUTAGEN 3: note = X stands for (S)-2-amino-3-(1H-pyrrolo[2,3-b]pyridin-3-yl)-propanoic acid
  MUTAGEN 5: note = X stands for (2S)-2-(methylamino)-3-phenyl-propanoic acid
  MUTAGEN 7: note = X stands for 2-(methylamino)-acetic acid
  MUTAGEN 9: note = X stands for (S)-4-(2-amino-2-carboxyethyl)-benzoic acid
  MUTAGEN 11: note = X stands for (2S)-2-(methylamino)-3-phenyl-propanoic acid
  MUTAGEN 13: note = X stands for (2S)-2-(methylamino)-propanoic acid
  MUTAGEN 14: note = X stands for (2S)-2-(methylamino)-3-phenyl-propanoic acid
  MUTAGEN 15: note = X stands for D-cysteine
  MUTAGEN 16: note = X stands for D-serine
  MUTAGEN 17: note = X stands for D-serine
  MUTAGEN 18: note = X stands for D-serine
  MUTAGEN 19: note = X stands for D-lysine
AAXYXIXFXRXLXXXXXXX

SEQ ID NO: 147 - protein, 19 aa, synthetic construct
  MUTAGEN 3: note = X stands for (S)-2-amino-3-(1H-pyrrolo[2,3-b]pyridin-3-yl)-propanoic acid
  MUTAGEN 5: note = X stands for (2S)-2-(methylamino)-3-phenyl-propanoic acid
  MUTAGEN 7: note = X stands for 2-(methylamino)-acetic acid
  MUTAGEN 8: note = X stands for (S)-2-amino-3-(pyridin-4-yl)-propanoic acid
  MUTAGEN 9: note = X stands for (S)-4-(2-amino-2-carboxyethyl)-benzoic acid
  MUTAGEN 11: note = X stands for (2S)-2-(methylamino)-3-phenyl-propanoic acid
  MUTAGEN 13: note = X stands for (2S)-2-(methylamino)-propanoic acid
  MUTAGEN 14: note = X stands for (2S)-2-(methylamino)-3-phenyl-propanoic acid
  MUTAGEN 15: note = X stands for D-cysteine
  MUTAGEN 16: note = X stands for D-serine
  MUTAGEN 17: note = X stands for D-serine
  MUTAGEN 18: note = X stands for D-serine
  MUTAGEN 19: note = X stands for D-lysine
AAXYXIXXXRXLXXXXXXX

SEQ ID NO: 148 - protein, 19 aa, synthetic construct
  MUTAGEN 1: note = X stands for 4-((carboxymethyl)amino)-butanoic acid
  MUTAGEN 3: note = X stands for (S)-2-amino-3-(1H-pyrrolo[2,3-b]pyridin-3-yl)-propanoic acid
  MUTAGEN 5: note = X stands for (2S)-2-(methylamino)-3-phenyl-propanoic acid
  MUTAGEN 7: note = X stands for 2-(methylamino)-acetic acid
  MUTAGEN 9: note = X stands for (S)-4-(2-amino-2-carboxyethyl)-benzoic acid
  MUTAGEN 11: note = X stands for (2S)-2-(methylamino)-3-phenyl-propanoic acid
  MUTAGEN 13: note = X stands for (2S)-2-(methylamino)-propanoic acid
  MUTAGEN 14: note = X stands for (2S)-2-(methylamino)-3-phenyl-propanoic acid
  MUTAGEN 15: note = X stands for D-cysteine
  MUTAGEN 16: note = X stands for D-serine
  MUTAGEN 17: note = X stands for D-serine
  MUTAGEN 18: note = X stands for D-serine
  MUTAGEN 19: note = X stands for D-lysine
XAXYXIXFXRXLXXXXXXX

SEQ ID NO: 149 - protein, 19 aa, synthetic construct
  MUTAGEN 1: note = X stands for 4-((carboxymethyl)amino)-butanoic acid
  MUTAGEN 3: note = X stands for (S)-2-amino-3-(1H-pyrrolo[2,3-b]pyridin-3-yl)-propanoic acid
  MUTAGEN 5: note = X stands for (2S)-2-(methylamino)-3-phenyl-propanoic acid
  MUTAGEN 7: note = X stands for 2-(methylamino)-acetic acid
  MUTAGEN 8: note = X stands for (S)-2-amino-3-(pyridin-4-yl)-propanoic acid
  MUTAGEN 9: note = X stands for (S)-4-(2-amino-2-carboxyethyl)-benzoic acid
  MUTAGEN 11: note = X stands for (2S)-2-(methylamino)-3-phenyl-propanoic acid
  MUTAGEN 13: note = X stands for (2S)-2-(methylamino)-propanoic acid
  MUTAGEN 14: note = X stands for (2S)-2-(methylamino)-3-phenyl-propanoic acid
  MUTAGEN 15: note = X stands for D-cysteine
  MUTAGEN 16: note = X stands for D-serine
  MUTAGEN 17: note = X stands for D-serine
  MUTAGEN 18: note = X stands for D-serine
  MUTAGEN 19: note = X stands for D-lysine
XAXYXIXXXRXLXXXXXXX

SEQ ID NO: 150 - protein, 19 aa, synthetic construct
  MUTAGEN 3: note = X stands for (S)-2-amino-3-(1H-pyrrolo[2,3-b]pyridin-3-yl)-propanoic acid
  MUTAGEN 5: note = X stands for (2S)-2-(methylamino)-3-phenyl-propanoic acid
  MUTAGEN 7: note = X stands for 2-(methylamino)-acetic acid
  MUTAGEN 9: note = X stands for (S)-4-(2-amino-2-carboxyethyl)-benzoic acid
  MUTAGEN 11: note = X stands for (2S)-2-(methylamino)-3-phenyl-propanoic acid
  MUTAGEN 13: note = X stands for (2S)-2-(methylamino)-propanoic acid
  MUTAGEN 14: note = X stands for (2S)-2-(methylamino)-3-phenyl-propanoic acid
  MUTAGEN 15: note = X stands for D-cysteine
  MUTAGEN 16: note = X stands for D-serine
  MUTAGEN 17: note = X stands for D-serine
  MUTAGEN 18: note = X stands for D-serine
  MUTAGEN 19: note = X stands for D-lysine
AEXYXIXFXRXLXXXXXXX

SEQ ID NO: 151 - protein, 19 aa, synthetic construct
  MUTAGEN 3: note = X stands for (S)-2-amino-3-(1H-pyrrolo[2,3-b]pyridin-3-yl)-propanoic acid
  MUTAGEN 5: note = X stands for (2S)-2-(methylamino)-3-phenyl-propanoic acid
  MUTAGEN 7: note = X stands for 2-(methylamino)-acetic acid
  MUTAGEN 8: note = X stands for (S)-2-amino-3-(pyridin-4-yl)-propanoic acid
  MUTAGEN 9: note = X stands for (S)-4-(2-amino-2-carboxyethyl)-benzoic acid
  MUTAGEN 11: note = X stands for (2S)-2-(methylamino)-3-phenyl-propanoic acid
  MUTAGEN 13: note = X stands for (2S)-2-(methylamino)-propanoic acid
  MUTAGEN 14: note = X stands for (2S)-2-(methylamino)-3-phenyl-propanoic acid
  MUTAGEN 15: note = X stands for D-cysteine
  MUTAGEN 16: note = X stands for D-serine
  MUTAGEN 17: note = X stands for D-serine
  MUTAGEN 18: note = X stands for D-serine
  MUTAGEN 19: note = X stands for D-lysine
AEXYXIXXXRXLXXXXXXX

SEQ ID NO: 152 - protein, 15 aa, synthetic construct
  MUTAGEN 1: note = X stands for 4-((carboxymethyl)amino)-butanoic acid
  MUTAGEN 3: note = X stands for (2S)-2-amino-3-[4-(pyridin-2-yl)phenyl]-propanoic acid
  MUTAGEN 4: note = X stands for (S)-2-amino-3-(4- phenoxyphenyl)-propanoic acid
  MUTAGEN 5: note = X stands for (2S)-2-(methylamino)-3-phenyl-propanoic acid
  MUTAGEN 7: note = X stands for 2-(methylamino)-acetic acid
  MUTAGEN 9: note = X stands for (S)-2-amino-3-(4-(carboxymethoxy)phenyl)-propanoic acid
  MUTAGEN 11: note = X stands for (2S)-2-(methylamino)-3-phenyl-propanoic acid
  MUTAGEN 13: note = X stands for (2S)-2-(methylamino)-propanoic acid
  MUTAGEN 14: note = X stands for (2S)-2-(methylamino)-3-phenyl-propanoic acid
  MUTAGEN 15: note = X stands for D-cysteine
XAXXXIXFXRXLXXX

SEQ ID NO: 153 - protein, 15 aa, synthetic construct
  MUTAGEN 1: note = X stands for 4-((carboxymethyl)amino)-butanoic acid
  MUTAGEN 3: note = X stands for (S)-3-([1,1'-biphenyl]-4-yl)-2-amino-propanoic acid
  MUTAGEN 5: note = X stands for (2S)-2-(methylamino)-3-phenyl-propanoic acid
  MUTAGEN 7: note = X stands for (2S)-2-(methylamino)-propanoic acid
  MUTAGEN 8: note = X stands for (S)-4-(2-amino-2-carboxyethyl)-benzoic acid
  MUTAGEN 9: note = X stands for (S)-2-amino-3-(4-carbamoylphenyl)-propanoic acid
  MUTAGEN 11: note = X stands for (2S)-2-(methylamino)-3-phenyl-propanoic acid
  MUTAGEN 13: note = X stands for (2S)-2-(methylamino)-propanoic acid
  MUTAGEN 14: note = X stands for (2S)-2-(methylamino)-3-phenyl-propanoic acid
  MUTAGEN 15: note = X stands for D-cysteine
XAXYXIXXXRXLXXX

SEQ ID NO: 154 - protein, 15 aa, synthetic construct
  MUTAGEN 1: note = X stands for 4-((carboxymethyl)amino)-butanoic acid
  MUTAGEN 3: note = X stands for (S)-3-([1,1'-biphenyl]-4-yl)-2-amino-propanoic acid
  MUTAGEN 5: note = X stands for (2S)-3-(4-hydroxyphenyl)-2-(methylamino)-propanoic acid
  MUTAGEN 7: note = X stands for 2-(methylamino)-acetic acid
  MUTAGEN 8: note = X stands for (S)-2-amino-3-(3-(carboxymethoxy)phenyl)-propanoic acid
  MUTAGEN 9: note = X stands for (S)-4-(2-amino-2-carboxyethyl)-benzoic acid
  MUTAGEN 11: note = X stands for (2S)-2-(methylamino)-3-phenyl-propanoic acid
  MUTAGEN 13: note = X stands for (2S)-2-(methylamino)-propanoic acid
  MUTAGEN 14: note = X stands for (S)-3-(3-ethylphenyl)-2-(methylamino)-propanoic acid
  MUTAGEN 15: note = X stands for D-cysteine
XAXYXIXXXRXLXXX

SEQ ID NO: 155 - protein, 15 aa, synthetic construct
  MUTAGEN 1: note = X stands for 4-((carboxymethyl)amino)-butanoic acid
  MUTAGEN 3: note = X stands for (S)-3-([1,1'-biphenyl]-4-yl)-2-amino-propanoic acid
  MUTAGEN 5: note = X stands for (S)-2-(methylamino)-3-(meta-tolyl)-propanoic acid
  MUTAGEN 7: note = X stands for 2-(methylamino)-acetic acid
  MUTAGEN 8: note = X stands for (S)-2-amino-3-(3-(carboxymethoxy)phenyl)-propanoic acid
  MUTAGEN 9: note = X stands for (S)-4-(2-amino-2-carboxyethyl)-benzoic acid
  MUTAGEN 11: note = X stands for (2S)-2-(methylamino)-3-phenyl-propanoic acid
  MUTAGEN 13: note = X stands for (2S)-2-(methylamino)-propanoic acid
  MUTAGEN 14: note = X stands for (2S)-2-(methylamino)-3-phenyl-propanoic acid
  MUTAGEN 15: note = X stands for D-cysteine
XAXYXIXXXRXLXXX

SEQ ID NO: 156 - protein, 15 aa, synthetic construct
  MUTAGEN 1: note = X stands for 4-((carboxymethyl)amino)-butanoic acid
  MUTAGEN 5: note = X stands for (2S)-2-(methylamino)-3-phenyl-propanoic acid
  MUTAGEN 7: note = X stands for (2S)-2-(methylamino)-propanoic acid
  MUTAGEN 8: note = X stands for (S)-2-amino-3-(3-methoxyphenyl)-propanoic acid
  MUTAGEN 9: note = X stands for (S)-2-amino-3-(4-(carboxymethoxy)phenyl)-propanoic acid
  MUTAGEN 11: note = X stands for (2S)-2-(methylamino)-3-phenyl-propanoic acid
  MUTAGEN 13: note = X stands for (2S)-2-(methylamino)-propanoic acid
  MUTAGEN 14: note = X stands for (2S)-2-(methylamino)-3-phenyl-propanoic acid
  MUTAGEN 15: note = X stands for D-cysteine
XAWYXIXXXRXLXXX

SEQ ID NO: 157 - protein, 15 aa, synthetic construct
  MUTAGEN 1: note = X stands for 4-((carboxymethyl)amino)-butanoic acid
  MUTAGEN 3: note = X stands for (S)-2-amino-3-(1H-pyrrolo[2,3-b]pyridin-3-yl)-propanoic acid
  MUTAGEN 5: note = X stands for (2S)-2-(methylamino)-3-phenyl-propanoic acid
  MUTAGEN 7: note = X stands for (2S)-2-(methylamino)-propanoic acid
  MUTAGEN 8: note = X stands for (S)-2-amino-3-(3-methoxyphenyl)-propanoic acid
  MUTAGEN 9: note = X stands for (S)-2-amino-3-(4-(carboxymethoxy)phenyl)-propanoic acid
  MUTAGEN 11: note = X stands for (2S)-2-(methylamino)-3-phenyl-propanoic acid
  MUTAGEN 13: note = X stands for (2S)-2-(methylamino)-propanoic acid
  MUTAGEN 14: note = X stands for (2S)-2-(methylamino)-3-phenyl-propanoic acid
  MUTAGEN 15: note = X stands for D-cysteine
XAXYXIXXXRXLXXX

SEQ ID NO: 158 - protein, 15 aa, synthetic construct
  MUTAGEN 5: note = X stands for (2S)-2-(methylamino)-3-phenyl-propanoic acid
  MUTAGEN 7: note = X stands for 2-(methylamino)-acetic acid
  MUTAGEN 8: note = X stands for (S)-2-amino-3-(3-(carboxymethoxy)phenyl)-propanoic acid
  MUTAGEN 9: note = X stands for (S)-2-amino-3-(pyridin-3-yl)-propanoic acid
  MUTAGEN 11: note = X stands for (2S)-2-(methylamino)-3-phenyl-propanoic acid
  MUTAGEN 12: note = X stands for (S)-2-amino-heptanoic acid
  MUTAGEN 13: note = X stands for (2S)-2-(methylamino)-propanoic acid
  MUTAGEN 14: note = X stands for (2S)-2-(methylamino)-3-phenyl-propanoic acid
  MUTAGEN 15: note = X stands for D-cysteine
AAWYXIXXXRXXXXX

SEQ ID NO: 159 - protein, 15 aa, synthetic construct
  MUTAGEN 5: note = X stands for (2S)-2-(methylamino)-3-phenyl-propanoic acid
  MUTAGEN 7: note = X stands for 2-(methylamino)-acetic acid
  MUTAGEN 8: note = X stands for (S)-2-amino-3-(3-(carboxymethoxy)phenyl)-propanoic acid
  MUTAGEN 9: note = X stands for (S)-4-(2-amino-2-carboxyethyl)-benzoic acid
  MUTAGEN 11: note = X stands for (2S)-2-(methylamino)-3-phenyl-propanoic acid
  MUTAGEN 12: note = X stands for (S)-2-amino-heptanoic acid
  MUTAGEN 13: note = X stands for (2S)-2-(methylamino)-propanoic acid
  MUTAGEN 14: note = X stands for (2S)-2-(methylamino)-3-phenyl-propanoic acid
  MUTAGEN 15: note = X stands for D-cysteine
AAWYXIXXXRXXXXX

SEQ ID NO: 160 - protein, 15 aa, synthetic construct
  MUTAGEN 3: note = X stands for (S)-2-amino-3-(1H-pyrrolo[2,3-c]pyridin-3-yl)-propanoic acid
  MUTAGEN 5: note = X stands for (2S)-2-(methylamino)-3-phenyl-propanoic acid
  MUTAGEN 7: note = X stands for 2-(methylamino)-acetic acid
  MUTAGEN 8: note = X stands for (S)-2-amino-3-(3-(carboxymethoxy)phenyl)-propanoic acid
  MUTAGEN 9: note = X stands for (S)-4-(2-amino-2-carboxyethyl)-benzoic acid
  MUTAGEN 11: note = X stands for (2S)-2-(methylamino)-3-phenyl-propanoic acid
  MUTAGEN 12: note = X stands for (S)-2-amino-nonanoic acid
  MUTAGEN 13: note = X stands for (2S)-2-(methylamino)-propanoic acid
  MUTAGEN 14: note = X stands for (2S)-2-(methylamino)-3-phenyl-propanoic acid
  MUTAGEN 15: note = X stands for D-cysteine
AAXYXIXXXRXXXXX

SEQ ID NO: 161 - protein, 15 aa, synthetic construct
  MUTAGEN 5: note = X stands for (2S)-2-(methylamino)-3-phenyl-propanoic acid
  MUTAGEN 7: note = X stands for 2-(methylamino)-acetic acid
  MUTAGEN 8: note = X stands for (S)-2-amino-3-(3-(carboxymethoxy)phenyl)-propanoic acid
  MUTAGEN 9: note = X stands for (S)-4-(2-amino-2-carboxyethyl)-benzoic acid
  MUTAGEN 11: note = X stands for (S)-2-(methylamino)-3-(pyridin-4-yl)-propanoic acid
  MUTAGEN 12: note = X stands for (S)-2-amino-nonanoic acid
  MUTAGEN 13: note = X stands for (2S)-2-(methylamino)-propanoic acid
  MUTAGEN 14: note = X stands for (2S)-2-(methylamino)-3-phenyl-propanoic acid
  MUTAGEN 15: note = X stands for D-cysteine
AAWYXIXXXRXXXXX

SEQ ID NO: 162 - protein, 15 aa, synthetic construct
  MUTAGEN 5: note = X stands for (2S)-2-(methylamino)-3-phenyl-propanoic acid
  MUTAGEN 7: note = X stands for 2-(methylamino)-acetic acid
  MUTAGEN 8: note = X stands for (S)-2-amino-3-(3-(carboxymethoxy)phenyl)-propanoic acid
  MUTAGEN 9: note = X stands for (S)-4-(2-amino-2-carboxyethyl)-benzoic acid
  MUTAGEN 11: note = X stands for (2S)-2-(methylamino)-3-phenyl-propanoic acid
  MUTAGEN 12: note = X stands for (S)-2-amino-nonanoic acid
  MUTAGEN 13: note = X stands for (2S)-2-(methylamino)-propanoic acid
  MUTAGEN 14: note = X stands for (S)-2-(methylamino)-3-(pyridin-4-yl)-propanoic acid
  MUTAGEN 15: note = X stands for D-cysteine
AAWYXIXXXRXXXXX

SEQ ID NO: 163 - protein, 15 aa, synthetic construct
  MUTAGEN 2: note = X stands for D-glutamic acid
  MUTAGEN 5: note = X stands for (2S)-2-(methylamino)-3-phenyl-propanoic acid
  MUTAGEN 7: note = X stands for 2-(methylamino)-acetic acid
  MUTAGEN 8: note = X stands for (S)-2-amino-3-(3-(carboxymethoxy)phenyl)-propanoic acid
  MUTAGEN 9: note = X stands for (S)-2-amino-3-(pyridin-4-yl)-propanoic acid
  MUTAGEN 11: note = X stands for (2S)-2-(methylamino)-3-phenyl-propanoic acid
  MUTAGEN 12: note = X stands for (S)-2-amino-nonanoic acid
  MUTAGEN 13: note = X stands for (2S)-2-(methylamino)-propanoic acid
  MUTAGEN 14: note = X stands for (2S)-2-(methylamino)-3-phenyl-propanoic acid
  MUTAGEN 15: note = X stands for D-cysteine
AXWYXIXXXRXXXXX

SEQ ID NO: 164 - protein, 16 aa, synthetic construct
  MUTAGEN 5: note = X stands for (2S)-2-(methylamino)-3-phenyl-propanoic acid
  MUTAGEN 7: note = X stands for 2-(methylamino)-acetic acid
  MUTAGEN 8: note = X stands for (S)-2-amino-3-(3-(carboxymethoxy)phenyl)-propanoic acid
  MUTAGEN 9: note = X stands for (S)-4-(2-amino-2-carboxyethyl)-benzoic acid
  MUTAGEN 11: note = X stands for (2S)-2-(methylamino)-3-phenyl-propanoic acid
  MUTAGEN 12: note = X stands for (S)-2-amino-nonanoic acid
  MUTAGEN 13: note = X stands for (2S)-2-(methylamino)-propanoic acid
  MUTAGEN 14: note = X stands for (2S)-2-(methylamino)-3-phenyl-propanoic acid
  MUTAGEN 16: note = X stands for 2-(piperazin-1-yl)-acetic acid
AAWYXIXXXRXXXXCX

SEQ ID NO: 165 - protein, 15 aa, synthetic construct
  MUTAGEN 1: note = X standards for 2,2'-imino-diacetic acid
  MUTAGEN 5: note = X stands for (2S)-2-(methylamino)-3-phenyl-propanoic acid
  MUTAGEN 7: note = X stands for 2-(methylamino)-acetic acid
  MUTAGEN 8: note = X stands for (S)-2-amino-3-(pyridin-4-yl)-propanoic acid
  MUTAGEN 9: note = X stands for (S)-4-(2-amino-2-carboxyethyl)-benzoic acid
  MUTAGEN 11: note = X stands for (2S)-2-(methylamino)-3-phenyl-propanoic acid
  MUTAGEN 12: note = X stands for (S)-2-amino-nonanoic acid
  MUTAGEN 13: note = X stands for (2S)-2-(methylamino)-propanoic acid
  MUTAGEN 14: note = X stands for (2S)-2-(methylamino)-3-phenyl-propanoic acid
  MUTAGEN 15: note = X stands for D-cysteine
XAWYXIXXXRXXXXX

SEQ ID NO: 166 - protein, 15 aa, synthetic construct
  MUTAGEN 1: note = X stands for 2-[(3-methoxypropyl)amino]-acetic acid
  MUTAGEN 5: note = X stands for (2S)-2-(methylamino)-3-phenyl-propanoic acid
  MUTAGEN 7: note = X stands for 2-(methylamino)-acetic acid
  MUTAGEN 8: note = X stands for (S)-2-amino-3-(pyridin-4-yl)-propanoic acid
  MUTAGEN 9: note = X stands for (S)-4-(2-amino-2-carboxyethyl)-benzoic acid
  MUTAGEN 11: note = X stands for (2S)-2-(methylamino)-3-phenyl-propanoic acid
  MUTAGEN 12: note = X stands for (S)-2-amino-nonanoic acid
  MUTAGEN 13: note = X stands for (2S)-2-(methylamino)-propanoic acid
  MUTAGEN 14: note = X stands for (2S)-2-(methylamino)-3-phenyl-propanoic acid
  MUTAGEN 15: note = X stands for D-cysteine
XAWYXIXXXRXXXXX

SEQ ID NO: 167 - protein, 15 aa, synthetic construct
  MUTAGEN 1: note = X standards for 2-[(2 -methoxyethyl)amino]-acetic acid
  MUTAGEN 5: note = X stands for (2S)-2-(methylamino)-3-phenyl-propanoic acid
  MUTAGEN 7: note = X stands for 2-(methylamino)-acetic acid
  MUTAGEN 8: note = X stands for (S)-2-amino-3-(pyridin-4-yl)-propanoic acid
  MUTAGEN 9: note = X stands for (S)-4-(2-amino-2-carboxyethyl)-benzoic acid
  MUTAGEN 11: note = X stands for (2S)-2-(methylamino)-3-phenyl-propanoic acid
  MUTAGEN 12: note = X stands for (S)-2-amino-nonanoic acid
  MUTAGEN 13: note = X stands for (2S)-2-(methylamino)-propanoic acid
  MUTAGEN 14: note = X stands for (2S)-2-(methylamino)-3-phenyl-propanoic acid
  MUTAGEN 15: note = X stands for D-cysteine
XAWYXIXXXRXXXXX

SEQ ID NO: 168 - protein, 15 aa, synthetic construct
  MUTAGEN 1: note = X standards for 2-[(3-acetamidopropyl)amino]-acetic acid
  MUTAGEN 5: note = X stands for (2S)-2-(methylamino)-3-phenyl-propanoic acid
  MUTAGEN 7: note = X stands for 2-(methylamino)-acetic acid
  MUTAGEN 8: note = X stands for (S)-2-amino-3-(pyridin-4-yl)-propanoic acid
  MUTAGEN 9: note = X stands for (S)-4-(2-amino-2-carboxyethyl)-benzoic acid
  MUTAGEN 11: note = X stands for (2S)-2-(methylamino)-3-phenyl-propanoic acid
  MUTAGEN 12: note = X stands for (S)-2-amino-nonanoic acid
  MUTAGEN 13: note = X stands for (2S)-2-(methylamino)-propanoic acid
  MUTAGEN 14: note = X stands for (2S)-2-(methylamino)-3-phenyl-propanoic acid
  MUTAGEN 15: note = X stands for D-cysteine
XAWYXIXXXRXXXXX

SEQ ID NO: 169 - protein, 15 aa, synthetic construct
  MUTAGEN 1: note = X stands for 4-((carboxymethyl)amino)-butanoic acid
  MUTAGEN 5: note = X stands for (2S)-2-(methylamino)-3-phenyl-propanoic acid
  MUTAGEN 7: note = X stands for 2-(methylamino)-acetic acid
  MUTAGEN 8: note = X stands for (S)-2-amino-3-(pyridin-4-yl)-propanoic acid
  MUTAGEN 9: note = X stands for (S)-4-(2-amino-2-carboxyethyl)-benzoic acid
  MUTAGEN 11: note = X stands for (2S)-2-(methylamino)-3-phenyl-propanoic acid
  MUTAGEN 12: note = X stands for (S)-2-amino-7-methoxy-heptanoic acid
  MUTAGEN 13: note = X stands for (2S)-2-(methylamino)-propanoic acid
  MUTAGEN 14: note = X stands for (2S)-2-(methylamino)-3-phenyl-propanoic acid
  MUTAGEN 15: note = X stands for D-cysteine
XAWYXIXXXRXXXXX

SEQ ID NO: 170 - protein, 15 aa, synthetic construct
  MUTAGEN 1: note = X stands for (S)-2-amino-3-(1-(carboxymethyl)piperidin-4-yl)-propanoic acid
  MUTAGEN 5: note = X stands for (2S)-2-(methylamino)-3-phenyl-propanoic acid
  MUTAGEN 7: note = X stands for 2-(methylamino)-acetic acid
  MUTAGEN 8: note = X stands for (S)-2-amino-3-(pyridin-4-yl)-propanoic acid
  MUTAGEN 9: note = X stands for (S)-4-(2-amino-2-carboxyethyl)-benzoic acid
  MUTAGEN 11: note = X stands for (2S)-2-(methylamino)-3-phenyl-propanoic acid
  MUTAGEN 12: note = X stands for (S)-2-amino-nonanoic acid
  MUTAGEN 13: note = X stands for (2S)-2-(methylamino)-propanoic acid
  MUTAGEN 14: note = X stands for (2S)-2-(methylamino)-3-phenyl-propanoic acid
  MUTAGEN 15: note = X stands for D-cysteine
XAWYXIXXXRXXXXX

SEQ ID NO: 171 - protein, 15 aa, synthetic construct
  MUTAGEN 1: note = X stands for 4-((carboxymethyl)amino)-butanoic acid
  MUTAGEN 5: note = X stands for (2S)-2-(methylamino)-3-phenyl-propanoic acid
  MUTAGEN 7: note = X stands for 2-(methylamino)-acetic acid
  MUTAGEN 8: note = X stands for (S)-2-amino-3-(1-(carboxymethyl)piperidin-4-yl)-propanoic acid
  MUTAGEN 9: note = X stands for (S)-4-(2-amino-2-carboxyethyl)-benzoic acid
  MUTAGEN 11: note = X stands for (2S)-2-(methylamino)-3-phenyl-propanoic acid
  MUTAGEN 12: note = X stands for (S)-2-amino-nonanoic acid
  MUTAGEN 13: note = X stands for (2S)-2-(methylamino)-propanoic acid
  MUTAGEN 14: note = X stands for (2S)-2-(methylamino)-3-phenyl-propanoic acid
  MUTAGEN 15: note = X stands for D-cysteine
XAWYXIXXXRXXXXX

SEQ ID NO: 172 - protein, 16 aa, synthetic construct
  MUTAGEN 1: note = X stands for 4-((carboxymethyl)amino)-butanoic acid
  MUTAGEN 5: note = X stands for (2S)-2-(methylamino)-3-phenyl-propanoic acid
  MUTAGEN 7: note = X stands for 2-(methylamino)-acetic acid
  MUTAGEN 8: note = X stands for (S)-2-amino-3-(pyridin-4-yl)-propanoic acid
  MUTAGEN 9: note = X stands for (S)-4-(2-amino-2-carboxyethyl)-benzoic acid
  MUTAGEN 11: note = X stands for (2S)-2-(methylamino)-3-phenyl-propanoic acid
  MUTAGEN 12: note = X stands for (S)-2-amino-nonanoic acid
  MUTAGEN 13: note = X stands for (2S)-2-(methylamino)-propanoic acid
  MUTAGEN 14: note = X stands for (2S)-2-(methylamino)-3-phenyl-propanoic acid
  MUTAGEN 15: note = X stands for D-cysteine
  MUTAGEN 16: note = X stands for (S)-2-amino-3-(1-(carboxymethyl)piperidin-4-yl)-propanoic acid
XAWYXIXXXRXXXXXX

SEQ ID NO: 173 - protein, 15 aa, synthetic construct
  MUTAGEN 1: note = X stands for (2S)-2-(methylamino)-propanoic acid
  MUTAGEN 5: note = X stands for (2S)-2-(methylamino)-3-phenyl-propanoic acid
  MUTAGEN 7: note = X stands for 2-(methylamino)-acetic acid
  MUTAGEN 8: note = X stands for (S)-2-amino-3-(3-(carboxymethoxy)phenyl)-propanoic acid
  MUTAGEN 9: note = X stands for (S)-4-(2-amino-2-carboxyethyl)-benzoic acid
  MUTAGEN 11: note = X stands for (2S)-2-(methylamino)-3-phenyl-propanoic acid
  MUTAGEN 12: note = X stands for (S)-2-amino-heptanoic acid
  MUTAGEN 13: note = X stands for (2S)-2-(methylamino)-propanoic acid
  MUTAGEN 14: note = X stands for (2S)-2-(methylamino)-3-phenyl-propanoic acid
  MUTAGEN 15: note = X stands for D-cysteine
XAWYXIXXXRXXXXX

SEQ ID NO: 174 - protein, 15 aa, synthetic construct
  MUTAGEN 1: note = X stands for 2-[(2-carbamoylethyl)amino]-acetic acid
  MUTAGEN 5: note = X stands for (2S)-2-(methylamino)-3-phenyl-propanoic acid
  MUTAGEN 7: note = X stands for 2-(methylamino)-acetic acid
  MUTAGEN 8: note = X stands for (S)-2-amino-3-(3-(carboxymethoxy)phenyl)-propanoic acid
  MUTAGEN 9: note = X stands for (S)-4-(2-amino-2-carboxyethyl)-benzoic acid
  MUTAGEN 11: note = X stands for (2S)-2-(methylamino)-3-phenyl-propanoic acid
  MUTAGEN 12: note = X stands for (S)-2-amino-heptanoic acid
  MUTAGEN 13: note = X stands for (2S)-2-(methylamino)-propanoic acid
  MUTAGEN 14: note = X stands for (2S)-2-(methylamino)-3-phenyl-propanoic acid
  MUTAGEN 15: note = X stands for D-cysteine
XAWYXIXXXRXXXXX

SEQ ID NO: 175 - protein, 16 aa, synthetic construct
  MUTAGEN 2: note = X stands for D-glutamic acid
  MUTAGEN 5: note = X stands for (S)-3-cyclohexyl-2-(methylamino)-propanoic acid
  MUTAGEN 7: note = X stands for D-proline
  MUTAGEN 8: note = X stands for (2S)-2-amino-6-{[4-(carboxymethyl)piperazine-1-carbonyl]amino} hexanoic acid
  MUTAGEN 9: note = X stands for (S)-4-(2-amino-2-carboxyethyl)-benzoic acid
  MUTAGEN 11: note = X stands for (S)-2-amino-3-cyclohexyl-propanoic acid
  MUTAGEN 12: note = X stands for (S)-2-amino-dodecanoic acid
  MUTAGEN 13: note = X stands for (2S)-2-(methylamino)-propanoic acid
  MUTAGEN 14: note = X stands for (2S)-2-(methylamino)-3-phenyl-propanoic acid
  MUTAGEN 15: note = X stands for D-cysteine
  MUTAGEN 16: note = X stands for 2-(piperazin-1-yl)-acetic acid
AXWYXIXXXRXXXXXX

SEQ ID NO: 176 - protein, 16 aa, synthetic construct
  MUTAGEN 2: note = X stands for D-glutamic acid
  MUTAGEN 3: note = X stands for (S)-2-amino-3-(4-(1-(2-(dimethylamino)-2-oxoethyl)-1H-pyrazole-4-yl)phenyl)-propanoic acid
  MUTAGEN 5: note = X stands for (S)-3-cyclohexyl-2-(methylamino)-propanoic acid
  MUTAGEN 7: note = X stands for D-proline
  MUTAGEN 8: note = X stands for (2S)-2-amino-6-{[4-(carboxymethyl)piperazine-1-carbonyl]amino} hexanoic acid
  MUTAGEN 9: note = X stands for (S)-4-(2-amino-2-carboxyethyl)-benzoic acid
  MUTAGEN 11: note = X stands for (S)-2-amino-3-cyclohexyl-propanoic acid
  MUTAGEN 12: note = X stands for (S)-2-amino-nonanoic acid
  MUTAGEN 13: note = X stands for (2S)-2-(methylamino)-propanoic acid
  MUTAGEN 14: note = X stands for (2S)-2-(methylamino)-3-phenyl-propanoic acid
  MUTAGEN 15: note = X stands for D-cysteine
  MUTAGEN 16: note = X stands for 2-(piperazin-1-yl)-acetic acid
AXXYXIXXXRXXXXXX

SEQ ID NO: 177 - protein, 16 aa, synthetic construct
  MUTAGEN 2: note = X stands for D-glutamic acid
  MUTAGEN 5: note = X stands for (S)-3-cyclohexyl-2-(methylamino)-propanoic acid
  MUTAGEN 7: note = X stands for 2-(ethylamino)-acetic acid
  MUTAGEN 8: note = X stands for (2S)-2-amino-6-{[4-(carboxymethyl)piperazine-1-carbonyl]amino} hexanoic acid
  MUTAGEN 9: note = X stands for (S)-4-(2-amino-2-carboxyethyl)-benzoic acid
  MUTAGEN 11: note = X stands for (2S)-2-(methylamino)-3-phenyl-propanoic acid
  MUTAGEN 12: note = X stands for (S)-2-amino-nonanoic acid
  MUTAGEN 13: note = X stands for (2S)-2-(methylamino)-propanoic acid
  MUTAGEN 14: note = X stands for (2S)-2-(methylamino)-3-phenyl-propanoic acid
  MUTAGEN 15: note = X stands for D-cysteine
  MUTAGEN 16: note = X stands for 2-(piperazin-1-yl)-acetic acid
AXWYXIXXXRXXXXXX

SEQ ID NO: 178 - protein, 16 aa, synthetic construct
  MUTAGEN 1: note = X stands for (2S)-2-amino-6-{[4-(carboxymethyl)piperazine-1-carbonyl]amino} hexanoic acid
  MUTAGEN 5: note = X stands for (2S)-2-(methylamino)-3-phenyl-propanoic acid
  MUTAGEN 7: note = X stands for 2-(methylamino)-acetic acid
  MUTAGEN 8: note = X stands for (S)-2-amino-3-(3-(carboxymethoxy)phenyl)-propanoic acid
  MUTAGEN 9: note = X stands for (S)-4-(2-amino-2-carboxyethyl)-benzoic acid
  MUTAGEN 11: note = X stands for (S)-2-amino-3-cyclohexyl-propanoic acid
  MUTAGEN 12: note = X stands for (S)-2-amino-dodecanoic acid
  MUTAGEN 13: note = X stands for (2S)-2-(methylamino)-propanoic acid
  MUTAGEN 14: note = X stands for (2S)-2-(methylamino)-3-phenyl-propanoic acid
  MUTAGEN 15: note = X stands for D-cysteine
  MUTAGEN 16: note = X stands for 2-(piperazin-1-yl)-acetic acid
XAWYXIXXXRXXXXXX

SEQ ID NO: 179 - protein, 16 aa, synthetic construct
  MUTAGEN 2: note = X stands for (2R)-2-amino-6-{[4-(carboxymethyl)piperazine-1-carbonyl]amino}-hexanoic acid
  MUTAGEN 5: note = X stands for (2S)-2-(methylamino)-3-phenyl-propanoic acid
  MUTAGEN 7: note = X stands for 2-(methylamino)-acetic acid
  MUTAGEN 8: note = X stands for (S)-2-amino-3-(3-(carboxymethoxy)phenyl)-propanoic acid
  MUTAGEN 9: note = X stands for (S)-4-(2-amino-2-carboxyethyl)-benzoic acid
  MUTAGEN 11: note = X stands for (S)-2-amino-3-cyclohexyl-propanoic acid
  MUTAGEN 12: note = X stands for (S)-2-amino-dodecanoic acid
  MUTAGEN 13: note = X stands for (2S)-2-(methylamino)-propanoic acid
  MUTAGEN 14: note = X stands for (2S)-2-(methylamino)-3-phenyl-propanoic acid
  MUTAGEN 15: note = X stands for D-cysteine
  MUTAGEN 16: note = X stands for 2-(piperazin-1-yl)-acetic acid
AXWYXIXXXRXXXXXX

SEQ ID NO: 180 - protein, 16 aa, synthetic construct
  MUTAGEN 5: note = X stands for (2S)-2-(methylamino)-3-phenyl-propanoic acid
  MUTAGEN 7: note = X stands for 2-(methylamino)-acetic acid
  MUTAGEN 8: note = X stands for (S)-2-amino-3-(3-(carboxymethoxy)phenyl)-propanoic acid
  MUTAGEN 9: note = X stands for (S)-4-(2-amino-2-carboxyethyl)-benzoic acid
  MUTAGEN 11: note = X stands for (S)-2-amino-3-cyclohexyl-propanoic acid
  MUTAGEN 12: note = X stands for (S)-2-amino-dodecanoic acid
  MUTAGEN 13: note = X stands for (2S)-6-{[4-(carboxymethyl)piperazine-1-carbonyl]amino}-2-(methylamino)-hexanoic acid
  MUTAGEN 14: note = X stands for (2S)-2-(methylamino)-3-phenyl-propanoic acid
  MUTAGEN 15: note = X stands for D-cysteine
  MUTAGEN 16: note = X stands for 2-(piperazin-1-yl)-acetic acid
AAWYXIXXXRXXXXXX

SEQ ID NO: 181 - protein, 16 aa, synthetic construct
  MUTAGEN 1: note = X stands for (2S)-2-amino-6-{[4-(carboxymethyl)piperazine-1-carbonyl]amino} hexanoic acid
  MUTAGEN 5: note = X stands for (2S)-2-(methylamino)-3-phenyl-propanoic acid
  MUTAGEN 7: note = X stands for 2-(methylamino)-acetic acid
  MUTAGEN 8: note = X stands for (S)-2-amino-3-(3-(carboxymethoxy)phenyl)-propanoic acid
  MUTAGEN 9: note = X stands for (S)-4-(2-amino-2-carboxyethyl)-benzoic acid
  MUTAGEN 11: note = X stands for (2S)-2-(methylamino)-3-phenyl-propanoic acid
  MUTAGEN 12: note = X stands for (S)-2-amino-dodecanoic acid
  MUTAGEN 13: note = X stands for (2S)-2-(methylamino)-propanoic acid
  MUTAGEN 14: note = X stands for (2S)-2-(methylamino)-3-phenyl-propanoic acid
  MUTAGEN 15: note = X stands for D-cysteine
  MUTAGEN 16: note = X stands for 2-(piperazin-1-yl)-acetic acid
XAWYXIXXXRXXXXXX

SEQ ID NO: 182 - protein, 16 aa, synthetic construct
  MUTAGEN 2: note = X stands for (2R)-2-amino-6-{[4-(carboxymethyl)piperazine-1-carbonyl]amino}-hexanoic acid
  MUTAGEN 5: note = X stands for (2S)-2-(methylamino)-3-phenyl-propanoic acid
  MUTAGEN 7: note = X stands for 2-(methylamino)-acetic acid
  MUTAGEN 8: note = X stands for (S)-2-amino-3-(3-(carboxymethoxy)phenyl)-propanoic acid
  MUTAGEN 9: note = X stands for (S)-4-(2-amino-2-carboxyethyl)-benzoic acid
  MUTAGEN 11: note = X stands for (2S)-2-(methylamino)-3-phenyl-propanoic acid
  MUTAGEN 12: note = X stands for (S)-2-amino-dodecanoic acid
  MUTAGEN 13: note = X stands for (2S)-2-(methylamino)-propanoic acid
  MUTAGEN 14: note = X stands for (2S)-2-(methylamino)-3-phenyl-propanoic acid
  MUTAGEN 15: note = X stands for D-cysteine
  MUTAGEN 16: note = X stands for 2-(piperazin-1-yl)-acetic acid
AXWYXIXXXRXXXXXX

SEQ ID NO: 183 - protein, 16 aa, synthetic construct
  MUTAGEN 1: note = X stands for (2S)-2-amino-6-{[4-(carboxymethyl)piperazine-1-carbonyl]amino} hexanoic acid
  MUTAGEN 5: note = X stands for (2S)-2-(methylamino)-3-phenyl-propanoic acid
  MUTAGEN 7: note = X stands for 2-(methylamino)-acetic acid
  MUTAGEN 8: note = X stands for (2S)-2-amino-6-{[4-(carboxymethyl)piperazine-1-carbonyl]amino} hexanoic acid
  MUTAGEN 9: note = X stands for (S)-4-(2-amino-2-carboxyethyl)-benzoic acid
  MUTAGEN 11: note = X stands for (S)-2-amino-3-cyclohexyl-propanoic acid
  MUTAGEN 12: note = X stands for (S)-2-amino-dodecanoic acid
  MUTAGEN 13: note = X stands for (2S)-2-(methylamino)-propanoic acid
  MUTAGEN 14: note = X stands for (2S)-2-(methylamino)-3-phenyl-propanoic acid
  MUTAGEN 15: note = X stands for D-cysteine
  MUTAGEN 16: note = X stands for 2-(piperazin-1-yl)-acetic acid
XAWYXIXXXRXXXXXX

SEQ ID NO: 184 - protein, 16 aa, synthetic construct
  MUTAGEN 2: note = X stands for (2R)-2-amino-6-{[4-(carboxymethyl)piperazine-1-carbonyl]amino}-hexanoic acid
  MUTAGEN 5: note = X stands for (2S)-2-(methylamino)-3-phenyl-propanoic acid
  MUTAGEN 7: note = X stands for 2-(methylamino)-acetic acid
  MUTAGEN 8: note = X stands for (2S)-2-amino-6-{[4-(carboxymethyl)piperazine-1-carbonyl]amino} hexanoic acid
  MUTAGEN 9: note = X stands for (S)-4-(2-amino-2-carboxyethyl)-benzoic acid
  MUTAGEN 11: note = X stands for (S)-2-amino-3-cyclohexyl-propanoic acid
  MUTAGEN 12: note = X stands for (S)-2-amino-dodecanoic acid
  MUTAGEN 13: note = X stands for (2S)-2-(methylamino)-propanoic acid
  MUTAGEN 14: note = X stands for (2S)-2-(methylamino)-3-phenyl-propanoic acid
  MUTAGEN 15: note = X stands for D-cysteine
  MUTAGEN 16: note = X stands for 2-(piperazin-1-yl)-acetic acid
AXWYXIXXXRXXXXXX

SEQ ID NO: 185 - protein, 16 aa, synthetic construct
  MUTAGEN 5: note = X stands for (2S)-2-(methylamino)-3-phenyl-propanoic acid
  MUTAGEN 7: note = X stands for 2-(methylamino)-acetic acid
  MUTAGEN 8: note = X stands for (2S)-2-amino-6-{[4-(carboxymethyl)piperazine-1-carbonyl]amino} hexanoic acid
  MUTAGEN 9: note = X stands for (S)-4-(2-amino-2-carboxyethyl)-benzoic acid
  MUTAGEN 11: note = X stands for (S)-2-amino-3-cyclohexyl-propanoic acid
  MUTAGEN 12: note = X stands for (S)-2-amino-dodecanoic acid
  MUTAGEN 13: note = X stands for (2S)-2-(methylamino)-pentanedioic acid
  MUTAGEN 14: note = X stands for (2S)-2-(methylamino)-3-phenyl-propanoic acid
  MUTAGEN 15: note = X stands for D-cysteine
  MUTAGEN 16: note = X stands for 2-(piperazin-1-yl)-acetic acid
AAWYXIXXXRXXXXXX

SEQ ID NO: 186 - protein, 16 aa, synthetic construct
  MUTAGEN 5: note = X stands for (2S)-2-(methylamino)-3-phenyl-propanoic acid
  MUTAGEN 7: note = X stands for 2-(methylamino)-acetic acid
  MUTAGEN 8: note = X stands for (2S)-2-amino-6-{[4-(carboxymethyl)piperazine-1-carbonyl]amino} hexanoic acid
  MUTAGEN 9: note = X stands for (S)-4-(2-amino-2-carboxyethyl)-benzoic acid
  MUTAGEN 11: note = X stands for (S)-2-amino-3-cyclohexyl-propanoic acid
  MUTAGEN 12: note = X stands for (S)-2-amino-dodecanoic acid
  MUTAGEN 13: note = X stands for (2S)-6-{[4-(carboxymethyl)piperazine-1-carbonyl]amino}-2-(methylamino)-hexanoic acid
  MUTAGEN 14: note = X stands for (2S)-2-(methylamino)-3-phenyl-propanoic acid
  MUTAGEN 15: note = X stands for D-cysteine
  MUTAGEN 16: note = X stands for 2-(piperazin-1-yl)-acetic acid
AAWYXIXXXRXXXXXX

SEQ ID NO: 187 - protein, 16 aa, synthetic construct
  MUTAGEN 5: note = X stands for (2S)-2-(methylamino)-3-phenyl-propanoic acid
  MUTAGEN 7: note = X stands for 2-(methylamino)-acetic acid
  MUTAGEN 8: note = X stands for (S)-2-amino-3-(3-(carboxymethoxy)phenyl)-propanoic acid
  MUTAGEN 9: note = X stands for (S)-4-(2-amino-2-carboxyethyl)-benzoic acid
  MUTAGEN 11: note = X stands for (2S)-2-(methylamino)-3-phenyl-propanoic acid
  MUTAGEN 12: note = X stands for (S)-2-amino-nonanoic acid
  MUTAGEN 13: note = X stands for (2S)-2-(methylamino)-propanoic acid
  MUTAGEN 14: note = X stands for (2S)-2-(methylamino)-3-phenyl-propanoic acid
  MUTAGEN 15: note = X stands for D-cysteine
  MUTAGEN 16: note = X stands for 2-(piperazin-1-yl)-acetic acid
KAWYXIXXXRXXXXXX

SEQ ID NO: 188 - protein, 16 aa, synthetic construct
  MUTAGEN 5: note = X stands for (2S)-2-(methylamino)-3-phenyl-propanoic acid
  MUTAGEN 7: note = X stands for 2-(methylamino)-acetic acid
  MUTAGEN 8: note = X stands for (S)-2-amino-3-(3-(carboxymethoxy)phenyl)-propanoic acid
  MUTAGEN 9: note = X stands for (S)-4-(2-amino-2-carboxyethyl)-benzoic acid
  MUTAGEN 11: note = X stands for (2S)-2-(methylamino)-3-phenyl-propanoic acid
  MUTAGEN 12: note = X stands for (S)-2-amino-nonanoic acid
  MUTAGEN 13: note = X stands for (2S)-6-amino-2-(methylamino)-hexanoic acid
  MUTAGEN 14: note = X stands for (2S)-2-(methylamino)-3-phenyl-propanoic acid
  MUTAGEN 15: note = X stands for D-cysteine
  MUTAGEN 16: note = X stands for 2-(piperazin-1-yl)-acetic acid
AAWYXIXXXRXXXXXX

SEQ ID NO: 189 - protein, 16 aa, synthetic construct
  MUTAGEN 5: note = X stands for (2S)-2-(methylamino)-3-phenyl-propanoic acid
  MUTAGEN 7: note = X stands for 2-(methylamino)-acetic acid
  MUTAGEN 9: note = X stands for (S)-4-(2-amino-2-carboxyethyl)-benzoic acid
  MUTAGEN 11: note = X stands for (2S)-2-(methylamino)-3-phenyl-propanoic acid
  MUTAGEN 12: note = X stands for (S)-2-amino-nonanoic acid
  MUTAGEN 13: note = X stands for (2S)-2-(methylamino)-propanoic acid
  MUTAGEN 14: note = X stands for (2S)-2-(methylamino)-3-phenyl-propanoic acid
  MUTAGEN 15: note = X stands for D-cysteine
  MUTAGEN 16: note = X stands for 2-(piperazin-1-yl)-acetic acid
AAWYXIXXXRXXXXXX

SEQ ID NO: 190 - protein, 16 aa, synthetic construct
  MUTAGEN 5: note = X stands for (2S)-2-(methylamino)-3-phenyl-propanoic acid
  MUTAGEN 7: note = X stands for 2-(methylamino)-acetic acid
  MUTAGEN 8: note = X stands for (S)-2-amino-3-(3-(carboxymethoxy)phenyl)-propanoic acid
  MUTAGEN 9: note = X stands for (S)-4-(2-amino-2-carboxyethyl)-benzoic acid
  MUTAGEN 11: note = X stands for (2S)-2-(methylamino)-3-phenyl-propanoic acid
  MUTAGEN 12: note = X stands for (S)-2-amino-nonanoic acid
  MUTAGEN 13: note = X stands for (2S)-2-(methylamino)-propanoic acid
  MUTAGEN 14: note = X stands for (2S)-2-(methylamino)-3-phenyl-propanoic acid
  MUTAGEN 15: note = X stands for D-cysteine
  MUTAGEN 16: note = X stands for 2-(piperazin-1-yl)-acetic acid
KAWYXIXXXRXXXXXX

SEQ ID NO: 191 - protein, 16 aa, synthetic construct
  MUTAGEN 5: note = X stands for (2S)-2-(methylamino)-3-phenyl-propanoic acid
  MUTAGEN 7: note = X stands for 2-(methylamino)-acetic acid
  MUTAGEN 8: note = X stands for (S)-2-amino-3-(3-(carboxymethoxy)phenyl)-propanoic acid
  MUTAGEN 9: note = X stands for (S)-4-(2-amino-2-carboxyethyl)-benzoic acid
  MUTAGEN 11: note = X stands for (2S)-2-(methylamino)-3-phenyl-propanoic acid
  MUTAGEN 12: note = X stands for (S)-2-amino-nonanoic acid
  MUTAGEN 13: note = X stands for (2S)-6-amino-2-(methylamino)-hexanoic acid
  MUTAGEN 14: note = X stands for (2S)-2-(methylamino)-3-phenyl-propanoic acid
  MUTAGEN 15: note = X stands for D-cysteine
  MUTAGEN 16: note = X stands for 2-(piperazin-1-yl)-acetic acid
AAWYXIXXXRXXXXXX

SEQ ID NO: 192 - protein, 16 aa, synthetic construct
  MUTAGEN 4: note = X stands for (S)-2-amino-3-(4-(2-aminoethoxy)phenyl)-propanoic acid
  MUTAGEN 5: note = X stands for (2S)-2-(methylamino)-3-phenyl-propanoic acid
  MUTAGEN 7: note = X stands for 2-(methylamino)-acetic acid
  MUTAGEN 8: note = X stands for (S)-2-amino-3-(3-(carboxymethoxy)phenyl)-propanoic acid
  MUTAGEN 9: note = X stands for (S)-4-(2-amino-2-carboxyethyl)-benzoic acid
  MUTAGEN 11: note = X stands for (2S)-2-(methylamino)-3-phenyl-propanoic acid
  MUTAGEN 12: note = X stands for (S)-2-amino-nonanoic acid
  MUTAGEN 13: note = X stands for (2S)-2-(methylamino)-propanoic acid
  MUTAGEN 14: note = X stands for (2S)-2-(methylamino)-3-phenyl-propanoic acid
  MUTAGEN 15: note = X stands for D-cysteine
  MUTAGEN 16: note = X stands for 2-(piperazin-1-yl)-acetic acid
AAWXXIXXXRXXXXXX

SEQ ID NO: 193 - protein, 16 aa, synthetic construct
  MUTAGEN 4: note = X stands for (S)-2-amino-3-(naphthalene-1-yl)-propanoic acid
  MUTAGEN 5: note = X stands for (2S)-2-(methylamino)-3-phenyl-propanoic acid
  MUTAGEN 7: note = X stands for 2-(methylamino)-acetic acid
  MUTAGEN 8: note = X stands for (S)-2-amino-3-(3-(carboxymethoxy)phenyl)-propanoic acid
  MUTAGEN 9: note = X stands for (S)-4-(2-amino-2-carboxyethyl)-benzoic acid
  MUTAGEN 11: note = X stands for (2S)-2-(methylamino)-3-phenyl-propanoic acid
  MUTAGEN 12: note = X stands for (S)-2-amino-nonanoic acid
  MUTAGEN 13: note = X stands for (2S)-2-(methylamino)-propanoic acid
  MUTAGEN 14: note = X stands for (2S)-2-(methylamino)-3-phenyl-propanoic acid
  MUTAGEN 15: note = X stands for D-cysteine
  MUTAGEN 16: note = X stands for 2-(piperazin-1-yl)-acetic acid
AAWXXIXXXRXXXXXX

SEQ ID NO: 194 - protein, 16 aa, synthetic construct
  MUTAGEN 4: note = X stands for (S)-3-([1,1'-biphenyl]-3-yl)-2-amino-propanoic acid
  MUTAGEN 5: note = X stands for (2S)-2-(methylamino)-3-phenyl-propanoic acid
  MUTAGEN 7: note = X stands for 2-(methylamino)-acetic acid
  MUTAGEN 8: note = X stands for (S)-2-amino-3-(3-(carboxymethoxy)phenyl)-propanoic acid
  MUTAGEN 9: note = X stands for (S)-4-(2-amino-2-carboxyethyl)-benzoic acid
  MUTAGEN 11: note = X stands for (2S)-2-(methylamino)-3-phenyl-propanoic acid
  MUTAGEN 12: note = X stands for (S)-2-amino-nonanoic acid
  MUTAGEN 13: note = X stands for (2S)-2-(methylamino)-propanoic acid
  MUTAGEN 14: note = X stands for (2S)-2-(methylamino)-3-phenyl-propanoic acid
  MUTAGEN 15: note = X stands for D-cysteine
  MUTAGEN 16: note = X stands for 2-(piperazin-1-yl)-acetic acid
AAWXXIXXXRXXXXXX

SEQ ID NO: 195 - protein, 16 aa, synthetic construct
  MUTAGEN 5: note = X stands for (S)-3-(4-(3-Aminopropoxy)phenyl)-2-(methylamino)-propanoic acid
  MUTAGEN 7: note = X stands for 2-(methylamino)-acetic acid
  MUTAGEN 8: note = X stands for (S)-2-amino-3-(3-(carboxymethoxy)phenyl)-propanoic acid
  MUTAGEN 9: note = X stands for (S)-4-(2-amino-2-carboxyethyl)-benzoic acid
  MUTAGEN 11: note = X stands for (2S)-2-(methylamino)-3-phenyl-propanoic acid
  MUTAGEN 12: note = X stands for (S)-2-amino-nonanoic acid
  MUTAGEN 13: note = X stands for (2S)-2-(methylamino)-propanoic acid
  MUTAGEN 14: note = X stands for (2S)-2-(methylamino)-3-phenyl-propanoic acid
  MUTAGEN 15: note = X stands for D-cysteine
  MUTAGEN 16: note = X stands for 2-(piperazin-1-yl)-acetic acid
AAWYXIXXXRXXXXXX

SEQ ID NO: 196 - protein, 16 aa, synthetic construct
  MUTAGEN 5: note = X stands for (S)-3-(1-acetylpiperidin-4-yl)-2-(methylamino)-propanoic acid
  MUTAGEN 7: note = X stands for 2-(methylamino)-acetic acid
  MUTAGEN 8: note = X stands for (S)-2-amino-3-(3-(carboxymethoxy)phenyl)-propanoic acid
  MUTAGEN 9: note = X stands for (S)-4-(2-amino-2-carboxyethyl)-benzoic acid
  MUTAGEN 11: note = X stands for (2S)-2-(methylamino)-3-phenyl-propanoic acid
  MUTAGEN 12: note = X stands for (S)-2-amino-nonanoic acid
  MUTAGEN 13: note = X stands for (2S)-2-(methylamino)-propanoic acid
  MUTAGEN 14: note = X stands for (2S)-2-(methylamino)-3-phenyl-propanoic acid
  MUTAGEN 15: note = X stands for D-cysteine
  MUTAGEN 16: note = X stands for 2-(piperazin-1-yl)-acetic acid
AAWYXIXXXRXXXXXX

SEQ ID NO: 197 - protein, 16 aa, synthetic construct
  MUTAGEN 5: note = X stands for (S)-3-([1,1'-biphenyl]-3-yl)-2-(methylamino)-propanoic acid
  MUTAGEN 7: note = X stands for 2-(methylamino)-acetic acid
  MUTAGEN 8: note = X stands for (S)-2-amino-3-(3-(carboxymethoxy)phenyl)-propanoic acid
  MUTAGEN 9: note = X stands for (S)-4-(2-amino-2-carboxyethyl)-benzoic acid
  MUTAGEN 11: note = X stands for (2S)-2-(methylamino)-3-phenyl-propanoic acid
  MUTAGEN 12: note = X stands for (S)-2-amino-nonanoic acid
  MUTAGEN 13: note = X stands for (2S)-2-(methylamino)-propanoic acid
  MUTAGEN 14: note = X stands for (2S)-2-(methylamino)-3-phenyl-propanoic acid
  MUTAGEN 15: note = X stands for D-cysteine
  MUTAGEN 16: note = X stands for 2-(piperazin-1-yl)-acetic acid
AAWYXIXXXRXXXXXX

SEQ ID NO: 198 - protein, 16 aa, synthetic construct
  MUTAGEN 5: note = X stands for (S)-2-(methylamino)-3-(naphthalene-1-yl)-propanoic acid
  MUTAGEN 7: note = X stands for 2-(methylamino)-acetic acid
  MUTAGEN 8: note = X stands for (S)-2-amino-3-(3-(carboxymethoxy)phenyl)-propanoic acid
  MUTAGEN 9: note = X stands for (S)-4-(2-amino-2-carboxyethyl)-benzoic acid
  MUTAGEN 11: note = X stands for (2S)-2-(methylamino)-3-phenyl-propanoic acid
  MUTAGEN 12: note = X stands for (S)-2-amino-nonanoic acid
  MUTAGEN 13: note = X stands for (2S)-2-(methylamino)-propanoic acid
  MUTAGEN 14: note = X stands for (2S)-2-(methylamino)-3-phenyl-propanoic acid
  MUTAGEN 15: note = X stands for D-cysteine
  MUTAGEN 16: note = X stands for 2-(piperazin-1-yl)-acetic acid
AAWYXIXXXRXXXXXX

SEQ ID NO: 199 - protein, 16 aa, synthetic construct
  MUTAGEN 5: note = X stands for (S)-2-(methylamino)-3-(naphthalene-2-yl)-propanoic acid
  MUTAGEN 7: note = X stands for 2-(methylamino)-acetic acid
  MUTAGEN 8: note = X stands for (S)-2-amino-3-(3-(carboxymethoxy)phenyl)-propanoic acid
  MUTAGEN 9: note = X stands for (S)-4-(2-amino-2-carboxyethyl)-benzoic acid
  MUTAGEN 11: note = X stands for (2S)-2-(methylamino)-3-phenyl-propanoic acid
  MUTAGEN 12: note = X stands for (S)-2-amino-nonanoic acid
  MUTAGEN 13: note = X stands for (2S)-2-(methylamino)-propanoic acid
  MUTAGEN 14: note = X stands for (2S)-2-(methylamino)-3-phenyl-propanoic acid
  MUTAGEN 15: note = X stands for D-cysteine
  MUTAGEN 16: note = X stands for 2-(piperazin-1-yl)-acetic acid
AAWYXIXXXRXXXXXX

SEQ ID NO: 200 - protein, 16 aa, synthetic construct
  ACT_SITE 5: note = X stands for (S)-3-(4-methoxyphenyl)-2-(methylamino)-propanoic acid
  MUTAGEN 7: note = X stands for 2-(methylamino)-acetic acid
  MUTAGEN 8: note = X stands for (S)-2-amino-3-(3-(carboxymethoxy)phenyl)-propanoic acid
  MUTAGEN 9: note = X stands for (S)-4-(2-amino-2-carboxyethyl)-benzoic acid
  MUTAGEN 11: note = X stands for (2S)-2-(methylamino)-3-phenyl-propanoic acid
  MUTAGEN 12: note = X stands for (S)-2-amino-nonanoic acid
  MUTAGEN 13: note = X stands for (2S)-2-(methylamino)-propanoic acid
  MUTAGEN 14: note = X stands for (2S)-2-(methylamino)-3-phenyl-propanoic acid
  MUTAGEN 15: note = X stands for D-cysteine
  MUTAGEN 16: note = X stands for 2-(piperazin-1-yl)-acetic acid
AAWYXIXXXRXXXXXX

SEQ ID NO: 201 - protein, 16 aa, synthetic construct
  MUTAGEN 5: note = X stands for (S)-3-(4-chlorophenyl)-2-(methylamino)-propanoic acid
  MUTAGEN 7: note = X stands for 2-(methylamino)-acetic acid
  MUTAGEN 8: note = X stands for (S)-2-amino-3-(3-(carboxymethoxy)phenyl)-propanoic acid
  MUTAGEN 9: note = X stands for (S)-4-(2-amino-2-carboxyethyl)-benzoic acid
  MUTAGEN 11: note = X stands for (2S)-2-(methylamino)-3-phenyl-propanoic acid
  MUTAGEN 12: note = X stands for (S)-2-amino-nonanoic acid
  MUTAGEN 13: note = X stands for (2S)-2-(methylamino)-propanoic acid
  MUTAGEN 14: note = X stands for (2S)-2-(methylamino)-3-phenyl-propanoic acid
  MUTAGEN 15: note = X stands for D-cysteine
  MUTAGEN 16: note = X stands for 2-(piperazin-1-yl)-acetic acid
AAWYXIXXXRXXXXXX

SEQ ID NO: 202 - protein, 16 aa, synthetic construct
  MUTAGEN 5: note = X stands for (2S)-2-(methylamino)-3-phenyl-propanoic acid
  MUTAGEN 7: note = X stands for 2-(methylamino)-acetic acid
  MUTAGEN 8: note = X stands for (S)-2-amino-3-(3-(carboxymethoxy)phenyl)-propanoic acid
  MUTAGEN 9: note = X stands for (S)-4-(2-amino-2-carboxyethyl)-benzoic acid
  MUTAGEN 11: note = X stands for (2S)-2-(methylamino)-3-phenyl-propanoic acid
  MUTAGEN 12: note = X stands for (S)-2-amino-nonanoic acid
  MUTAGEN 13: note = X stands for (2S)-2-(methylamino)-pentanedioic acid
  MUTAGEN 14: note = X stands for (2S)-2-(methylamino)-3-phenyl-propanoic acid
  MUTAGEN 15: note = X stands for D-cysteine
  MUTAGEN 16: note = X stands for 2-(piperazin-1-yl)-acetic acid
AAWYXIXXXRXXXXXX

SEQ ID NO: 203 - protein, 16 aa, synthetic construct
  MUTAGEN 3: note = X stands for (2S)-2-amino-3-(1-benzyl-1H-indol-3-yl)-propanoic acid
  MUTAGEN 5: note = X stands for (2S)-2-(methylamino)-3-phenyl-propanoic acid
  MUTAGEN 7: note = X stands for 2-(methylamino)-acetic acid
  MUTAGEN 8: note = X stands for (S)-2-amino-3-(3-(carboxymethoxy)phenyl)-propanoic acid
  MUTAGEN 9: note = X stands for (S)-4-(2-amino-2-carboxyethyl)-benzoic acid
  MUTAGEN 11: note = X stands for (2S)-2-(methylamino)-3-phenyl-propanoic acid
  MUTAGEN 12: note = X stands for (S)-2-amino-nonanoic acid
  MUTAGEN 13: note = X stands for (2S)-2-(methylamino)-propanoic acid
  MUTAGEN 14: note = X stands for (2S)-2-(methylamino)-3-phenyl-propanoic acid
  MUTAGEN 15: note = X stands for D-cysteine
  MUTAGEN 16: note = X stands for 2-(piperazin-1-yl)-acetic acid
AAXYXIXXXRXXXXXX

SEQ ID NO: 204 - protein, 16 aa, synthetic construct
  MUTAGEN 5: note = X stands for (2S)-2-(methylamino)-3-phenyl-propanoic acid
  MUTAGEN 7: note = X stands for 2-(methylamino)-acetic acid
  MUTAGEN 8: note = X stands for (S)-2-amino-3-(3-(carboxymethoxy)phenyl)-propanoic acid
  MUTAGEN 9: note = X stands for (S)-4-(2-amino-2-carboxyethyl)-benzoic acid
  MUTAGEN 11: note = X stands for (2S)-2-(methylamino)-3-phenyl-propanoic acid
  MUTAGEN 12: note = X stands for (S)-2-amino-nonanoic acid
  MUTAGEN 13: note = X stands for (2S)-2-(methylamino)-propanoic acid
  MUTAGEN 14: note = X stands for (2S)-2-(methylamino)-3-phenyl-propanoic acid
  MUTAGEN 15: note = X stands for D-cysteine
  MUTAGEN 16: note = X stands for 2-(piperidine-4-yl)-acetic acid
AAWYXIXXXRXXXXXX

SEQ ID NO: 205 - protein, 16 aa, synthetic construct
  MUTAGEN 5: note = X stands for (2S)-2-(methylamino)-3-phenyl-propanoic acid
  MUTAGEN 7: note = X stands for 2-(methylamino)-acetic acid
  MUTAGEN 8: note = X stands for (S)-2-amino-3-(3-(carboxymethoxy)phenyl)-propanoic acid
  MUTAGEN 9: note = X stands for (S)-4-(2-amino-2-carboxyethyl)-benzoic acid
  MUTAGEN 11: note = X stands for (2S)-2-(methylamino)-3-phenyl-propanoic acid
  MUTAGEN 12: note = X stands for (S)-2-amino-nonanoic acid
  MUTAGEN 13: note = X stands for (2S)-2-(methylamino)-propanoic acid
  MUTAGEN 14: note = X stands for (2S)-2-(methylamino)-3-phenyl-propanoic acid
  MUTAGEN 15: note = X stands for D-cysteine
  MUTAGEN 16: note = X stands for 3-(piperidine-4-yl)-propanoic acid
AAWYXIXXXRXXXXXX

SEQ ID NO: 206 - protein, 15 aa, synthetic construct
  MUTAGEN 1: note = X stands for 4-((carboxymethyl)amino)-butanoic acid
  MUTAGEN 3: note = X stands for (S)-2-amino-3-(6-hydroxy-1H-indol-3-yl)-propanoic acid
  MUTAGEN 5: note = X stands for (2S)-2-(methylamino)-3-phenyl-propanoic acid
  MUTAGEN 7: note = X stands for (2S)-2-(methylamino)-propanoic acid
  MUTAGEN 8: note = X stands for (S)-2-amino-3-(3-(carboxymethoxy)phenyl)-propanoic acid
  MUTAGEN 9: note = X stands for (S)-4-(2-amino-2-carboxyethyl)-benzoic acid
  MUTAGEN 11: note = X stands for (2S)-2-(methylamino)-3-phenyl-propanoic acid
  MUTAGEN 12: note = X stands for (S)-2-amino-nonanoic acid
  MUTAGEN 13: note = X stands for (2S)-2-(methylamino)-propanoic acid
  MUTAGEN 14: note = X stands for (2S)-2-(methylamino)-3-phenyl-propanoic acid
  MUTAGEN 15: note = X stands for D-cysteine
XAXYXIXXXRXXXXX

SEQ ID NO: 207 - protein, 15 aa, synthetic construct
  MUTAGEN 1: note = X stands for 4-((carboxymethyl)amino)-butanoic acid
  MUTAGEN 3: note = X stands for (S)-2-amino-3-(4-(1-(2-(dimethylamino)-2-oxoethyl)-1H-pyrazole-4-yl)phenyl)-propanoic acid
  MUTAGEN 5: note = X stands for (2S)-2-(methylamino)-3-phenyl-propanoic acid
  MUTAGEN 7: note = X stands for (2S)-2-(methylamino)-propanoic acid
  MUTAGEN 8: note = X stands for (S)-2-amino-3-(2'-chloro-[1,1'-biphenyl]-4-yl)propanoic acid
  MUTAGEN 9: note = X stands for (S)-4-(2-amino-2-carboxyethyl)-benzoic acid
  MUTAGEN 11: note = X stands for (2S)-2-(methylamino)-3-phenyl-propanoic acid
  MUTAGEN 12: note = X stands for (S)-2-amino-nonanoic acid
  MUTAGEN 13: note = X stands for (2S)-2-(methylamino)-pentanedioic acid
  MUTAGEN 14: note = X stands for (2S)-2-(methylamino)-3-phenyl-propanoic acid
  MUTAGEN 15: note = X stands for D-cysteine
XAXYXIXXXRXXXXX

SEQ ID NO: 208 - protein, 15 aa, synthetic construct
  MUTAGEN 1: note = X stands for 4-((carboxymethyl)amino)-butanoic acid
  MUTAGEN 3: note = X stands for (S)-2-amino-3-(6-hydroxy-1H-indol-3-yl)-propanoic acid
  MUTAGEN 5: note = X stands for (2S)-2-(methylamino)-3-phenyl-propanoic acid
  MUTAGEN 7: note = X stands for (2S)-2-(methylamino)-propanoic acid
  MUTAGEN 8: note = X stands for (S)-2-amino-3-(2'-methoxy-[1,1'-biphenyl]-4-yl) propanoic acid
  MUTAGEN 9: note = X stands for (S)-4-(2-amino-2-carboxyethyl)-benzoic acid
  MUTAGEN 11: note = X stands for (2S)-2-(methylamino)-3-phenyl-propanoic acid
  MUTAGEN 12: note = X stands for (S)-2-amino-nonanoic acid
  MUTAGEN 13: note = X stands for (2S)-2-(methylamino)-pentanedioic acid
  MUTAGEN 14: note = X stands for (2S)-2-(methylamino)-3-phenyl-propanoic acid
  MUTAGEN 15: note = X stands for D-cysteine
XAXYXIXXXRXXXXX

SEQ ID NO: 209 - protein, 16 aa, synthetic construct
  MUTAGEN 3: note = X stands for (S)-2-amino-3-(6-hydroxy-1H-indol-3-yl)-propanoic acid
  MUTAGEN 5: note = X stands for (2S)-2-(methylamino)-3-phenyl-propanoic acid
  MUTAGEN 7: note = X stands for 2-(methylamino)-acetic acid
  MUTAGEN 8: note = X stands for (S)-2-amino-3-(2'-chloro-[1,1'-biphenyl]-4-yl)propanoic acid
  MUTAGEN 9: note = X stands for (S)-4-(2-amino-2-carboxyethyl)-benzoic acid
  MUTAGEN 11: note = X stands for (2S)-2-(methylamino)-3-phenyl-propanoic acid
  MUTAGEN 12: note = X stands for (S)-2-amino-nonanoic acid
  MUTAGEN 13: note = X stands for (2S)-2-(methylamino)-pentanedioic acid
  MUTAGEN 14: note = X stands for (2S)-2-(methylamino)-3-phenyl-propanoic acid
  MUTAGEN 15: note = X stands for D-cysteine
  MUTAGEN 16: note = X stands for 2-(piperazin-1-yl)-acetic acid
AAXYXIXXXRXXXXXX

SEQ ID NO: 210 - protein, 16 aa, synthetic construct
  MUTAGEN 3: note = X stands for (2S)-2-amino-3-(1-phenyl-1H-indol-3-yl)-propanoic acid
  MUTAGEN 5: note = X stands for (2S)-2-(methylamino)-3-phenyl-propanoic acid
  MUTAGEN 7: note = X stands for (2S)-2-(methylamino)-propanoic acid
  MUTAGEN 8: note = X stands for (S)-2-amino-3-(3-(carboxymethoxy)phenyl)-propanoic acid
  MUTAGEN 9: note = X stands for (S)-4-(2-amino-2-carboxyethyl)-benzoic acid
  MUTAGEN 11: note = X stands for (2S)-2-(methylamino)-3-phenyl-propanoic acid
  MUTAGEN 12: note = X stands for (S)-2-amino-nonanoic acid
  MUTAGEN 13: note = X stands for (2S)-2-(methylamino)-pentanedioic acid
  MUTAGEN 14: note = X stands for (S)-3-([1,1'-biphenyl]-3-yl)-2-(methylamino)-propanoic acid
  MUTAGEN 15: note = X stands for D-cysteine
  MUTAGEN 16: note = X stands for 2-(piperazin-1-yl)-acetic acid
AAXYXIXXXRXXXXXX

SEQ ID NO: 211 - protein, 16 aa, synthetic construct
  MUTAGEN 3: note = X stands for (2S)-2-amino-3-(1-phenyl-1H-indol-3-yl)-propanoic acid
  MUTAGEN 5: note = X stands for (2S)-2-(methylamino)-3-phenyl-propanoic acid
  MUTAGEN 7: note = X stands for D-proline
  MUTAGEN 8: note = X stands for (S)-2-amino-3-(3-(carboxymethoxy)phenyl)-propanoic acid
  MUTAGEN 9: note = X stands for (S)-4-(2-amino-2-carboxyethyl)-benzoic acid
  MUTAGEN 11: note = X stands for (2S)-2-(methylamino)-3-phenyl-propanoic acid
  MUTAGEN 12: note = X stands for (S)-2-amino-dodecanoic acid
  MUTAGEN 13: note = X stands for (2S)-2-(methylamino)-pentanedioic acid
  MUTAGEN 14: note = X stands for (S)-3-([1,1'-biphenyl]-3-yl)-2-(methylamino)-propanoic acid
  MUTAGEN 15: note = X stands for D-cysteine
  MUTAGEN 16: note = X stands for 2-(piperazin-1-yl)-acetic acid
AAXYXIXXXRXXXXXX

SEQ ID NO: 212 - protein, 16 aa, synthetic construct
  MUTAGEN 3: note = X stands for (2S)-2-amino-3-(1-phenyl-1H-indol-3-yl)-propanoic acid
  MUTAGEN 5: note = X stands for (2S)-2-(methylamino)-3-phenyl-propanoic acid
  MUTAGEN 7: note = X stands for (2S)-2-(methylamino)-propanoic acid
  MUTAGEN 8: note = X stands for (S)-2-amino-3-(3-(carboxymethoxy)phenyl)-propanoic acid
  MUTAGEN 9: note = X stands for (S)-4-(2-amino-2-carboxyethyl)-benzoic acid
  MUTAGEN 11: note = X stands for (S)-2-amino-3-cyclohexyl-propanoic acid
  MUTAGEN 12: note = X stands for (S)-2-amino-dodecanoic acid
  MUTAGEN 13: note = X stands for (2S)-2-(methylamino)-pentanedioic acid
  MUTAGEN 14: note = X stands for (S)-3-([1,1'-biphenyl]-3-yl)-2-(methylamino)-propanoic acid
  MUTAGEN 15: note = X stands for D-cysteine
  MUTAGEN 16: note = X stands for 2-(piperazin-1-yl)-acetic acid
AAXYXIXXXRXXXXXX

SEQ ID NO: 213 - protein, 16 aa, synthetic construct
  MUTAGEN 3: note = X stands for (2S)-2-amino-3-(1-phenyl-1H-indol-3-yl)-propanoic acid
  MUTAGEN 5: note = X stands for (2S)-2-(methylamino)-3-phenyl-propanoic acid
  MUTAGEN 7: note = X stands for (2S)-2-(methylamino)-propanoic acid
  MUTAGEN 8: note = X stands for (S)-2-amino-3-(3-(carboxymethoxy)phenyl)-propanoic acid
  MUTAGEN 9: note = X stands for (S)-4-(2-amino-2-carboxyethyl)-benzoic acid
  MUTAGEN 11: note = X stands for (S)-2-amino-3-cyclohexyl-propanoic acid
  MUTAGEN 12: note = X stands for (S)-2-amino-dodecanoic acid
  MUTAGEN 13: note = X stands for (2S)-2-(methylamino)-pentanedioic acid
  MUTAGEN 14: note = X stands for (2S)-2-(methylamino)-3-phenyl-propanoic acid
  MUTAGEN 15: note = X stands for D-cysteine
  MUTAGEN 16: note = X stands for 2-(piperazin-1-yl)-acetic acid
AAXYXIXXXRXXXXXX

SEQ ID NO: 214 - protein, 16 aa, synthetic construct
  MUTAGEN 5: note = X stands for (2S)-2-(methylamino)-3-phenyl-propanoic acid
  MUTAGEN 7: note = X stands for 2-(propylamino)-acetic acid
  MUTAGEN 8: note = X stands for (S)-2-amino-3-(3-(carboxymethoxy)phenyl)-propanoic acid
  MUTAGEN 9: note = X stands for (S)-4-(2-amino-2-carboxyethyl)-benzoic acid
  MUTAGEN 11: note = X stands for (2S)-2-(methylamino)-3-phenyl-propanoic acid
  MUTAGEN 12: note = X stands for (S)-2-amino-dodecanoic acid
  MUTAGEN 13: note = X stands for (2S)-2-(methylamino)-pentanedioic acid
  MUTAGEN 14: note = X stands for (2S)-2-(methylamino)-3-phenyl-propanoic acid
  MUTAGEN 15: note = X stands for D-cysteine
  MUTAGEN 16: note = X stands for 2-(piperidine-4-yl)-acetic acid
AAWYXIXXXRXXXXXX

SEQ ID NO: 215 - protein, 16 aa, synthetic construct
  MUTAGEN 5: note = X stands for (2S)-2-(methylamino)-3-phenyl-propanoic acid
  MUTAGEN 7: note = X stands for 2-(ethylamino)-acetic acid
  MUTAGEN 8: note = X stands for (S)-2-amino-3-(3-(carboxymethoxy)phenyl)-propanoic acid
  MUTAGEN 9: note = X stands for (S)-4-(2-amino-2-carboxyethyl)-benzoic acid
  MUTAGEN 11: note = X stands for (2S)-2-(methylamino)-3-phenyl-propanoic acid
  MUTAGEN 12: note = X stands for (S)-2-amino-dodecanoic acid
  MUTAGEN 13: note = X stands for (2S)-2-(methylamino)-pentanedioic acid
  MUTAGEN 14: note = X stands for (2S)-2-(methylamino)-3-phenyl-propanoic acid
  MUTAGEN 15: note = X stands for D-cysteine
  MUTAGEN 16: note = X stands for 2-(piperidine-4-yl)-acetic acid
AAWYXIXXXRXXXXXX

SEQ ID NO: 216 - protein, 16 aa, synthetic construct
  MUTAGEN 3: note = X stands for (S)-2-amino-3-(1H-pyrrolo[2,3-c]pyridin-3-yl)-propanoic acid
  MUTAGEN 5: note = X stands for (2S)-2-(methylamino)-3-phenyl-propanoic acid
  MUTAGEN 7: note = X stands for 2-(propylamino)-acetic acid
  MUTAGEN 8: note = X stands for (S)-2-amino-3-(3-(carboxymethoxy)phenyl)-propanoic acid
  MUTAGEN 9: note = X stands for (S)-4-(2-amino-2-carboxyethyl)-benzoic acid
  MUTAGEN 11: note = X stands for (2S)-2-(methylamino)-3-phenyl-propanoic acid
  MUTAGEN 12: note = X stands for (S)-2-amino-dodecanoic acid
  MUTAGEN 13: note = X stands for (2S)-2-(methylamino)-pentanedioic acid
  MUTAGEN 14: note = X stands for (2S)-2-(methylamino)-3-phenyl-propanoic acid
  MUTAGEN 15: note = X stands for D-cysteine
  MUTAGEN 16: note = X stands for 2-(piperidine-4-yl)-acetic acid
AAXYXIXXXRXXXXXX

SEQ ID NO: 217 - protein, 16 aa, synthetic construct
  MUTAGEN 5: note = X stands for (2S)-2-(methylamino)-3-phenyl-propanoic acid
  MUTAGEN 6: note = X stands for (2S, 3R)-2-amino-3-methoxy-butanoic acid
  MUTAGEN 7: note = X stands for 2-(methylamino)-acetic acid
  MUTAGEN 8: note = X stands for (S)-2-amino-3-(3-(carboxymethoxy)phenyl)-propanoic acid
  MUTAGEN 9: note = X stands for (S)-4-(2-amino-2-carboxyethyl)-benzoic acid
  MUTAGEN 11: note = X stands for (2S)-2-(methylamino)-3-phenyl-propanoic acid
  MUTAGEN 12: note = X stands for (S)-2-amino-dodecanoic acid
  MUTAGEN 13: note = X stands for (2S)-2-(methylamino)-pentanedioic acid
  MUTAGEN 14: note = X stands for (2S)-2-(methylamino)-3-phenyl-propanoic acid
  MUTAGEN 15: note = X stands for D-cysteine
  MUTAGEN 16: note = X stands for 2-(piperidine-4-yl)-acetic acid
AAWYXXXXXRXXXXXX

SEQ ID NO: 218 - protein, 16 aa, synthetic construct
  MUTAGEN 3: note = X stands for (S)-2-amino-3-(4'-(methylsulfonyl)-[1,1'-biphenyl]-4-yl)-propanoic acid
  MUTAGEN 5: note = X stands for (2S)-2-(methylamino)-3-phenyl-propanoic acid
  MUTAGEN 7: note = X stands for D-proline
  MUTAGEN 8: note = X stands for (S)-2-amino-3-(3-(carboxymethoxy)phenyl)-propanoic acid
  MUTAGEN 9: note = X stands for (S)-4-(2-amino-2-carboxyethyl)-benzoic acid
  MUTAGEN 11: note = X stands for (2S)-2-(methylamino)-3-phenyl-propanoic acid
  MUTAGEN 12: note = X stands for (S)-2-amino-dodecanoic acid
  MUTAGEN 13: note = X stands for (2S)-2-(methylamino)-pentanedioic acid
  MUTAGEN 14: note = X stands for (2S)-2-(methylamino)-3-phenyl-propanoic acid
  MUTAGEN 15: note = X stands for D-cysteine
  MUTAGEN 16: note = X stands for 2-(piperidine-4-yl)-acetic acid
AAXYXIXXXRXXXXXX

SEQ ID NO: 219 - protein, 16 aa, synthetic construct
  MUTAGEN 3: note = X stands for (S)-2-amino-3-(4'-(methylsulfonyl)-[1,1'-biphenyl]-4-yl)-propanoic acid
  MUTAGEN 5: note = X stands for (2S)-2-(methylamino)-3-phenyl-propanoic acid
  MUTAGEN 7: note = X stands for D-proline
  MUTAGEN 8: note = X stands for (S)-2-amino-3-(3-(carboxymethoxy)phenyl)-propanoic acid
  MUTAGEN 9: note = X stands for (S)-4-(2-amino-2-carboxyethyl)-benzoic acid
  MUTAGEN 11: note = X stands for (2S)-2-(methylamino)-3-phenyl-propanoic acid
  MUTAGEN 12: note = X stands for (S)-2-amino-dodecanoic acid
  MUTAGEN 13: note = X stands for (2S)-2-(methylamino)-pentanedioic acid
  MUTAGEN 14: note = X stands for (2S)-2-(methylamino)-3-phenyl-propanoic acid
  MUTAGEN 15: note = X stands for D-cysteine
  MUTAGEN 16: note = X stands for 3-(piperidine-4-yl)-propanoic acid
AAXYXIXXXRXXXXXX

SEQ ID NO: 220 - protein, 16 aa, synthetic construct
  MUTAGEN 5: note = X stands for (2S)-2-(methylamino)-3-phenyl-propanoic acid
  MUTAGEN 7: note = X stands for D-proline
  MUTAGEN 8: note = X stands for (S)-2-amino-3-(3-(carboxymethoxy)phenyl)-propanoic acid
  MUTAGEN 9: note = X stands for (S)-4-(2-amino-2-carboxyethyl)-benzoic acid
  MUTAGEN 11: note = X stands for (2S)-2-(methylamino)-3-phenyl-propanoic acid
  MUTAGEN 12: note = X stands for (S)-2-amino-dodecanoic acid
  MUTAGEN 13: note = X stands for (2S)-2-(methylamino)-pentanedioic acid
  MUTAGEN 14: note = X stands for (2S)-2-(methylamino)-3-phenyl-propanoic acid
  MUTAGEN 15: note = X stands for D-cysteine
  MUTAGEN 16: note = X stands for 2-(piperidine-4-yl)-acetic acid
AAWYXIXXXRXXXXXX

SEQ ID NO: 221 - protein, 15 aa, synthetic construct
  MUTAGEN 1: note = X stands for 4-((carboxymethyl)amino)-butanoic acid
  MUTAGEN 3: note = X stands for (S)-2-amino-3-(4'-(methylsulfonyl)-[1,1'-biphenyl]-4-yl)-propanoic acid
  MUTAGEN 5: note = X stands for (2S)-2-(methylamino)-3-phenyl-propanoic acid
  MUTAGEN 7: note = X stands for (2S)-2-(methylamino)-propanoic acid
  MUTAGEN 8: note = X stands for (S)-2-amino-3-(3-(carboxymethoxy)phenyl)-propanoic acid
  MUTAGEN 9: note = X stands for (S)-4-(2-amino-2-carboxyethyl)-benzoic acid
  MUTAGEN 11: note = X stands for (2S)-2-(methylamino)-3-phenyl-propanoic acid
  MUTAGEN 12: note = X stands for (S)-2-amino-nonanoic acid
  MUTAGEN 13: note = X stands for (2S)-2-(methylamino)-propanoic acid
  MUTAGEN 14: note = X stands for (2S)-2-(methylamino)-3-phenyl-propanoic acid
  MUTAGEN 15: note = X stands for D-cysteine
XAXYXIXXXRXXXXX

SEQ ID NO: 222 - protein, 15 aa, synthetic construct
  MUTAGEN 1: note = X stands for 4-((carboxymethyl)amino)-butanoic acid
  MUTAGEN 5: note = X stands for (2S)-2-(methylamino)-3-phenyl-propanoic acid
  MUTAGEN 7: note = X stands for (2S)-2-(methylamino)-propanoic acid
  MUTAGEN 8: note = X stands for (S)-2-amino-3-(2'-(carboxymethoxy)-[1,1'-biphenyl]-4-yl )propanoic acid
  MUTAGEN 9: note = X stands for (S)-4-(2-amino-2-carboxyethyl)-benzoic acid
  MUTAGEN 11: note = X stands for (2S)-2-(methylamino)-3-phenyl-propanoic acid
  MUTAGEN 12: note = X stands for (S)-2-amino-nonanoic acid
  MUTAGEN 13: note = X stands for (2S)-2-(methylamino)-propanoic acid
  MUTAGEN 14: note = X stands for (2S)-2-(methylamino)-3-phenyl-propanoic acid
  MUTAGEN 15: note = X stands for D-cysteine
XAWYXIXXXRXXXXX

SEQ ID NO: 223 - protein, 15 aa, synthetic construct
  MUTAGEN 1: note = X stands for 4-((carboxymethyl)amino)-butanoic acid
  MUTAGEN 3: note = X stands for (S)-2-amino-3-(6-hydroxy-1H-indol-3-yl)-propanoic acid
  MUTAGEN 5: note = X stands for (2S)-2-(methylamino)-3-phenyl-propanoic acid
  MUTAGEN 7: note = X stands for (2S)-2-(methylamino)-propanoic acid
  MUTAGEN 8: note = X stands for (S)-2-amino-3-(2'-(carboxymethoxy)-[1,1'-biphenyl]-4-yl )propanoic acid
  MUTAGEN 9: note = X stands for (S)-4-(2-amino-2-carboxyethyl)-benzoic acid
  MUTAGEN 11: note = X stands for (2S)-2-(methylamino)-3-phenyl-propanoic acid
  MUTAGEN 12: note = X stands for (S)-2-amino-nonanoic acid
  MUTAGEN 13: note = X stands for (2S)-2-(methylamino)-propanoic acid
  MUTAGEN 14: note = X stands for (2S)-2-(methylamino)-3-phenyl-propanoic acid
  MUTAGEN 15: note = X stands for D-cysteine
XAXYXIXXXRXXXXX

SEQ ID NO: 224 - protein, 15 aa, synthetic construct
  MUTAGEN 1: note = X stands for 4-((carboxymethyl)amino)-butanoic acid
  MUTAGEN 3: note = X stands for (S)-2-amino-3-(7-(3-chlorophenyl)-1H-indole-3-yl)-propanoic acid
  MUTAGEN 5: note = X stands for (2S)-2-(methylamino)-3-phenyl-propanoic acid
  MUTAGEN 7: note = X stands for (2S)-2-(methylamino)-propanoic acid
  MUTAGEN 8: note = X stands for (S)-2-amino-3-(3-(carboxymethoxy)phenyl)-propanoic acid
  MUTAGEN 9: note = X stands for (S)-4-(2-amino-2-carboxyethyl)-benzoic acid
  MUTAGEN 11: note = X stands for (2S)-2-(methylamino)-3-phenyl-propanoic acid
  MUTAGEN 12: note = X stands for (S)-2-amino-nonanoic acid
  MUTAGEN 13: note = X stands for (2S)-2-(methylamino)-propanoic acid
  MUTAGEN 14: note = X stands for (2S)-2-(methylamino)-3-phenyl-propanoic acid
  MUTAGEN 15: note = X stands for D-cysteine
XAXYXIXXXRXXXXX

SEQ ID NO: 225 - protein, 15 aa, synthetic construct
  MUTAGEN 1: note = X stands for 4-((carboxymethyl)amino)-butanoic acid
  MUTAGEN 3: note = X stands for (2S)-2-amino-3-(1-(4-methoxyphenyl)-1H-indole-3-yl)-propanoic acid
  MUTAGEN 5: note = X stands for (2S)-2-(methylamino)-3-phenyl-propanoic acid
  MUTAGEN 7: note = X stands for (2S)-2-(methylamino)-propanoic acid
  MUTAGEN 8: note = X stands for (S)-2-amino-3-(3-(carboxymethoxy)phenyl)-propanoic acid
  MUTAGEN 9: note = X stands for (S)-4-(2-amino-2-carboxyethyl)-benzoic acid
  MUTAGEN 11: note = X stands for (2S)-2-(methylamino)-3-phenyl-propanoic acid
  MUTAGEN 12: note = X stands for (S)-2-amino-nonanoic acid
  MUTAGEN 13: note = X stands for (2S)-2-(methylamino)-propanoic acid
  MUTAGEN 14: note = X stands for (2S)-2-(methylamino)-3-phenyl-propanoic acid
  MUTAGEN 15: note = X stands for D-cysteine
XAXYXIXXXRXXXXX

SEQ ID NO: 226 - protein, 15 aa, synthetic construct
  MUTAGEN 1: note = X stands for 4-((carboxymethyl)amino)-butanoic acid
  MUTAGEN 3: note = X stands for (2S)-2-amino-3-(1-phenyl-1H-indol-3-yl)-propanoic acid
  MUTAGEN 5: note = X stands for (2S)-2-(methylamino)-3-phenyl-propanoic acid
  MUTAGEN 7: note = X stands for (2S)-2-(methylamino)-propanoic acid
  MUTAGEN 8: note = X stands for (S)-2-amino-3-(3-(carboxymethoxy)phenyl)-propanoic acid
  MUTAGEN 9: note = X stands for (S)-4-(2-amino-2-carboxyethyl)-benzoic acid
  MUTAGEN 11: note = X stands for (2S)-2-(methylamino)-3-phenyl-propanoic acid
  MUTAGEN 12: note = X stands for (S)-2-amino-nonanoic acid
  MUTAGEN 13: note = X stands for (2S)-2-(methylamino)-propanoic acid
  MUTAGEN 14: note = X stands for (2S)-2-(methylamino)-3-phenyl-propanoic acid
  MUTAGEN 15: note = X stands for D-cysteine
XAXYXIXXXRXXXXX

SEQ ID NO: 227 - protein, 16 aa, synthetic construct
  MUTAGEN 5: note = X stands for (2S)-2-(methylamino)-3-phenyl-propanoic acid
  MUTAGEN 7: note = X stands for 2-(methylamino)-acetic acid
  MUTAGEN 8: note = X stands for (S)-2-amino-3-(3-(carboxymethoxy)phenyl)-propanoic acid
  MUTAGEN 9: note = X stands for (S)-4-(2-amino-2-carboxyethyl)-benzoic acid
  MUTAGEN 11: note = X stands for (2S)-2-(methylamino)-3-phenyl-propanoic acid
  MUTAGEN 12: note = X stands for (S)-2-amino-nonanoic acid
  MUTAGEN 13: note = X stands for (2S)-2-(methylamino)-propanoic acid
  MUTAGEN 14: note = X stands for (2S)-2-(methylamino)-3-phenyl-propanoic acid
  MUTAGEN 15: note = X stands for D-cysteine
  MUTAGEN 16: note = X stands for (2S)-2-amino-6-{[4-(carboxymethyl)piperazine-1-carbonyl]amino} hexanoic acid
AAWYXIXXXRXXXXXX

SEQ ID NO: 228 - protein, 16 aa, synthetic construct
  MUTAGEN 1: note = X stands for 4-((carboxymethyl)amino)-butanoic acid
  MUTAGEN 5: note = X stands for (2S)-2-(methylamino)-3-phenyl-propanoic acid
  MUTAGEN 7: note = X stands for (2S)-2-(methylamino)-propanoic acid
  MUTAGEN 8: note = X stands for (S)-2-amino-3-(3-(carboxymethoxy)phenyl)-propanoic acid
  MUTAGEN 9: note = X stands for (S)-4-(2-amino-2-carboxyethyl)-benzoic acid
  MUTAGEN 11: note = X stands for (2S)-2-(methylamino)-3-phenyl-propanoic acid
  MUTAGEN 12: note = X stands for (S)-2-amino-nonanoic acid
  MUTAGEN 13: note = X stands for (2S)-2-(methylamino)-propanoic acid
  MUTAGEN 14: note = X stands for (2S)-2-(methylamino)-3-phenyl-propanoic acid
  MUTAGEN 15: note = X stands for D-cysteine
  MUTAGEN 16: note = X stands for (2S)-2-amino-6-{[4-(carboxymethyl)piperazine-1-carbonyl]amino} hexanoic acid
XAWYXIXXXRXXXXXX

SEQ ID NO: 229 - protein, 16 aa, unidentified
  MUTAGEN 1: note = X stands for 4-((carboxymethyl)amino)-butanoic acid
  MUTAGEN 5: note = X stands for (2S)-2-(methylamino)-3-phenyl-propanoic acid
  MUTAGEN 7: note = X stands for (2S)-2-(methylamino)-propanoic acid
  MUTAGEN 8: note = X stands for (S)-2-amino-3-(3-(carboxymethoxy)phenyl)-propanoic acid
  MUTAGEN 9: note = X stands for (S)-4-(2-amino-2-carboxyethyl)-benzoic acid
  MUTAGEN 11: note = X stands for (2S)-2-(methylamino)-3-phenyl-propanoic acid
  MUTAGEN 12: note = X stands for (S)-2-amino-nonanoic acid
  MUTAGEN 13: note = X stands for (2S)-2-(methylamino)-propanoic acid
  MUTAGEN 14: note = X stands for (2S)-2-(methylamino)-3-phenyl-propanoic acid
  MUTAGEN 15: note = X stands for D-cysteine
  MUTAGEN 16: note = X stands for 2-(piperazin-1-yl)-acetic acid
XAWYXIXXXRXXXXXX

SEQ ID NO: 230 - protein, 16 aa, synthetic construct
  MUTAGEN 1: note = X stands for 4-((carboxymethyl)amino)-butanoic acid
  MUTAGEN 5: note = X stands for (2S)-2-(methylamino)-3-phenyl-propanoic acid
  MUTAGEN 7: note = X stands for (2S)-2-(methylamino)-propanoic acid
  MUTAGEN 8: note = X stands for (S)-2-amino-3-(3-(carboxymethoxy)phenyl)-propanoic acid
  MUTAGEN 9: note = X stands for (S)-4-(2-amino-2-carboxyethyl)-benzoic acid
  MUTAGEN 11: note = X stands for (2S)-2-(methylamino)-3-phenyl-propanoic acid
  MUTAGEN 12: note = X stands for (S)-2-amino-nonanoic acid
  MUTAGEN 13: note = X stands for (2S)-2-(methylamino)-propanoic acid
  MUTAGEN 14: note = X stands for (2S)-2-(methylamino)-3-phenyl-propanoic acid
  MUTAGEN 15: note = X stands for D-cysteine
  MUTAGEN 16: note = X stands for 2-(piperidine-4-yl)-acetic acid
XAWYXIXXXRXXXXXX

SEQ ID NO: 231 - protein, 16 aa, synthetic construct
  MUTAGEN 1: note = X stands for 4-((carboxymethyl)amino)-butanoic acid
  MUTAGEN 5: note = X stands for (2S)-2-(methylamino)-3-phenyl-propanoic acid
  MUTAGEN 7: note = X stands for (2S)-2-(methylamino)-propanoic acid
  MUTAGEN 8: note = X stands for (S)-2-amino-3-(3-(carboxymethoxy)phenyl)-propanoic acid
  MUTAGEN 9: note = X stands for (S)-4-(2-amino-2-carboxyethyl)-benzoic acid
  MUTAGEN 11: note = X stands for (2S)-2-(methylamino)-3-phenyl-propanoic acid
  MUTAGEN 12: note = X stands for (S)-2-amino-nonanoic acid
  MUTAGEN 13: note = X stands for (2S)-2-(methylamino)-propanoic acid
  MUTAGEN 14: note = X stands for (2S)-2-(methylamino)-3-phenyl-propanoic acid
  MUTAGEN 15: note = X stands for D-cysteine
  MUTAGEN 16: note = X stands for 3-(piperidine-4-yl)-propanoic acid
XAWYXIXXXRXXXXXX

SEQ ID NO: 232 - protein, 16 aa, synthetic construct
  MUTAGEN 1: note = X stands for 4-((carboxymethyl)amino)-butanoic acid
  MUTAGEN 5: note = X stands for (2S)-2-(methylamino)-3-phenyl-propanoic acid
  MUTAGEN 7: note = X stands for (2S)-2-(methylamino)-propanoic acid
  MUTAGEN 8: note = X stands for (S)-2-amino-3-(3-(carboxymethoxy)phenyl)-propanoic acid
  MUTAGEN 9: note = X stands for (S)-4-(2-amino-2-carboxyethyl)-benzoic acid
  MUTAGEN 11: note = X stands for (2S)-2-(methylamino)-3-phenyl-propanoic acid
  MUTAGEN 12: note = X stands for (S)-2-amino-nonanoic acid
  MUTAGEN 13: note = X stands for (2S)-2-(methylamino)-propanoic acid
  MUTAGEN 14: note = X stands for (2S)-2-(methylamino)-3-phenyl-propanoic acid
  MUTAGEN 15: note = X stands for D-cysteine
  MUTAGEN 16: note = X stands for 2-(piperidine-4-yl)-acetic acid
XAWYXIXXXRXXXXXX

SEQ ID NO: 233 - protein, 16 aa, synthetic construct
  MUTAGEN 1: note = X stands for 4-((carboxymethyl)amino)-butanoic acid
  MUTAGEN 5: note = X stands for (2S)-2-(methylamino)-3-phenyl-propanoic acid
  MUTAGEN 7: note = X stands for (2S)-2-(methylamino)-propanoic acid
  MUTAGEN 8: note = X stands for (S)-2-amino-3-(3-(carboxymethoxy)phenyl)-propanoic acid
  MUTAGEN 9: note = X stands for (S)-4-(2-amino-2-carboxyethyl)-benzoic acid
  MUTAGEN 11: note = X stands for (2S)-2-(methylamino)-3-phenyl-propanoic acid
  MUTAGEN 12: note = X stands for (S)-2-amino-nonanoic acid
  MUTAGEN 13: note = X stands for (2S)-2-(methylamino)-propanoic acid
  MUTAGEN 14: note = X stands for (2S)-2-(methylamino)-3-phenyl-propanoic acid
  MUTAGEN 15: note = X stands for D-cysteine
  MUTAGEN 16: note = X stands for piperidine-4-carboxylic acid
XAWYXIXXXRXXXXXX

SEQ ID NO: 234 - protein, 15 aa, synthetic construct
  MUTAGEN 1: note = X stands for 4-((carboxymethyl)amino)-butanoic acid
  MUTAGEN 5: note = X stands for (2S)-2-(methylamino)-3-phenyl-propanoic acid
  MUTAGEN 7: note = X stands for (2S)-2-(methylamino)-propanoic acid
  MUTAGEN 8: note = X stands for (S)-2-amino-3-(3-(carboxymethoxy)phenyl)-propanoic acid
  MUTAGEN 9: note = X stands for (S)-4-(2-amino-2-carboxyethyl)-benzoic acid
  MUTAGEN 11: note = X stands for (2S)-2-(methylamino)-3-phenyl-propanoic acid
  MUTAGEN 12: note = X stands for (S)-2-amino-nonanoic acid
  MUTAGEN 13: note = X stands for (2S)-2-(methylamino)-propanoic acid
  MUTAGEN 14: note = X stands for (2S)-2-(methylamino)-3-phenyl-propanoic acid
  MUTAGEN 15: note = X stands for (2S )-2-(methylamino)-3-sulfanyl-propanoic acid
XAWYXIXXXRXXXXX

SEQ ID NO: 235 - protein, 15 aa, synthetic construct
  MUTAGEN 1: note = X stands for 4-((carboxymethyl)amino)-butanoic acid
  MUTAGEN 5: note = X stands for (2S)-2-(methylamino)-3-phenyl-propanoic acid
  MUTAGEN 7: note = X stands for (2S)-2-(methylamino)-propanoic acid
  MUTAGEN 8: note = X stands for (S)-2-amino-3-(3-(carboxymethoxy)phenyl)-propanoic acid
  MUTAGEN 9: note = X stands for (S)-4-(2-amino-2-carboxyethyl)-benzoic acid
  MUTAGEN 11: note = X stands for (2S)-2-(methylamino)-3-phenyl-propanoic acid
  MUTAGEN 12: note = X stands for (S)-2-amino-nonanoic acid
  MUTAGEN 13: note = X stands for (2S)-2-(methylamino)-propanoic acid
  MUTAGEN 14: note = X stands for (2S)-2-(methylamino)-3-phenyl-propanoic acid
  MUTAGEN 15: note = X stands for (2R)-2-(methylamino)-3-sulfanyl-propanoic acid
XAWYXIXXXRXXXXX

SEQ ID NO: 236 - protein, 15 aa, synthetic construct
  MUTAGEN 1: note = X stands for 4-((carboxymethyl)amino)-butanoic acid
  MUTAGEN 5: note = X stands for (2S)-2-(methylamino)-3-phenyl-propanoic acid
  MUTAGEN 7: note = X stands for (2S)-2-(methylamino)-propanoic acid
  MUTAGEN 8: note = X stands for (S)-2-amino-3-(3-(carboxymethoxy)phenyl)-propanoic acid
  MUTAGEN 9: note = X stands for (S)-4-(2-amino-2-carboxyethyl)-benzoic acid
  MUTAGEN 11: note = X stands for (2S)-2-(methylamino)-3-phenyl-propanoic acid
  MUTAGEN 12: note = X stands for (S)-2-amino-nonanoic acid
  MUTAGEN 13: note = X stands for (2S)-2-(methylamino)-propanoic acid
  MUTAGEN 14: note = X stands for (2S)-2-(methylamino)-3-phenyl-propanoic acid
  MUTAGEN 15: note = X stands for (2R)-2-amino-4-sulfanyl-butanoic acid
XAWYXIXXXRXXXXX

SEQ ID NO: 237 - protein, 15 aa, synthetic construct
  MUTAGEN 1: note = X stands for 4-((carboxymethyl)amino)-butanoic acid
  MUTAGEN 5: note = X stands for (2S)-2-(methylamino)-3-phenyl-propanoic acid
  MUTAGEN 7: note = X stands for (2S)-2-(methylamino)-propanoic acid
  MUTAGEN 8: note = X stands for (S)-2-amino-3-(3-(carboxymethoxy)phenyl)-propanoic acid
  MUTAGEN 9: note = X stands for (S)-4-(2-amino-2-carboxyethyl)-benzoic acid
  MUTAGEN 11: note = X stands for (2S)-2-(methylamino)-3-phenyl-propanoic acid
  MUTAGEN 12: note = X stands for (S)-2-amino-nonanoic acid
  MUTAGEN 13: note = X stands for (2S)-2-(methylamino)-propanoic acid
  MUTAGEN 14: note = X stands for (2S)-2-(methylamino)-3-phenyl-propanoic acid
  MUTAGEN 15: note = X stands for (2S)-2-amino-4-sulfanyl-butanoic acid
XAWYXIXXXRXXXXX

SEQ ID NO: 238 - protein, 15 aa, synthetic construct
  MUTAGEN 5: note = X stands for (2S)-2-(methylamino)-3-phenyl-propanoic acid
  MUTAGEN 7: note = X stands for (2S)-2-(methylamino)-propanoic acid
  MUTAGEN 8: note = X stands for (S)-2-amino-3-(3-(carboxymethoxy)phenyl)-propanoic acid
  MUTAGEN 9: note = X stands for (S)-4-(2-amino-2-carboxyethyl)-benzoic acid
  MUTAGEN 11: note = X stands for (S)-3-(4-(aminomethyl)phenyl)-2-(methylamino)-propanoic acid
  MUTAGEN 12: note = X stands for (S)-2-amino-nonanoic acid
  MUTAGEN 13: note = X stands for (2S)-2-(methylamino)-propanoic acid
  MUTAGEN 14: note = X stands for (2S)-2-(methylamino)-3-phenyl-propanoic acid
  MUTAGEN 15: note = X stands for D-cysteine
EAWYXIXXXRXXXXX

SEQ ID NO: 239 - protein, 15 aa, synthetic construct
  MUTAGEN 5: note = X stands for (2S)-2-(methylamino)-3-phenyl-propanoic acid
  MUTAGEN 7: note = X stands for (2S)-2-(methylamino)-propanoic acid
  MUTAGEN 8: note = X stands for (S)-2-amino-3-(3-(carboxymethoxy)phenyl)-propanoic acid
  MUTAGEN 9: note = X stands for (S)-4-(2-amino-2-carboxyethyl)-benzoic acid
  MUTAGEN 11: note = X stands for (2S)-2-(methylamino)-3-phenyl-propanoic acid
  MUTAGEN 12: note = X stands for (S)-2-amino-nonanoic acid
  MUTAGEN 13: note = X stands for (S)-4-amino-2-(methylamino)-butanoic acid
  MUTAGEN 14: note = X stands for (2S)-2-(methylamino)-3-phenyl-propanoic acid
  MUTAGEN 15: note = X stands for D-cysteine
DAWYXIXXXRXXXXX

SEQ ID NO: 240 - protein, 15 aa, synthetic construct
  MUTAGEN 5: note = X stands for (2S)-2-(methylamino)-3-phenyl-propanoic acid
  MUTAGEN 7: note = X stands for (2S)-2-(methylamino)-propanoic acid
  MUTAGEN 8: note = X stands for (S)-2-amino-3-(3-(carboxymethoxy)phenyl)-propanoic acid
  MUTAGEN 9: note = X stands for (S)-4-(2-amino-2-carboxyethyl)-benzoic acid
  MUTAGEN 11: note = X stands for (S)-3-(4-(aminomethyl)phenyl)-2-(methylamino)-propanoic acid
  MUTAGEN 12: note = X stands for (S)-2-amino-nonanoic acid
  MUTAGEN 13: note = X stands for (2S)-2-(methylamino)-propanoic acid
  MUTAGEN 14: note = X stands for (2S)-2-(methylamino)-3-phenyl-propanoic acid
  MUTAGEN 15: note = X stands for D-cysteine
DAWYXIXXXRXXXXX

SEQ ID NO: 241 - protein, 15 aa, synthetic construct
  MUTAGEN 3: note = X stands for (S)-2-amino-3-(6-hydroxy-1H-indol-3-yl)-propanoic acid
  MUTAGEN 5: note = X stands for (2S)-2-(methylamino)-3-phenyl-propanoic acid
  MUTAGEN 7: note = X stands for (2S)-2-(methylamino)-propanoic acid
  MUTAGEN 8: note = X stands for (S)-2-amino-3-(3-(carboxymethoxy)phenyl)-propanoic acid
  MUTAGEN 9: note = X stands for (S)-4-(2-amino-2-carboxyethyl)-benzoic acid
  MUTAGEN 11: note = X stands for (S)-3-(4-(aminomethyl)phenyl)-2-(methylamino)-propanoic acid
  MUTAGEN 12: note = X stands for (S)-2-amino-nonanoic acid
  MUTAGEN 13: note = X stands for (2S)-2-(methylamino)-propanoic acid
  MUTAGEN 14: note = X stands for (2S)-2-(methylamino)-3-phenyl-propanoic acid
  MUTAGEN 15: note = X stands for D-cysteine
EAXYXIXXXRXXXXX

SEQ ID NO: 242 - protein, 15 aa, synthetic construct
  MUTAGEN 3: note = X stands for 4-{3-[(2S)-2-amino-2-carboxyethyl]-1H-indole-1-yl}-benzoic acid
  MUTAGEN 5: note = X stands for (2S)-2-(methylamino)-3-phenyl-propanoic acid
  MUTAGEN 7: note = X stands for (2S)-2-(methylamino)-propanoic acid
  MUTAGEN 8: note = X stands for (S)-2-amino-3-(3-(carboxymethoxy)phenyl)-propanoic acid
  MUTAGEN 9: note = X stands for (S)-4-(2-amino-2-carboxyethyl)-benzoic acid
  MUTAGEN 11: note = X stands for (S)-3-(4-(aminomethyl)phenyl)-2-(methylamino)-propanoic acid
  MUTAGEN 12: note = X stands for (S)-2-amino-nonanoic acid
  MUTAGEN 13: note = X stands for (2S)-2-(methylamino)-propanoic acid
  MUTAGEN 14: note = X stands for (2S)-2-(methylamino)-3-phenyl-propanoic acid
  MUTAGEN 15: note = X stands for D-cysteine
EAXYXIXXXRXXXXX

SEQ ID NO: 243 - protein, 15 aa, synthetic construct
  MUTAGEN 3: note = X stands for (S)-2-amino-3-(6-hydroxy-1H-indol-3-yl)-propanoic acid
  MUTAGEN 5: note = X stands for (2S)-2-(methylamino)-3-phenyl-propanoic acid
  MUTAGEN 7: note = X stands for (2S)-2-(methylamino)-propanoic acid
  MUTAGEN 8: note = X stands for (S)-2-amino-3-(3-(carboxymethoxy)phenyl)-propanoic acid
  MUTAGEN 9: note = X stands for (S)-4-(2-amino-2-carboxyethyl)-benzoic acid
  MUTAGEN 11: note = X stands for (S)-3-(4-(aminomethyl)phenyl)-2-(methylamino)-propanoic acid
  MUTAGEN 12: note = X stands for (S)-2-amino-nonanoic acid
  MUTAGEN 13: note = X stands for (2S)-2-(methylamino)-pentanedioic acid
  MUTAGEN 14: note = X stands for (2S)-2-(methylamino)-3-phenyl-propanoic acid
  MUTAGEN 15: note = X stands for D-cysteine
EAXYXIXXXRXXXXX

SEQ ID NO: 244 - protein, 15 aa, synthetic construct
  MUTAGEN 1: note = X stands for (2S)-2-(methylamino)-pentanedioic acid
  MUTAGEN 2: note = X stands for D-alanine
  MUTAGEN 5: note = X stands for (2S)-2-(methylamino)-3-phenyl-propanoic acid
  MUTAGEN 7: note = X stands for (2S)-2-(methylamino)-propanoic acid
  MUTAGEN 8: note = X stands for (S)-2-amino-3-(3-(carboxymethoxy)phenyl)-propanoic acid
  MUTAGEN 9: note = X stands for (S)-4-(2-amino-2-carboxyethyl)-benzoic acid
  MUTAGEN 11: note = X stands for (S)-3-(4-(aminomethyl)phenyl)-2-(methylamino)-propanoic acid
  MUTAGEN 12: note = X stands for (S)-2-amino-nonanoic acid
  MUTAGEN 13: note = X stands for (2S)-2-(methylamino)-propanoic acid
  MUTAGEN 14: note = X stands for (2S)-2-(methylamino)-3-phenyl-propanoic acid
  MUTAGEN 15: note = X stands for D-cysteine
XXWYXIXXXRXXXXX

SEQ ID NO: 245 - protein, 15 aa, synthetic construct
  MUTAGEN 1: note = X stands for 3-((carboxymethyl)amino)-propanoic acid
  MUTAGEN 3: note = X stands for (S)-2-amino-3-(6-hydroxy-1H-indol-3-yl)-propanoic acid
  MUTAGEN 5: note = X stands for (2S)-2-(methylamino)-3-phenyl-propanoic acid
  MUTAGEN 7: note = X stands for (2S)-2-(methylamino)-propanoic acid
  MUTAGEN 8: note = X stands for (S)-2-amino-3-(3-(carboxymethoxy)phenyl)-propanoic acid
  MUTAGEN 9: note = X stands for (S)-2-amino-3-(4-fluorophenyl)-propanoic acid
  MUTAGEN 11: note = X stands for (2S)-2-(methylamino)-3-phenyl-propanoic acid
  MUTAGEN 12: note = X stands for (S)-2-amino-nonanoic acid
  MUTAGEN 13: note = X stands for (S)-3-amino-2-(methylamino)-propanoic acid
  MUTAGEN 14: note = X stands for (2S)-2-(methylamino)-3-phenyl-propanoic acid
  MUTAGEN 15: note = X stands for D-cysteine
XAXYXIXXXRXXXXX

SEQ ID NO: 246 - protein, 16 aa, synthetic construct
  MUTAGEN 3: note = X stands for 4-{3-[(2S)-2-amino-2-carboxyethyl]-1H-indole-1-yl}-benzoic acid
  MUTAGEN 5: note = X stands for (2S)-2-(methylamino)-3-phenyl-propanoic acid
  MUTAGEN 7: note = X stands for D-proline
  MUTAGEN 8: note = X stands for (S)-2-amino-3-(3-(carboxymethoxy)phenyl)-propanoic acid
  MUTAGEN 9: note = X stands for (S)-4-(2-amino-2-carboxyethyl)-benzoic acid
  MUTAGEN 11: note = X stands for (S)-3-(4-(aminomethyl)phenyl)-2-(methylamino)-propanoic acid
  MUTAGEN 12: note = X stands for (S)-2-amino-dodecanoic acid
  MUTAGEN 13: note = X stands for (2S)-2-(methylamino)-pentanedioic acid
  MUTAGEN 14: note = X stands for (2S)-2-(methylamino)-3-phenyl-propanoic acid
  MUTAGEN 15: note = X stands for D-cysteine
  MUTAGEN 16: note = X stands for 3-(piperidine-4-yl)-propanoic acid
EAXYXIXXXRXXXXXX

SEQ ID NO: 247 - protein, 15 aa, synthetic construct
  MUTAGEN 1: note = X stands for (2S)-2-(methylamino)-pentanedioic acid
  MUTAGEN 3: note = X stands for (S)-2-amino-3-(6-hydroxy-1H-indol-3-yl)-propanoic acid
  MUTAGEN 5: note = X stands for (2S)-2-(methylamino)-3-phenyl-propanoic acid
  MUTAGEN 7: note = X stands for 2-(methylamino)-acetic acid
  MUTAGEN 8: note = X stands for (S)-2-amino-3-(3-(carboxymethoxy)phenyl)-propanoic acid
  MUTAGEN 9: note = X stands for (S)-4-(2-amino-2-carboxyethyl)-benzoic acid
  MUTAGEN 11: note = X stands for (S)-3-(4-(aminomethyl)phenyl)-2-(methylamino)-propanoic acid
  MUTAGEN 12: note = X stands for (S)-2-amino-decanoic acid
  MUTAGEN 13: note = X stands for (2S)-2-(methylamino)-propanoic acid
  MUTAGEN 14: note = X stands for (2S)-2-(methylamino)-3-phenyl-propanoic acid
  MUTAGEN 15: note = X stands for D-cysteine
XAXYXIXXXRXXXXX

SEQ ID NO: 248 - protein, 15 aa, synthetic construct
  MUTAGEN 1: note = X stands for 3-((carboxymethyl)amino)-propanoic acid
  MUTAGEN 3: note = X stands for (S)-2-amino-3-(6-hydroxy-1H-indol-3-yl)-propanoic acid
  MUTAGEN 5: note = X stands for (2S)-2-(methylamino)-3-phenyl-propanoic acid
  MUTAGEN 7: note = X stands for 2-(methylamino)-acetic acid
  MUTAGEN 8: note = X stands for (S)-2-amino-3-(3-(carboxymethoxy)phenyl)-propanoic acid
  MUTAGEN 9: note = X stands for (S)-4-(2-amino-2-carboxyethyl)-benzoic acid
  MUTAGEN 11: note = X stands for (2S)-2-(methylamino)-3-phenyl-propanoic acid
  MUTAGEN 12: note = X stands for (S)-2-amino-decanoic acid
  MUTAGEN 13: note = X stands for (S)-3-amino-2-(methylamino)-propanoic acid
  MUTAGEN 14: note = X stands for (2S)-2-(methylamino)-3-phenyl-propanoic acid
  MUTAGEN 15: note = X stands for D-cysteine
XAXYXIXXXRXXXXX

SEQ ID NO: 249 - protein, 15 aa, synthetic construct
  MUTAGEN 1: note = X stands for (2S)-2-(methylamino)-pentanedioic acid
  MUTAGEN 3: note = X stands for (S)-2-amino-3-(6-hydroxy-1H-indol-3-yl)-propanoic acid
  MUTAGEN 5: note = X stands for (2S)-2-(methylamino)-3-phenyl-propanoic acid
  MUTAGEN 7: note = X stands for 2-(methylamino)-acetic acid
  MUTAGEN 8: note = X stands for (S)-2-amino-3-(3-(carboxymethoxy)phenyl)-propanoic acid
  MUTAGEN 9: note = X stands for (S)-2-amino-3-(4-methoxyphenyl)-propanoic acid
  MUTAGEN 11: note = X stands for (S)-3-(4-(aminomethyl)phenyl)-2-(methylamino)-propanoic acid
  MUTAGEN 12: note = X stands for (S)-2-amino-decanoic acid
  MUTAGEN 13: note = X stands for (2S)-2-(methylamino)-propanoic acid
  MUTAGEN 14: note = X stands for (2S)-2-(methylamino)-3-phenyl-propanoic acid
  MUTAGEN 15: note = X stands for D-cysteine
XAXYXIXXXRXXXXX

SEQ ID NO: 250 - protein, 15 aa, synthetic construct
  MUTAGEN 1: note = X stands for 3-((carboxymethyl)amino)-propanoic acid
  MUTAGEN 3: note = X stands for (S)-2-amino-3-(6-hydroxy-1H-indol-3-yl)-propanoic acid
  MUTAGEN 5: note = X stands for (2S)-2-(methylamino)-3-phenyl-propanoic acid
  MUTAGEN 7: note = X stands for 2-(methylamino)-acetic acid
  MUTAGEN 8: note = X stands for (S)-2-amino-3-(3-(carboxymethoxy)phenyl)-propanoic acid
  MUTAGEN 9: note = X stands for (S)-2-amino-3-(4-methoxyphenyl)-propanoic acid
  MUTAGEN 11: note = X stands for (2S)-2-(methylamino)-3-phenyl-propanoic acid
  MUTAGEN 12: note = X stands for (S)-2-amino-decanoic acid
  MUTAGEN 13: note = X stands for (S)-3-amino-2-(methylamino)-propanoic acid
  MUTAGEN 14: note = X stands for (2S)-2-(methylamino)-3-phenyl-propanoic acid
  MUTAGEN 15: note = X stands for D-cysteine
XAXYXIXXXRXXXXX

SEQ ID NO: 251 - protein, 15 aa, synthetic construct
  MUTAGEN 1: note = X stands for 2-[(3-methoxypropyl)amino]-acetic acid
  MUTAGEN 3: note = X stands for (S)-2-amino-3-(6-hydroxy-1H-indol-3-yl)-propanoic acid
  MUTAGEN 5: note = X stands for (2S)-2-(methylamino)-3-phenyl-propanoic acid
  MUTAGEN 7: note = X stands for 2-(methylamino)-acetic acid
  MUTAGEN 8: note = X stands for (S)-2-amino-3-(3-(carboxymethoxy)phenyl)-propanoic acid
  MUTAGEN 9: note = X stands for (S)-2-amino-3-(4-methoxyphenyl)-propanoic acid
  MUTAGEN 11: note = X stands for (2S)-2-(methylamino)-3-phenyl-propanoic acid
  MUTAGEN 12: note = X stands for (S)-2-amino-decanoic acid
  MUTAGEN 13: note = X stands for (2S)-2-(methylamino)-propanoic acid
  MUTAGEN 14: note = X stands for (2S)-2-(methylamino)-3-phenyl-propanoic acid
  MUTAGEN 15: note = X stands for D-cysteine
XAXYXIXXXRXXXXX

SEQ ID NO: 252 - protein, 16 aa, synthetic construct
  MUTAGEN 1: note = X stands for (2S)-2-(methylamino)-pentanedioic acid
  MUTAGEN 3: note = X stands for (S)-2-amino-3-(6-hydroxy-1H-indol-3-yl)-propanoic acid
  MUTAGEN 5: note = X stands for (2S)-2-(methylamino)-3-phenyl-propanoic acid
  MUTAGEN 7: note = X stands for D-proline
  MUTAGEN 8: note = X stands for (S)-2-amino-3-(3-(carboxymethoxy)phenyl)-propanoic acid
  MUTAGEN 9: note = X stands for (S)-4-(2-amino-2-carboxyethyl)-benzoic acid
  MUTAGEN 11: note = X stands for (S)-3-(4-(aminomethyl)phenyl)-2-(methylamino)-propanoic acid
  MUTAGEN 12: note = X stands for (S)-2-amino-dodecanoic acid
  MUTAGEN 13: note = X stands for (2S)-2-(methylamino)-pentanedioic acid
  MUTAGEN 14: note = X stands for (2S)-2-(methylamino)-3-phenyl-propanoic acid
  MUTAGEN 15: note = X stands for D-cysteine
  MUTAGEN 16: note = X stands for 3-(piperidine-4-yl)-propanoic acid
XAXYXIXXXRXXXXXX

SEQ ID NO: 253 - protein, 15 aa, synthetic construct
  MUTAGEN 1: note = X stands for 3-((carboxymethyl)amino)-propanoic acid
  MUTAGEN 3: note = X stands for (S)-2-amino-3-(6-hydroxy-1H-indol-3-yl)-propanoic acid
  MUTAGEN 5: note = X stands for (2S)-2-(methylamino)-3-phenyl-propanoic acid
  MUTAGEN 7: note = X stands for 2-(methylamino)-acetic acid
  MUTAGEN 8: note = X stands for (S)-2-amino-3-(3-(carboxymethoxy)phenyl)-propanoic acid
  MUTAGEN 9: note = X stands for (S)-4-(2-amino-2-carboxyethyl)-benzoic acid
  MUTAGEN 11: note = X stands for (2S)-2-(methylamino)-3-phenyl-propanoic acid
  MUTAGEN 12: note = X stands for (S)-2-amino-decanoic acid
  MUTAGEN 13: note = X stands for (S)-3-amino-2-(methylamino)-propanoic acid
  MUTAGEN 14: note = X stands for (2S)-2-(methylamino)-3-phenyl-propanoic acid
  MUTAGEN 15: note = X stands for D-cysteine
XAXYXIXXXRXXXXX

SEQ ID NO: 254 - protein, 15 aa, synthetic construct
  MUTAGEN 1: note = X stands for 3-((carboxymethyl)amino)-propanoic acid
  MUTAGEN 3: note = X stands for 4-{3-[(2S)-2-amino-2-carboxyethyl]-1H-indole-1-yl}-benzoic acid
  MUTAGEN 5: note = X stands for (2S)-2-(methylamino)-3-phenyl-propanoic acid
  MUTAGEN 7: note = X stands for D-proline
  MUTAGEN 8: note = X stands for (S)-2-amino-3-(3-(carboxymethoxy)phenyl)-propanoic acid
  MUTAGEN 9: note = X stands for (S)-4-(2-amino-2-carboxyethyl)-benzoic acid
  MUTAGEN 11: note = X stands for (2S)-2-(methylamino)-3-phenyl-propanoic acid
  MUTAGEN 12: note = X stands for (S)-2-amino-nonanoic acid
  MUTAGEN 13: note = X stands for (S)-3-amino-2-(methylamino)-propanoic acid
  MUTAGEN 14: note = X stands for (2S)-2-(methylamino)-3-phenyl-propanoic acid
  MUTAGEN 15: note = X stands for D-cysteine
XAXYXIXXXRXXXXX

SEQ ID NO: 255 - protein, 15 aa, synthetic construct
  MUTAGEN 3: note = X stands for (S)-4-(3-(2-amino-2-carboxyetyl)-6-hydroxy-1H-indol-1-yl) benzoic acid
  MUTAGEN 5: note = X stands for (2S)-2-(methylamino)-3-phenyl-propanoic acid
  MUTAGEN 7: note = X stands for D-proline
  MUTAGEN 8: note = X stands for (S)-2-amino-3-(3-(carboxymethoxy)phenyl)-propanoic acid
  MUTAGEN 9: note = X stands for (S)-4-(2-amino-2-carboxyethyl)-benzoic acid
  MUTAGEN 11: note = X stands for (S)-3-(4-(aminomethyl)phenyl)-2-(methylamino)-propanoic acid
  MUTAGEN 12: note = X stands for (S)-2-amino-nonanoic acid
  MUTAGEN 13: note = X stands for (2S)-2-(methylamino)-propanoic acid
  MUTAGEN 14: note = X stands for (2S)-2-(methylamino)-3-phenyl-propanoic acid
  MUTAGEN 15: note = X stands for D-cysteine
EAXYXIXXXRXXXXX

SEQ ID NO: 256 - protein, 15 aa, synthetic construct
  MUTAGEN 1: note = X stands for (2S)-2-(methylamino)-pentanedioic acid
  MUTAGEN 3: note = X stands for 4-{3-[(2S)-2-amino-2-carboxyethyl]-1H-indole-1-yl}-benzoic acid
  MUTAGEN 5: note = X stands for (2S)-2-(methylamino)-3-phenyl-propanoic acid
  MUTAGEN 7: note = X stands for D-proline
  MUTAGEN 8: note = X stands for (S)-2-amino-3-(3-(carboxymethoxy)phenyl)-propanoic acid
  MUTAGEN 9: note = X stands for (S)-4-(2-amino-2-carboxyethyl)-benzoic acid
  MUTAGEN 11: note = X stands for (S)-3-(4-(aminomethyl)phenyl)-2-(methylamino)-propanoic acid
  MUTAGEN 12: note = X stands for (S)-2-amino-nonanoic acid
  MUTAGEN 13: note = X stands for (2S)-2-(methylamino)-propanoic acid
  MUTAGEN 14: note = X stands for (2S)-2-(methylamino)-3-phenyl-propanoic acid
  MUTAGEN 15: note = X stands for D-cysteine
XAXYXIXXXRXXXXX

SEQ ID NO: 257 - protein, 15 aa, synthetic construct
  MUTAGEN 1: note = X stands for (2S)-2-(methylamino)-pentanedioic acid
  MUTAGEN 3: note = X stands for 4-{3-[(2S)-2-amino-2-carboxyethyl]-1H-indole-1-yl}-benzoic acid
  MUTAGEN 5: note = X stands for (2S)-2-(methylamino)-3-phenyl-propanoic acid
  MUTAGEN 7: note = X stands for D-proline
  MUTAGEN 8: note = X stands for (S)-2-amino-3-(3-(carboxymethoxy)phenyl)-propanoic acid
  MUTAGEN 9: note = X stands for (S)-2-amino-3-(4-methoxyphenyl)-propanoic acid
  MUTAGEN 11: note = X stands for (S)-3-(4-(aminomethyl)phenyl)-2-(methylamino)-propanoic acid
  MUTAGEN 12: note = X stands for (S)-2-amino-nonanoic acid
  MUTAGEN 13: note = X stands for (2S)-2-(methylamino)-propanoic acid
  MUTAGEN 14: note = X stands for (2S)-2-(methylamino)-3-phenyl-propanoic acid
  MUTAGEN 15: note = X stands for D-cysteine
XAXYXIXXXRXXXXX

SEQ ID NO: 258 - protein, 15 aa, synthetic construct
  MUTAGEN 1: note = X stands for 3-((carboxymethyl)amino)-propanoic acid
  MUTAGEN 5: note = X stands for (2S)-2-(methylamino)-3-phenyl-propanoic acid
  MUTAGEN 7: note = X stands for (2S)-2-(methylamino)-propanoic acid
  MUTAGEN 8: note = X stands for (S)-2-amino-3-(3-(carboxymethoxy)phenyl)-propanoic acid
  MUTAGEN 9: note = X stands for (S)-4-(2-amino-2-carboxyethyl)-benzoic acid
  MUTAGEN 11: note = X stands for (2S)-2-(methylamino)-3-phenyl-propanoic acid
  MUTAGEN 12: note = X stands for (S)-2-amino-nonanoic acid
  MUTAGEN 13: note = X stands for (S)-3-amino-2-(methylamino)-propanoic acid
  MUTAGEN 14: note = X stands for (2S)-2-(methylamino)-3-phenyl-propanoic acid
  MUTAGEN 15: note = X stands for D-cysteine
XAWYXIXXXRXXXXX

SEQ ID NO: 259 - protein, 15 aa, synthetic construct
  MUTAGEN 1: note = X stands for 3-((carboxymethyl)amino)-propanoic acid
  MUTAGEN 5: note = X stands for (2S)-2-(methylamino)-3-phenyl-propanoic acid
  MUTAGEN 7: note = X stands for (2S)-2-(methylamino)-propanoic acid
  MUTAGEN 8: note = X stands for (S)-2-amino-3-(3-(carboxymethoxy)phenyl)-propanoic acid
  MUTAGEN 9: note = X stands for (S)-4-(2-amino-2-carboxyethyl)-benzoic acid
  MUTAGEN 11: note = X stands for (2S)-6-amino-2-(methylamino)-hexanoic acid
  MUTAGEN 12: note = X stands for (S)-2-amino-nonanoic acid
  MUTAGEN 13: note = X stands for (2S)-2-(methylamino)-propanoic acid
  MUTAGEN 14: note = X stands for (2S)-2-(methylamino)-3-phenyl-propanoic acid
  MUTAGEN 15: note = X stands for D-cysteine
XAWYXIXXXRXXXXX

SEQ ID NO: 260 - protein, 15 aa, synthetic construct
  MUTAGEN 1: note = X stands for 4-((carboxymethyl)amino)-butanoic acid
  MUTAGEN 5: note = X stands for (2S)-2-(methylamino)-3-phenyl-propanoic acid
  MUTAGEN 7: note = X stands for (2S)-2-(methylamino)-propanoic acid
  MUTAGEN 8: note = X stands for (S)-2-amino-3-(3-(carboxymethoxy)phenyl)-propanoic acid
  MUTAGEN 9: note = X stands for (S)-4-(2-amino-2-carboxyethyl)-benzoic acid
  MUTAGEN 11: note = X stands for (2S)-6-amino-2-(methylamino)-hexanoic acid
  MUTAGEN 12: note = X stands for (S)-2-amino-nonanoic acid
  MUTAGEN 13: note = X stands for (2S)-2-(methylamino)-propanoic acid
  MUTAGEN 14: note = X stands for (2S)-2-(methylamino)-3-phenyl-propanoic acid
  MUTAGEN 15: note = X stands for D-cysteine
XAWYXIXXXRXXXXX

SEQ ID NO: 261 - protein, 15 aa, synthetic construct
  MUTAGEN 1: note = X stands for 4-((carboxymethyl)amino)-butanoic acid
  MUTAGEN 5: note = X stands for (2S)-2-(methylamino)-3-phenyl-propanoic acid
  MUTAGEN 7: note = X stands for (2S)-2-(methylamino)-propanoic acid
  MUTAGEN 8: note = X stands for (S)-2-amino-3-(3-(carboxymethoxy)phenyl)-propanoic acid
  MUTAGEN 9: note = X stands for (S)-4-(2-amino-2-carboxyethyl)-benzoic acid
  MUTAGEN 11: note = X stands for (2S)-2,6-bis(methylamino)hexanoic acid
  MUTAGEN 12: note = X stands for (S)-2-amino-nonanoic acid
  MUTAGEN 13: note = X stands for (2S)-2-(methylamino)-propanoic acid
  MUTAGEN 14: note = X stands for (2S)-2-(methylamino)-3-phenyl-propanoic acid
  MUTAGEN 15: note = X stands for D-cysteine
XAWYXIXXXRXXXXX

SEQ ID NO: 262 - protein, 15 aa, synthetic construct
  MUTAGEN 1: note = X stands for 5-((carboxymethyl)amino)pentanoic acid
  MUTAGEN 5: note = X stands for (2S)-2-(methylamino)-3-phenyl-propanoic acid
  MUTAGEN 7: note = X stands for (2S)-2-(methylamino)-propanoic acid
  MUTAGEN 8: note = X stands for (S)-2-amino-3-(3-(carboxymethoxy)phenyl)-propanoic acid
  MUTAGEN 9: note = X stands for (S)-4-(2-amino-2-carboxyethyl)-benzoic acid
  MUTAGEN 11: note = X stands for (2S)-6-amino-2-(methylamino)-hexanoic acid
  MUTAGEN 12: note = X stands for (S)-2-amino-nonanoic acid
  MUTAGEN 13: note = X stands for (2S)-2-(methylamino)-propanoic acid
  MUTAGEN 14: note = X stands for (2S)-2-(methylamino)-3-phenyl-propanoic acid
  MUTAGEN 15: note = X stands for D-cysteine
XAWYXIXXXRXXXXX

SEQ ID NO: 263 - protein, 15 aa, synthetic construct
  MUTAGEN 1: note = X stands for 4-((carboxymethyl)amino)-butanoic acid
  MUTAGEN 5: note = X stands for (2S)-2-(methylamino)-3-phenyl-propanoic acid
  MUTAGEN 7: note = X stands for (2S)-2-(methylamino)-propanoic acid
  MUTAGEN 8: note = X stands for (S)-2-amino-3-(3-(carboxymethoxy)phenyl)-propanoic acid
  MUTAGEN 9: note = X stands for (S)-4-(2-amino-2-carboxyethyl)-benzoic acid
  MUTAGEN 11: note = X stands for (S)-3-(4-(aminomethyl)phenyl)-2-(methylamino)-propanoic acid
  MUTAGEN 12: note = X stands for (S)-2-amino-nonanoic acid
  MUTAGEN 13: note = X stands for (2S)-2-(methylamino)-propanoic acid
  MUTAGEN 14: note = X stands for (2S)-2-(methylamino)-3-phenyl-propanoic acid
  MUTAGEN 15: note = X stands for D-cysteine
XAWYXIXXXRXXXXX

SEQ ID NO: 264 - protein, 15 aa, synthetic construct
  MUTAGEN 1: note = X stands for 3-((carboxymethyl)amino)-propanoic acid
  MUTAGEN 5: note = X stands for (2S)-2-(methylamino)-3-phenyl-propanoic acid
  MUTAGEN 7: note = X stands for (2S)-2-(methylamino)-propanoic acid
  MUTAGEN 8: note = X stands for (S)-2-amino-3-(3-(carboxymethoxy)phenyl)-propanoic acid
  MUTAGEN 9: note = X stands for (S)-4-(2-amino-2-carboxyethyl)-benzoic acid
  MUTAGEN 11: note = X stands for (S)-3-(4-(aminomethyl)phenyl)-2-(methylamino)-propanoic acid
  MUTAGEN 12: note = X stands for (S)-2-amino-nonanoic acid
  MUTAGEN 13: note = X stands for (2S)-2-(methylamino)-propanoic acid
  MUTAGEN 14: note = X stands for (2S)-2-(methylamino)-3-phenyl-propanoic acid
  MUTAGEN 15: note = X stands for D-cysteine
XAWYXIXXXRXXXXX

SEQ ID NO: 265 - protein, 15 aa, synthetic construct
  MUTAGEN 5: note = X stands for (2S)-2-(methylamino)-3-phenyl-propanoic acid
  MUTAGEN 7: note = X stands for (2S)-2-(methylamino)-propanoic acid
  MUTAGEN 8: note = X stands for (S)-2-amino-3-(3-(carboxymethoxy)phenyl)-propanoic acid
  MUTAGEN 9: note = X stands for (S)-4-(2-amino-2-carboxyethyl)-benzoic acid
  MUTAGEN 11: note = X standards for (2S)-2-(methylamino)-butanedioic acid
  MUTAGEN 12: note = X stands for (S)-2-amino-nonanoic acid
  MUTAGEN 13: note = X stands for (2S)-2-(methylamino)-propanoic acid
  MUTAGEN 14: note = X stands for (2S)-2-(methylamino)-3-phenyl-propanoic acid
  MUTAGEN 15: note = X stands for D-cysteine
KAWYXIXXXRXXXXX

SEQ ID NO: 266 - protein, 15 aa, synthetic construct
  MUTAGEN 1: note = X stands for (2S)-2-amino-6-(methylamino)-hexanoic acid
  MUTAGEN 5: note = X stands for (2S)-2-(methylamino)-3-phenyl-propanoic acid
  MUTAGEN 7: note = X stands for (2S)-2-(methylamino)-propanoic acid
  MUTAGEN 8: note = X stands for (S)-2-amino-3-(3-(carboxymethoxy)phenyl)-propanoic acid
  MUTAGEN 9: note = X stands for (S)-4-(2-amino-2-carboxyethyl)-benzoic acid
  MUTAGEN 11: note = X standards for (2S)-2-(methylamino)-butanedioic acid
  MUTAGEN 12: note = X stands for (S)-2-amino-nonanoic acid
  MUTAGEN 13: note = X stands for (2S)-2-(methylamino)-propanoic acid
  MUTAGEN 14: note = X stands for (2S)-2-(methylamino)-3-phenyl-propanoic acid
  MUTAGEN 15: note = X stands for D-cysteine
XAWYXIXXXRXXXXX

SEQ ID NO: 267 - protein, 15 aa, synthetic construct
  MUTAGEN 5: note = X stands for (2S)-2-(methylamino)-3-phenyl-propanoic acid
  MUTAGEN 7: note = X stands for (2S)-2-(methylamino)-propanoic acid
  MUTAGEN 8: note = X stands for (S)-2-amino-3-(3-(carboxymethoxy)phenyl)-propanoic acid
  MUTAGEN 9: note = X stands for (S)-4-(2-amino-2-carboxyethyl)-benzoic acid
  MUTAGEN 11: note = X stands for (2S)-2-(methylamino)-pentanedioic acid
  MUTAGEN 12: note = X stands for (S)-2-amino-nonanoic acid
  MUTAGEN 13: note = X stands for (2S)-2-(methylamino)-propanoic acid
  MUTAGEN 14: note = X stands for (2S)-2-(methylamino)-3-phenyl-propanoic acid
  MUTAGEN 15: note = X stands for D-cysteine
KAWYXIXXXRXXXXX

SEQ ID NO: 268 - protein, 15 aa, synthetic construct
  MUTAGEN 1: note = X stands for (2S)-2,7-diamino-heptanoic acid
  MUTAGEN 5: note = X stands for (2S)-2-(methylamino)-3-phenyl-propanoic acid
  MUTAGEN 7: note = X stands for (2S)-2-(methylamino)-propanoic acid
  MUTAGEN 8: note = X stands for (S)-2-amino-3-(3-(carboxymethoxy)phenyl)-propanoic acid
  MUTAGEN 9: note = X stands for (S)-4-(2-amino-2-carboxyethyl)-benzoic acid
  MUTAGEN 11: note = X standards for (2S)-2-(methylamino)-butanedioic acid
  MUTAGEN 12: note = X stands for (S)-2-amino-nonanoic acid
  MUTAGEN 13: note = X stands for (2S)-2-(methylamino)-propanoic acid
  MUTAGEN 14: note = X stands for (2S)-2-(methylamino)-3-phenyl-propanoic acid
  MUTAGEN 15: note = X stands for D-cysteine
XAWYXIXXXRXXXXX

SEQ ID NO: 269 - protein, 15 aa, synthetic construct
  MUTAGEN 1: note = X stands for 4-((carboxymethyl)amino)-butanoic acid
  MUTAGEN 2: note = X stands for (2R)-2,4-diamino-butanoic acid
  MUTAGEN 5: note = X stands for (2S)-2-(methylamino)-3-phenyl-propanoic acid
  MUTAGEN 7: note = X stands for (2S)-2-(methylamino)-propanoic acid
  MUTAGEN 8: note = X stands for (S)-2-amino-3-(3-(carboxymethoxy)phenyl)-propanoic acid
  MUTAGEN 9: note = X stands for (S)-4-(2-amino-2-carboxyethyl)-benzoic acid
  MUTAGEN 11: note = X standards for (2S)-2-(methylamino)-butanedioic acid
  MUTAGEN 12: note = X stands for (S)-2-amino-nonanoic acid
  MUTAGEN 13: note = X stands for (2S)-2-(methylamino)-propanoic acid
  MUTAGEN 14: note = X stands for (2S)-2-(methylamino)-3-phenyl-propanoic acid
  MUTAGEN 15: note = X stands for D-cysteine
XXWYXIXXXRXXXXX

SEQ ID NO: 270 - protein, 15 aa, synthetic construct
  MUTAGEN 1: note = X stands for 4-((carboxymethyl)amino)-butanoic acid
  MUTAGEN 2: note = X stands for (2R)-2,5-diamino-pentanoic acid
  MUTAGEN 5: note = X stands for (2S)-2-(methylamino)-3-phenyl-propanoic acid
  MUTAGEN 7: note = X stands for (2S)-2-(methylamino)-propanoic acid
  MUTAGEN 8: note = X stands for (S)-2-amino-3-(3-(carboxymethoxy)phenyl)-propanoic acid
  MUTAGEN 9: note = X stands for (S)-4-(2-amino-2-carboxyethyl)-benzoic acid
  MUTAGEN 11: note = X standards for (2S)-2-(methylamino)-butanedioic acid
  MUTAGEN 12: note = X stands for (S)-2-amino-nonanoic acid
  MUTAGEN 13: note = X stands for (2S)-2-(methylamino)-propanoic acid
  MUTAGEN 14: note = X stands for (2S)-2-(methylamino)-3-phenyl-propanoic acid
  MUTAGEN 15: note = X stands for D-cysteine
XXWYXIXXXRXXXXX

SEQ ID NO: 271 - protein, 15 aa, synthetic construct
  MUTAGEN 1: note = X stands for 4-((carboxymethyl)amino)-butanoic acid
  MUTAGEN 2: note = X stands for (2R)-2,4-diamino-butanoic acid
  MUTAGEN 5: note = X stands for (2S)-2-(methylamino)-3-phenyl-propanoic acid
  MUTAGEN 7: note = X stands for (2S)-2-(methylamino)-propanoic acid
  MUTAGEN 8: note = X stands for (S)-2-amino-3-(3-(carboxymethoxy)phenyl)-propanoic acid
  MUTAGEN 9: note = X stands for (S)-4-(2-amino-2-carboxyethyl)-benzoic acid
  MUTAGEN 11: note = X stands for (2S)-2-(methylamino)-pentanedioic acid
  MUTAGEN 12: note = X stands for (S)-2-amino-nonanoic acid
  MUTAGEN 13: note = X stands for (2S)-2-(methylamino)-propanoic acid
  MUTAGEN 14: note = X stands for (2S)-2-(methylamino)-3-phenyl-propanoic acid
  MUTAGEN 15: note = X stands for D-cysteine
XXWYXIXXXRXXXXX

SEQ ID NO: 272 - protein, 15 aa, synthetic construct
  MUTAGEN 1: note = X stands for 4-((carboxymethyl)amino)-butanoic acid
  MUTAGEN 5: note = X stands for (2S)-2-(methylamino)-3-phenyl-propanoic acid
  MUTAGEN 7: note = X stands for (2S)-2-(methylamino)-propanoic acid
  MUTAGEN 8: note = X stands for (S)-2-amino-3-(3-(carboxymethoxy)phenyl)-propanoic acid
  MUTAGEN 9: note = X stands for (S)-4-(2-amino-2-carboxyethyl)-benzoic acid
  MUTAGEN 11: note = X stands for (2S)-2-(methylamino)-3-phenyl-propanoic acid
  MUTAGEN 12: note = X stands for (S)-2-amino-nonanoic acid
  MUTAGEN 13: note = X stands for (S)-3-amino-2-(methylamino)-propanoic acid
  MUTAGEN 14: note = X stands for (2S)-2-(methylamino)-3-phenyl-propanoic acid
  MUTAGEN 15: note = X stands for D-cysteine
XAWYXIXXXRXXXXX

SEQ ID NO: 273 - protein, 15 aa, synthetic construct
  MUTAGEN 1: note = X stands for 3-((carboxymethyl)amino)-propanoic acid
  MUTAGEN 5: note = X stands for (2S)-2-(methylamino)-3-phenyl-propanoic acid
  MUTAGEN 7: note = X stands for (2S)-2-(methylamino)-propanoic acid
  MUTAGEN 8: note = X stands for (S)-2-amino-3-(3-(carboxymethoxy)phenyl)-propanoic acid
  MUTAGEN 9: note = X stands for (S)-4-(2-amino-2-carboxyethyl)-benzoic acid
  MUTAGEN 11: note = X stands for (2S)-2-(methylamino)-3-phenyl-propanoic acid
  MUTAGEN 12: note = X stands for (S)-2-amino-nonanoic acid
  MUTAGEN 13: note = X stands for (S)-4-amino-2-(methylamino)-butanoic acid
  MUTAGEN 14: note = X stands for (2S)-2-(methylamino)-3-phenyl-propanoic acid
  MUTAGEN 15: note = X stands for D-cysteine
XAWYXIXXXRXXXXX

SEQ ID NO: 274 - protein, 15 aa, synthetic construct
  MUTAGEN 1: note = X stands for (2S)-2,3-diamino-propionic acid
  MUTAGEN 5: note = X stands for (2S)-2-(methylamino)-3-phenyl-propanoic acid
  MUTAGEN 7: note = X stands for (2S)-2-(methylamino)-propanoic acid
  MUTAGEN 8: note = X stands for (S)-2-amino-3-(3-(carboxymethoxy)phenyl)-propanoic acid
  MUTAGEN 9: note = X stands for (S)-4-(2-amino-2-carboxyethyl)-benzoic acid
  MUTAGEN 11: note = X stands for (2S)-2-(methylamino)-3-phenyl-propanoic acid
  MUTAGEN 12: note = X stands for (S)-2-amino-nonanoic acid
  MUTAGEN 13: note = X stands for (2S)-2-(methylamino)-pentanedioic acid
  MUTAGEN 14: note = X stands for (2S)-2-(methylamino)-3-phenyl-propanoic acid
  MUTAGEN 15: note = X stands for D-cysteine
XAWYXIXXXRXXXXX

SEQ ID NO: 275 - protein, 15 aa, synthetic construct
  MUTAGEN 5: note = X stands for (2S)-2-(methylamino)-3-phenyl-propanoic acid
  MUTAGEN 7: note = X stands for (2S)-2-(methylamino)-propanoic acid
  MUTAGEN 8: note = X stands for (S)-2-amino-3-(3-(carboxymethoxy)phenyl)-propanoic acid
  MUTAGEN 9: note = X stands for (S)-4-(2-amino-2-carboxyethyl)-benzoic acid
  MUTAGEN 11: note = X stands for (2S)-2-(methylamino)-3-phenyl-propanoic acid
  MUTAGEN 12: note = X stands for (S)-2-amino-nonanoic acid
  MUTAGEN 13: note = X stands for (S)-4-amino-2-(methylamino)-butanoic acid
  MUTAGEN 14: note = X stands for (2S)-2-(methylamino)-3-phenyl-propanoic acid
  MUTAGEN 15: note = X stands for D-cysteine
EAWYXIXXXRXXXXX

SEQ ID NO: 276 - protein, 15 aa, synthetic construct
  MUTAGEN 1: note = X stands for 4-((carboxymethyl)amino)-butanoic acid
  MUTAGEN 3: note = X stands for (2S)-2-amino-3-[1-(carboxymethyl)-1H-indol-3-yl]-propanoic acid
  MUTAGEN 5: note = X stands for (2S)-2-(methylamino)-3-phenyl-propanoic acid
  MUTAGEN 7: note = X stands for (2S)-2-(methylamino)-propanoic acid
  MUTAGEN 8: note = X stands for (S)-2-amino-3-(3-(carboxymethoxy)phenyl)-propanoic acid
  MUTAGEN 9: note = X stands for (S)-4-(2-amino-2-carboxyethyl)-benzoic acid
  MUTAGEN 11: note = X stands for (2S)-6-amino-2-(methylamino)-hexanoic acid
  MUTAGEN 12: note = X stands for (S)-2-amino-nonanoic acid
  MUTAGEN 13: note = X stands for (2S)-2-(methylamino)-propanoic acid
  MUTAGEN 14: note = X stands for (2S)-2-(methylamino)-3-phenyl-propanoic acid
  MUTAGEN 15: note = X stands for D-cysteine
XAXYXIXXXRXXXXX

SEQ ID NO: 277 - protein, 15 aa, synthetic construct
  MUTAGEN 1: note = X stands for (S)-2-amino-hexanedioic acid
  MUTAGEN 5: note = X stands for (2S)-2-(methylamino)-3-phenyl-propanoic acid
  MUTAGEN 7: note = X stands for (2S)-2-(methylamino)-propanoic acid
  MUTAGEN 8: note = X stands for (S)-2-amino-3-(3-(carboxymethoxy)phenyl)-propanoic acid
  MUTAGEN 9: note = X stands for (S)-4-(2-amino-2-carboxyethyl)-benzoic acid
  MUTAGEN 11: note = X stands for (S)-3-(4-(aminomethyl)phenyl)-2-(methylamino)-propanoic acid
  MUTAGEN 12: note = X stands for (S)-2-amino-nonanoic acid
  MUTAGEN 13: note = X stands for (2S)-2-(methylamino)-propanoic acid
  MUTAGEN 14: note = X stands for (2S)-2-(methylamino)-3-phenyl-propanoic acid
  MUTAGEN 15: note = X stands for D-cysteine
XAWYXIXXXRXXXXX

SEQ ID NO: 278 - protein, 15 aa, synthetic construct
  MUTAGEN 1: note = X stands for (2S)-2,5-diamino-pentanoic acid
  MUTAGEN 5: note = X stands for (2S)-2-(methylamino)-3-phenyl-propanoic acid
  MUTAGEN 7: note = X stands for (2S)-2-(methylamino)-propanoic acid
  MUTAGEN 8: note = X stands for (S)-2-amino-3-(3-(carboxymethoxy)phenyl)-propanoic acid
  MUTAGEN 9: note = X stands for (S)-4-(2-amino-2-carboxyethyl)-benzoic acid
  MUTAGEN 11: note = X stands for (S)-4-(2-carboxy-2-(methylamino)ethyl)-benzoic acid
  MUTAGEN 12: note = X stands for (S)-2-amino-nonanoic acid
  MUTAGEN 13: note = X stands for (2S)-2-(methylamino)-propanoic acid
  MUTAGEN 14: note = X stands for (2S)-2-(methylamino)-3-phenyl-propanoic acid
  MUTAGEN 15: note = X stands for D-cysteine
XAWYXIXXXRXXXXX

SEQ ID NO: 279 - protein, 15 aa, synthetic construct
  MUTAGEN 5: note = X stands for (2S)-2-(methylamino)-3-phenyl-propanoic acid
  MUTAGEN 7: note = X stands for (2S)-2-(methylamino)-propanoic acid
  MUTAGEN 8: note = X stands for (S)-2-amino-3-(3-(carboxymethoxy)phenyl)-propanoic acid
  MUTAGEN 9: note = X stands for (S)-4-(2-amino-2-carboxyethyl)-benzoic acid
  MUTAGEN 11: note = X stands for (S)-4-(2-carboxy-2-(methylamino)ethyl)-benzoic acid
  MUTAGEN 12: note = X stands for (S)-2-amino-nonanoic acid
  MUTAGEN 13: note = X stands for (2S)-2-(methylamino)-propanoic acid
  MUTAGEN 14: note = X stands for (2S)-2-(methylamino)-3-phenyl-propanoic acid
  MUTAGEN 15: note = X stands for D-cysteine
KAWYXIXXXRXXXXX

SEQ ID NO: 280 - protein, 15 aa, synthetic construct
  MUTAGEN 1: note = X stands for (2S)-2, 4-diamino-butanoic acid
  MUTAGEN 5: note = X stands for (2S)-2-(methylamino)-3-phenyl-propanoic acid
  MUTAGEN 7: note = X stands for (2S)-2-(methylamino)-propanoic acid
  MUTAGEN 8: note = X stands for (S)-2-amino-3-(3-(carboxymethoxy)phenyl)-propanoic acid
  MUTAGEN 9: note = X stands for (S)-4-(2-amino-2-carboxyethyl)-benzoic acid
  MUTAGEN 11: note = X stands for (S)-4-(2-carboxy-2-(methylamino)ethyl)-benzoic acid
  MUTAGEN 12: note = X stands for (S)-2-amino-nonanoic acid
  MUTAGEN 13: note = X stands for (2S)-2-(methylamino)-propanoic acid
  MUTAGEN 14: note = X stands for (2S)-2-(methylamino)-3-phenyl-propanoic acid
  MUTAGEN 15: note = X stands for D-cysteine
XAWYXIXXXRXXXXX

SEQ ID NO: 281 - protein, 15 aa, synthetic construct
  MUTAGEN 1: note = X stands for (2S)-2-amino-6-(methylamino)-hexanoic acid
  MUTAGEN 5: note = X stands for (2S)-2-(methylamino)-3-phenyl-propanoic acid
  MUTAGEN 7: note = X stands for (2S)-2-(methylamino)-propanoic acid
  MUTAGEN 8: note = X stands for (S)-2-amino-3-(3-(carboxymethoxy)phenyl)-propanoic acid
  MUTAGEN 9: note = X stands for (S)-4-(2-amino-2-carboxyethyl)-benzoic acid
  MUTAGEN 11: note = X stands for (S)-4-(2-carboxy-2-(methylamino)ethyl)-benzoic acid
  MUTAGEN 12: note = X stands for (S)-2-amino-nonanoic acid
  MUTAGEN 13: note = X stands for (2S)-2-(methylamino)-propanoic acid
  MUTAGEN 14: note = X stands for (2S)-2-(methylamino)-3-phenyl-propanoic acid
  MUTAGEN 15: note = X stands for D-cysteine
XAWYXIXXXRXXXXX

SEQ ID NO: 282 - protein, 15 aa, synthetic construct
  MUTAGEN 5: note = X stands for (2S)-2-(methylamino)-3-phenyl-propanoic acid
  MUTAGEN 7: note = X stands for (2S)-2-(methylamino)-propanoic acid
  MUTAGEN 8: note = X stands for (S)-2-amino-3-(3-(carboxymethoxy)phenyl)-propanoic acid
  MUTAGEN 9: note = X stands for (S)-4-(2-amino-2-carboxyethyl)-benzoic acid
  MUTAGEN 11: note = X stands for (S)-2-amino-3-(4-(aminomethyl)phenyl)propionic acd
  MUTAGEN 12: note = X stands for (S)-2-amino-nonanoic acid
  MUTAGEN 13: note = X stands for (2S)-2-(methylamino)-propanoic acid
  MUTAGEN 14: note = X stands for (2S)-2-(methylamino)-3-phenyl-propanoic acid
  MUTAGEN 15: note = X stands for D-cysteine
EAWYXIXXXRXXXXX

SEQ ID NO: 283 - protein, 15 aa, synthetic construct
  MUTAGEN 1: note = X stands for (2S)-2-(methylamino)-pentanedioic acid
  MUTAGEN 5: note = X stands for (2S)-2-(methylamino)-3-phenyl-propanoic acid
  MUTAGEN 7: note = X stands for (2S)-2-(methylamino)-propanoic acid
  MUTAGEN 8: note = X stands for (S)-2-amino-3-(3-(carboxymethoxy)phenyl)-propanoic acid
  MUTAGEN 9: note = X stands for (S)-4-(2-amino-2-carboxyethyl)-benzoic acid
  MUTAGEN 11: note = X stands for (S)-3-(4-(aminomethyl)phenyl)-2-(methylamino)-propanoic acid
  MUTAGEN 12: note = X stands for (S)-2-amino-nonanoic acid
  MUTAGEN 13: note = X stands for (2S)-2-(methylamino)-propanoic acid
  MUTAGEN 14: note = X stands for (2S)-2-(methylamino)-3-phenyl-propanoic acid
  MUTAGEN 15: note = X stands for D-cysteine
XAWYXIXXXRXXXXX

SEQ ID NO: 284 - protein, 15 aa, synthetic construct
  MUTAGEN 2: note = X stands for D-alanine
  MUTAGEN 5: note = X stands for (2S)-2-(methylamino)-3-phenyl-propanoic acid
  MUTAGEN 7: note = X stands for (2S)-2-(methylamino)-propanoic acid
  MUTAGEN 8: note = X stands for (S)-2-amino-3-(3-(carboxymethoxy)phenyl)-propanoic acid
  MUTAGEN 9: note = X stands for (S)-4-(2-amino-2-carboxyethyl)-benzoic acid
  MUTAGEN 11: note = X stands for (S)-3-(4-(aminomethyl)phenyl)-2-(methylamino)-propanoic acid
  MUTAGEN 12: note = X stands for (S)-2-amino-nonanoic acid
  MUTAGEN 13: note = X stands for (2S)-2-(methylamino)-propanoic acid
  MUTAGEN 14: note = X stands for (2S)-2-(methylamino)-3-phenyl-propanoic acid
  MUTAGEN 15: note = X stands for D-cysteine
EXWYXIXXXRXXXXX

SEQ ID NO: 285 - protein, 15 aa, synthetic construct
  MUTAGEN 5: note = X stands for (2S)-2-(methylamino)-3-phenyl-propanoic acid
  MUTAGEN 7: note = X stands for 2-(methylamino)-acetic acid
  MUTAGEN 8: note = X stands for (S)-2-amino-3-(3-(carboxymethoxy)phenyl)-propanoic acid
  MUTAGEN 9: note = X stands for (S)-4-(2-amino-2-carboxyethyl)-benzoic acid
  MUTAGEN 11: note = X stands for (S)-3-(4-(aminomethyl)phenyl)-2-(methylamino)-propanoic acid
  MUTAGEN 12: note = X stands for (S)-2-amino-decanoic acid
  MUTAGEN 13: note = X stands for (2S)-2-(methylamino)-pentanedioic acid
  MUTAGEN 14: note = X stands for (2S)-2-(methylamino)-3-phenyl-propanoic acid
  MUTAGEN 15: note = X stands for D-cysteine
EAWYXIXXXRXXXXX

SEQ ID NO: 286 - protein, 15 aa, synthetic construct
  MUTAGEN 5: note = X stands for (2S)-2-(methylamino)-3-phenyl-propanoic acid
  MUTAGEN 7: note = X stands for 2-(methylamino)-acetic acid
  MUTAGEN 8: note = X stands for (S)-2-amino-3-(3-(carboxymethoxy)phenyl)-propanoic acid
  MUTAGEN 9: note = X stands for (S)-4-(2-amino-2-carboxyethyl)-benzoic acid
  MUTAGEN 11: note = X stands for (S)-3-(4-(aminomethyl)phenyl)-2-(methylamino)-propanoic acid
  MUTAGEN 12: note = X stands for (S)-2-amino-undecanoic acid
  MUTAGEN 13: note = X stands for (2S)-2-(methylamino)-pentanedioic acid
  MUTAGEN 14: note = X stands for (2S)-2-(methylamino)-3-phenyl-propanoic acid
  MUTAGEN 15: note = X stands for D-cysteine
EAWYXIXXXRXXXXX

SEQ ID NO: 287 - protein, 15 aa, synthetic construct
  MUTAGEN 5: note = X stands for (2S)-2-(methylamino)-3-phenyl-propanoic acid
  MUTAGEN 7: note = X stands for 2-(methylamino)-acetic acid
  MUTAGEN 8: note = X stands for (S)-2-amino-3-(3-(carboxymethoxy)phenyl)-propanoic acid
  MUTAGEN 9: note = X stands for (S)-4-(2-amino-2-carboxyethyl)-benzoic acid
  MUTAGEN 11: note = X stands for (S)-3-(4-(aminomethyl)phenyl)-2-(methylamino)-propanoic acid
  MUTAGEN 12: note = X stands for (S)-2-amino-dodecanoic acid
  MUTAGEN 13: note = X stands for (2S)-2-(methylamino)-pentanedioic acid
  MUTAGEN 14: note = X stands for (2S)-2-(methylamino)-3-phenyl-propanoic acid
  MUTAGEN 15: note = X stands for D-cysteine
EAWYXIXXXRXXXXX

SEQ ID NO: 288 - protein, 15 aa, synthetic construct
  MUTAGEN 1: note = X stands for 2-[(3-methoxypropyl)amino]-acetic acid
  MUTAGEN 3: note = X stands for (S)-2-amino-3-(6-hydroxy-1H-indol-3-yl)-propanoic acid
  MUTAGEN 5: note = X stands for (2S)-2-(methylamino)-3-phenyl-propanoic acid
  MUTAGEN 7: note = X stands for 2-(methylamino)-acetic acid
  MUTAGEN 8: note = X stands for (S)-2-amino-3-(3-(carboxymethoxy)phenyl)-propanoic acid
  MUTAGEN 9: note = X stands for (S)-4-(2-amino-2-carboxyethyl)-benzoic acid
  MUTAGEN 11: note = X stands for (2S)-2-(methylamino)-3-phenyl-propanoic acid
  MUTAGEN 12: note = X stands for (S)-2-amino-decanoic acid
  MUTAGEN 13: note = X stands for (2S)-2-(methylamino)-propanoic acid
  MUTAGEN 14: note = X stands for (2S)-2-(methylamino)-3-phenyl-propanoic acid
  MUTAGEN 15: note = X stands for D-cysteine
XAXYXIXXXRXXXXX

SEQ ID NO: 289 - protein, 15 aa, synthetic construct
  MUTAGEN 1: note = X stands for (2S)-2-(methylamino)-pentanedioic acid
  MUTAGEN 3: note = X stands for (S)-2-amino-3-(6-hydroxy-1H-indol-3-yl)-propanoic acid
  MUTAGEN 5: note = X stands for (2S)-2-(methylamino)-3-phenyl-propanoic acid
  MUTAGEN 7: note = X stands for 2-(methylamino)-acetic acid
  MUTAGEN 8: note = X stands for (S)-2-amino-3-(3-(carboxymethoxy)phenyl)-propanoic acid
  MUTAGEN 9: note = X stands for (S)-4-(2-amino-2-carboxyethyl)-benzoic acid
  MUTAGEN 11: note = X stands for (S)-3-(4-(aminomethyl)phenyl)-2-(methylamino)-propanoic acid
  MUTAGEN 12: note = X stands for (S)-2-amino-decanoic acid
  MUTAGEN 13: note = X stands for (2S)-2-(methylamino)-propanoic acid
  MUTAGEN 14: note = X stands for (2S)-2-(methylamino)-3-phenyl-propanoic acid
  MUTAGEN 15: note = X stands for D-cysteine
XAXYXIXXXRXXXXX

SEQ ID NO: 290 - protein, 15 aa, synthetic construct
  MUTAGEN 1: note = X stands for (2S)-2-(methylamino)-pentanedioic acid
  MUTAGEN 3: note = X stands for 4-{3-[(2S)-2-amino-2-carboxyethyl]-1H-indole-1-yl}-benzoic acid
  MUTAGEN 5: note = X stands for (2S)-2-(methylamino)-3-phenyl-propanoic acid
  MUTAGEN 7: note = X stands for D-proline
  MUTAGEN 8: note = X stands for (S)-2-amino-3-(3-(carboxymethoxy)phenyl)-propanoic acid
  MUTAGEN 9: note = X stands for (S)-4-(2-amino-2-carboxyethyl)-benzoic acid
  MUTAGEN 11: note = X stands for (S)-3-(4-(aminomethyl)phenyl)-2-(methylamino)-propanoic acid
  MUTAGEN 12: note = X stands for (S)-2-amino-nonanoic acid
  MUTAGEN 13: note = X stands for (2S)-2-(methylamino)-propanoic acid
  MUTAGEN 14: note = X stands for (2S)-2-(methylamino)-3-phenyl-propanoic acid
  MUTAGEN 15: note = X stands for D-cysteine
XAXYXIXXXRXXXXX

SEQ ID NO: 291 - protein, 15 aa, synthetic construct
  MUTAGEN 1: note = X stands for 4-((carboxymethyl)amino)-butanoic acid
  MUTAGEN 5: note = X stands for (2S)-2-(methylamino)-3-phenyl-propanoic acid
  MUTAGEN 7: note = X stands for (2S)-2-(methylamino)-propanoic acid
  MUTAGEN 8: note = X stands for (S)-2-amino-3-(3-(carboxymethoxy)phenyl)-propanoic acid
  MUTAGEN 9: note = X stands for (S)-4-(2-amino-2-carboxyethyl)-benzoic acid
  MUTAGEN 11: note = X stands for (2S)-2-(methylamino)-3-phenyl-propanoic acid
  MUTAGEN 12: note = X stands for (S)-2-amino-nonanoic acid
  MUTAGEN 13: note = X stands for (2S)-2-(methylamino)-propanoic acid
  MUTAGEN 14: note = X stands for (2S)-2-(methylamino)-3-phenyl-propanoic acid
  MUTAGEN 15: note = X stands for (R)-2-amino-hexanedioic acid
XAWYXIXXXRXXXXX

SEQ ID NO: 292 - protein, 15 aa, synthetic construct
  MUTAGEN 1: note = X stands for 4-((carboxymethyl)amino)-butanoic acid
  MUTAGEN 5: note = X stands for (2S)-2-(methylamino)-3-phenyl-propanoic acid
  MUTAGEN 7: note = X stands for (2S)-2-(methylamino)-propanoic acid
  MUTAGEN 8: note = X stands for (S)-2-amino-3-(3-(carboxymethoxy)phenyl)-propanoic acid
  MUTAGEN 9: note = X stands for (S)-4-(2-amino-2-carboxyethyl)-benzoic acid
  MUTAGEN 11: note = X stands for (2S)-2-(methylamino)-3-phenyl-propanoic acid
  MUTAGEN 12: note = X stands for (S)-2-amino-nonanoic acid
  MUTAGEN 13: note = X stands for (2S)-2-(methylamino)-propanoic acid
  MUTAGEN 14: note = X stands for (2S)-2-(methylamino)-3-phenyl-propanoic acid
  MUTAGEN 15: note = X stands for (S)-2-amino-hexanedioic acid
XAWYXIXXXRXXXXX

SEQ ID NO: 293 - protein, 15 aa, synthetic construct
  MUTAGEN 1: note = X stands for 4-((carboxymethyl)amino)-butanoic acid
  MUTAGEN 5: note = X stands for (2S)-2-(methylamino)-3-phenyl-propanoic acid
  MUTAGEN 7: note = X stands for (2S)-2-(methylamino)-propanoic acid
  MUTAGEN 8: note = X stands for (S)-2-amino-3-(3-(carboxymethoxy)phenyl)-propanoic acid
  MUTAGEN 9: note = X stands for (S)-4-(2-amino-2-carboxyethyl)-benzoic acid
  MUTAGEN 11: note = X stands for (2S)-2-(methylamino)-3-phenyl-propanoic acid
  MUTAGEN 12: note = X stands for (S)-2-amino-nonanoic acid
  MUTAGEN 13: note = X stands for (2S)-2-(methylamino)-propanoic acid
  MUTAGEN 14: note = X stands for (2S)-2-(methylamino)-3-phenyl-propanoic acid
  MUTAGEN 15: note = X stands for (S)-2-(methylamino)-hexanedioic acid
XAWYXIXXXRXXXXX

SEQ ID NO: 294 - protein, 15 aa, synthetic construct
  MUTAGEN 1: note = X stands for 4-((carboxymethyl)amino)-butanoic acid
  MUTAGEN 5: note = X stands for (2S)-2-(methylamino)-3-phenyl-propanoic acid
  MUTAGEN 7: note = X stands for (2S)-2-(methylamino)-propanoic acid
  MUTAGEN 8: note = X stands for (S)-2-amino-3-(3-(carboxymethoxy)phenyl)-propanoic acid
  MUTAGEN 9: note = X stands for (S)-4-(2-amino-2-carboxyethyl)-benzoic acid
  MUTAGEN 11: note = X stands for (2S)-2-(methylamino)-3-phenyl-propanoic acid
  MUTAGEN 12: note = X stands for (S)-2-amino-nonanoic acid
  MUTAGEN 13: note = X stands for (2S)-2-(methylamino)-propanoic acid
  MUTAGEN 14: note = X stands for (2S)-2-(methylamino)-3-phenyl-propanoic acid
  MUTAGEN 15: note = X stands for (R)-2-(methylamino)-hexanedioic acid
XAWYXIXXXRXXXXX

SEQ ID NO: 295 - protein, 16 aa, synthetic construct
  MUTAGEN 1: note = X stands for 4-((carboxymethyl)amino)-butanoic acid
  MUTAGEN 5: note = X stands for (2S)-2-(methylamino)-3-phenyl-propanoic acid
  MUTAGEN 7: note = X stands for (2S)-2-(methylamino)-propanoic acid
  MUTAGEN 8: note = X stands for (S)-2-amino-3-(3-(carboxymethoxy)phenyl)-propanoic acid
  MUTAGEN 9: note = X stands for (S)-4-(2-amino-2-carboxyethyl)-benzoic acid
  MUTAGEN 11: note = X stands for (2S)-2-(methylamino)-3-phenyl-propanoic acid
  MUTAGEN 12: note = X stands for (S)-2-amino-nonanoic acid
  MUTAGEN 13: note = X stands for (2S)-2-(methylamino)-propanoic acid
  MUTAGEN 14: note = X stands for (2S)-2-(methylamino)-3-phenyl-propanoic acid
  MUTAGEN 16: note = X stands for (2S)-2-(methylamino)-propanoic acid
XAWYXIXXXRXXXXGX

SEQ ID NO: 296 - protein, 16 aa, synthetic construct
  MUTAGEN 1: note = X stands for 4-((carboxymethyl)amino)-butanoic acid
  MUTAGEN 5: note = X stands for (2S)-2-(methylamino)-3-phenyl-propanoic acid
  MUTAGEN 7: note = X stands for (2S)-2-(methylamino)-propanoic acid
  MUTAGEN 8: note = X stands for (S)-2-amino-3-(3-(carboxymethoxy)phenyl)-propanoic acid
  MUTAGEN 9: note = X stands for (S)-4-(2-amino-2-carboxyethyl)-benzoic acid
  MUTAGEN 11: note = X stands for (2S)-2-(methylamino)-3-phenyl-propanoic acid
  MUTAGEN 12: note = X stands for (S)-2-amino-nonanoic acid
  MUTAGEN 13: note = X stands for (2S)-2-(methylamino)-propanoic acid
  MUTAGEN 14: note = X stands for (2S)-2-(methylamino)-3-phenyl-propanoic acid
  MUTAGEN 16: note = X stands for (2R)-2-(methylamino)-propanoic acid
XAWYXIXXXRXXXXGX

SEQ ID NO: 297 - protein, 16 aa, synthetic construct
  MUTAGEN 1: note = X stands for 4-((carboxymethyl)amino)-butanoic acid
  MUTAGEN 5: note = X stands for (2S)-2-(methylamino)-3-phenyl-propanoic acid
  MUTAGEN 7: note = X stands for (2S)-2-(methylamino)-propanoic acid
  MUTAGEN 8: note = X stands for (S)-2-amino-3-(3-(carboxymethoxy)phenyl)-propanoic acid
  MUTAGEN 9: note = X stands for (S)-4-(2-amino-2-carboxyethyl)-benzoic acid
  MUTAGEN 11: note = X stands for (2S)-2-(methylamino)-3-phenyl-propanoic acid
  MUTAGEN 12: note = X stands for (S)-2-amino-nonanoic acid
  MUTAGEN 13: note = X stands for (2S)-2-(methylamino)-propanoic acid
  MUTAGEN 14: note = X stands for (2S)-2-(methylamino)-3-phenyl-propanoic acid
  MUTAGEN 15: note = X stands for D-alanine
XAWYXIXXXRXXXXXG

SEQ ID NO: 298 - protein, 16 aa, synthetic construct
  MUTAGEN 1: note = X stands for 4-((carboxymethyl)amino)-butanoic acid
  MUTAGEN 5: note = X stands for (2S)-2-(methylamino)-3-phenyl-propanoic acid
  MUTAGEN 7: note = X stands for (2S)-2-(methylamino)-propanoic acid
  MUTAGEN 8: note = X stands for (S)-2-amino-3-(3-(carboxymethoxy)phenyl)-propanoic acid
  MUTAGEN 9: note = X stands for (S)-4-(2-amino-2-carboxyethyl)-benzoic acid
  MUTAGEN 11: note = X stands for (2S)-2-(methylamino)-3-phenyl-propanoic acid
  MUTAGEN 12: note = X stands for (S)-2-amino-nonanoic acid
  MUTAGEN 13: note = X stands for (2S)-2-(methylamino)-propanoic acid
  MUTAGEN 14: note = X stands for (2S)-2-(methylamino)-3-phenyl-propanoic acid
  MUTAGEN 16: note = X stands for D-alanine
XAWYXIXXXRXXXXAX

SEQ ID NO: 299 - protein, 16 aa, synthetic construct
  MUTAGEN 1: note = X stands for 4-((carboxymethyl)amino)-butanoic acid
  MUTAGEN 5: note = X stands for (2S)-2-(methylamino)-3-phenyl-propanoic acid
  MUTAGEN 7: note = X stands for (2S)-2-(methylamino)-propanoic acid
  MUTAGEN 8: note = X stands for (S)-2-amino-3-(3-(carboxymethoxy)phenyl)-propanoic acid
  MUTAGEN 9: note = X stands for (S)-4-(2-amino-2-carboxyethyl)-benzoic acid
  MUTAGEN 11: note = X stands for (2S)-2-(methylamino)-3-phenyl-propanoic acid
  MUTAGEN 12: note = X stands for (S)-2-amino-nonanoic acid
  MUTAGEN 13: note = X stands for (2S)-2-(methylamino)-propanoic acid
  MUTAGEN 14: note = X stands for (2S)-2-(methylamino)-3-phenyl-propanoic acid
  MUTAGEN 16: note = X stands for 2-(methylamino)-acetic acid
XAWYXIXXXRXXXXAX

SEQ ID NO: 300 - protein, 16 aa, synthetic construct
  MUTAGEN 1: note = X stands for 4-((carboxymethyl)amino)-butanoic acid
  MUTAGEN 5: note = X stands for (2S)-2-(methylamino)-3-phenyl-propanoic acid
  MUTAGEN 7: note = X stands for (2S)-2-(methylamino)-propanoic acid
  MUTAGEN 8: note = X stands for (S)-2-amino-3-(3-(carboxymethoxy)phenyl)-propanoic acid
  MUTAGEN 9: note = X stands for (S)-4-(2-amino-2-carboxyethyl)-benzoic acid
  MUTAGEN 11: note = X stands for (2S)-2-(methylamino)-3-phenyl-propanoic acid
  MUTAGEN 12: note = X stands for (S)-2-amino-nonanoic acid
  MUTAGEN 13: note = X stands for (2S)-2-(methylamino)-propanoic acid
  MUTAGEN 14: note = X stands for (2S)-2-(methylamino)-3-phenyl-propanoic acid
  MUTAGEN 15: note = X stands for D-alanine
  MUTAGEN 16: note = X stands for 2-(methylamino)-acetic acid
XAWYXIXXXRXXXXXX

SEQ ID NO: 301 - protein, 16 aa, synthetic construct
  MUTAGEN 1: note = X stands for 4-((carboxymethyl)amino)-butanoic acid
  MUTAGEN 5: note = X stands for (2S)-2-(methylamino)-3-phenyl-propanoic acid
  MUTAGEN 7: note = X stands for (2S)-2-(methylamino)-propanoic acid
  MUTAGEN 8: note = X stands for (S)-2-amino-3-(3-(carboxymethoxy)phenyl)-propanoic acid
  MUTAGEN 9: note = X stands for (S)-4-(2-amino-2-carboxyethyl)-benzoic acid
  MUTAGEN 11: note = X stands for (2S)-2-(methylamino)-3-phenyl-propanoic acid
  MUTAGEN 12: note = X stands for (S)-2-amino-nonanoic acid
  MUTAGEN 13: note = X stands for (2S)-2-(methylamino)-propanoic acid
  MUTAGEN 14: note = X stands for (2S)-2-(methylamino)-3-phenyl-propanoic acid
XAWYXIXXXRXXXXGG

SEQ ID NO: 302 - protein, 16 aa, synthetic construct
  MUTAGEN 1: note = X stands for 4-((carboxymethyl)amino)-butanoic acid
  MUTAGEN 5: note = X stands for (2S)-2-(methylamino)-3-phenyl-propanoic acid
  MUTAGEN 7: note = X stands for (2S)-2-(methylamino)-propanoic acid
  MUTAGEN 8: note = X stands for (S)-2-amino-3-(3-(carboxymethoxy)phenyl)-propanoic acid
  MUTAGEN 9: note = X stands for (S)-4-(2-amino-2-carboxyethyl)-benzoic acid
  MUTAGEN 11: note = X stands for (2S)-2-(methylamino)-3-phenyl-propanoic acid
  MUTAGEN 12: note = X stands for (S)-2-amino-nonanoic acid
  MUTAGEN 13: note = X stands for (2S)-2-(methylamino)-propanoic acid
  MUTAGEN 14: note = X stands for (2S)-2-(methylamino)-3-phenyl-propanoic acid
  MUTAGEN 15: note = X stands for D-alanine
  MUTAGEN 16: note = X stands for (2S)-2-(methylamino)-propanoic acid
XAWYXIXXXRXXXXXX

SEQ ID NO: 303 - protein, 16 aa, synthetic construct
  MUTAGEN 1: note = X stands for 4-((carboxymethyl)amino)-butanoic acid
  MUTAGEN 5: note = X stands for (2S)-2-(methylamino)-3-phenyl-propanoic acid
  MUTAGEN 7: note = X stands for (2S)-2-(methylamino)-propanoic acid
  MUTAGEN 8: note = X stands for (S)-2-amino-3-(3-(carboxymethoxy)phenyl)-propanoic acid
  MUTAGEN 9: note = X stands for (S)-4-(2-amino-2-carboxyethyl)-benzoic acid
  MUTAGEN 11: note = X stands for (2S)-2-(methylamino)-3-phenyl-propanoic acid
  MUTAGEN 12: note = X stands for (S)-2-amino-nonanoic acid
  MUTAGEN 13: note = X stands for (2S)-2-(methylamino)-propanoic acid
  MUTAGEN 14: note = X stands for (2S)-2-(methylamino)-3-phenyl-propanoic acid
XAWYXIXXXRXXXXGP

SEQ ID NO: 304 - protein, 16 aa, synthetic construct
  MUTAGEN 1: note = X stands for 4-((carboxymethyl)amino)-butanoic acid
  MUTAGEN 5: note = X stands for (2S)-2-(methylamino)-3-phenyl-propanoic acid
  MUTAGEN 7: note = X stands for (2S)-2-(methylamino)-propanoic acid
  MUTAGEN 8: note = X stands for (S)-2-amino-3-(3-(carboxymethoxy)phenyl)-propanoic acid
  MUTAGEN 9: note = X stands for (S)-4-(2-amino-2-carboxyethyl)-benzoic acid
  MUTAGEN 11: note = X stands for (2S)-2-(methylamino)-3-phenyl-propanonic acid
  MUTAGEN 12: note = X stands for (S)-2-amino-nonanoic acid
  MUTAGEN 13: note = X stands for (2S)-2-(methylamino)-propanoic acid
  MUTAGEN 14: note = X stands for (2S)-2-(methylamino)-3-phenyl-propanoic acid
XAWYXIXXXRXXXXAG

SEQ ID NO: 305 - protein, 16 aa, synthetic construct
  MUTAGEN 1: note = X stands for 4-((carboxymethyl)amino)-butanoic acid
  MUTAGEN 5: note = X stands for (2S)-2-(methylamino)-3-phenyl-propanoic acid
  MUTAGEN 7: note = X stands for (2S)-2-(methylamino)-propanoic acid
  MUTAGEN 8: note = X stands for (S)-2-amino-3-(3-(carboxymethoxy)phenyl)-propanoic acid
  MUTAGEN 9: note = X stands for (S)-4-(2-amino-2-carboxyethyl)-benzoic acid
  MUTAGEN 11: note = X stands for (2S)-2-(methylamino)-3-phenyl-propanoic acid
  MUTAGEN 12: note = X stands for (S)-2-amino-nonanoic acid
  MUTAGEN 13: note = X stands for (2S)-2-(methylamino)-propanoic acid
  MUTAGEN 14: note = X stands for (2S)-2-(methylamino)-3-phenyl-propanoic acid
  MUTAGEN 16: note = X stands for (2R)-2-(methylamino)-propanoic acid
XAWYXIXXXRXXXXAX

SEQ ID NO: 306 - protein, 16 aa, synthetic construct
  MUTAGEN 1: note = X stands for 4-((carboxymethyl)amino)-butanoic acid
  MUTAGEN 5: note = X stands for (2S)-2-(methylamino)-3-phenyl-propanoic acid
  MUTAGEN 7: note = X stands for (2S)-2-(methylamino)-propanoic acid
  MUTAGEN 8: note = X stands for (S)-2-amino-3-(3-(carboxymethoxy)phenyl)-propanoic acid
  MUTAGEN 9: note = X stands for (S)-4-(2-amino-2-carboxyethyl)-benzoic acid
  MUTAGEN 11: note = X stands for (2S)-2-(methylamino)-3-phenyl-propanoic acid
  MUTAGEN 12: note = X stands for (S)-2-amino-nonanoic acid
  MUTAGEN 13: note = X stands for (2S)-2-(methylamino)-propanoic acid
  MUTAGEN 14: note = X stands for (2S)-2-(methylamino)-3-phenyl-propanoic acid
  MUTAGEN 15: note = X stands for D-alanine
XAWYXIXXXRXXXXXA

SEQ ID NO: 307 - protein, 16 aa, synthetic construct
  MUTAGEN 1: note = X stands for (2S)-2-(methylamino)-propanoic acid
  MUTAGEN 5: note = X stands for (2S)-2-(methylamino)-3-phenyl-propanoic acid
  MUTAGEN 7: note = X stands for (2S)-2-(methylamino)-propanoic acid
  MUTAGEN 8: note = X stands for (S)-2-amino-3-(3-(carboxymethoxy)phenyl)-propanoic acid
  MUTAGEN 9: note = X stands for (S)-4-(2-amino-2-carboxyethyl)-benzoic acid
  MUTAGEN 11: note = X stands for (2S)-2-(methylamino)-3-phenyl-propanoic acid
  MUTAGEN 12: note = X stands for (S)-2-amino-nonanoic acid
  MUTAGEN 13: note = X stands for (2S)-2-(methylamino)-propanoic acid
  MUTAGEN 14: note = X stands for (2S)-2-(methylamino)-3-phenyl-propanoic acid
  MUTAGEN 16: note = X stands for (2S)-2-(methylamino)-propanoic acid
XAWYXIXXXRXXXXGX

SEQ ID NO: 308 - protein, 16 aa, synthetic construct
  MUTAGEN 1: note = X stands for (2S)-2-(methylamino)-propanoic acid
  MUTAGEN 5: note = X stands for (2S)-2-(methylamino)-3-phenyl-propanoic acid
  MUTAGEN 7: note = X stands for (2S)-2-(methylamino)-propanoic acid
  MUTAGEN 8: note = X stands for (S)-2-amino-3-(3-(carboxymethoxy)phenyl)-propanoic acid
  MUTAGEN 9: note = X stands for (S)-4-(2-amino-2-carboxyethyl)-benzoic acid
  MUTAGEN 11: note = X stands for (2S)-2-(methylamino)-3-phenyl-propanoic acid
  MUTAGEN 12: note = X stands for (S)-2-amino-nonanoic acid
  MUTAGEN 13: note = X stands for (2S)-2-(methylamino)-propanoic acid
  MOTIF 14: note = X stands for (2S)-2-(methylamino)-3-phenyl-propanoic acid
  MUTAGEN 15: note = X stands for D-alanine
  MUTAGEN 16: note = X stands for (2S)-2-(methylamino)-propanoic acid
XAWYXIXXXRXXXXXX

SEQ ID NO: 309 - protein, 16 aa, synthetic construct
  MUTAGEN 1: note = X stands for (2S)-2-(methylamino)-propanoic acid
  MUTAGEN 5: note = X stands for (2S)-2-(methylamino)-3-phenyl-propanoic acid
  MUTAGEN 7: note = X stands for (2S)-2-(methylamino)-propanoic acid
  MUTAGEN 8: note = X stands for (S)-2-amino-3-(3-(carboxymethoxy)phenyl)-propanoic acid
  MUTAGEN 9: note = X stands for (S)-4-(2-amino-2-carboxyethyl)-benzoic acid
  MUTAGEN 11: note = X stands for (2S)-2-(methylamino)-3-phenyl-propanoic acid
  MUTAGEN 12: note = X stands for (S)-2-amino-nonanoic acid
  MUTAGEN 13: note = X stands for (2S)-2-(methylamino)-propanoic acid
  MUTAGEN 14: note = X stands for (2S)-2-(methylamino)-3-phenyl-propanoic acid
XAWYXIXXXRXXXXGA

SEQ ID NO: 310 - protein, 16 aa, synthetic construct
  MUTAGEN 1: note = X stands for (2S)-2-(methylamino)-propanoic acid
  MUTAGEN 5: note = X stands for (2S)-2-(methylamino)-3-phenyl-propanoic acid
  MUTAGEN 7: note = X stands for (2S)-2-(methylamino)-propanoic acid
  MUTAGEN 8: note = X stands for (S)-2-amino-3-(3-(carboxymethoxy)phenyl)-propanoic acid
  MUTAGEN 9: note = X stands for (S)-4-(2-amino-2-carboxyethyl)-benzoic acid
  MUTAGEN 11: note = X stands for (2S)-2-(methylamino)-3-phenyl-propanoic acid
  MUTAGEN 12: note = X stands for (S)-2-amino-nonanoic acid
  MUTAGEN 13: note = X stands for (2S)-2-(methylamino)-propanoic acid
  MUTAGEN 14: note = X stands for (2S)-2-(methylamino)-3-phenyl-propanoic acid
  MOTIF 15: note = X stands for D-alanine
  MUTAGEN 16: note = X stands for 2-(methylamino)-acetic acid
XAWYXIXXXRXXXXXX

SEQ ID NO: 311 - protein, 15 aa, synthetic construct
  MUTAGEN 1: note = X stands for 4-((carboxymethyl)amino)-butanoic acid
  MUTAGEN 5: note = X stands for (2S)-2-(methylamino)-3-phenyl-propanoic acid
  MUTAGEN 7: note = X stands for (2S)-2-(methylamino)-propanoic acid
  MUTAGEN 8: note = X stands for (S)-2-amino-3-(3-(carboxymethoxy)phenyl)-propanoic acid
  MUTAGEN 9: note = X stands for (S)-4-(2-amino-2-carboxyethyl)-benzoic acid
  MUTAGEN 11: note = X stands for (2S)-2-(methylamino)-3-phenyl-propanoic acid
  MUTAGEN 12: note = X stands for (S)-2-amino-nonanoic acid
  MUTAGEN 13: note = X stands for (2S)-2-(methylamino)-propanoic acid
  MUTAGEN 14: note = X stands for (2S)-2-(methylamino)-3-phenyl-propanoic acid
  MUTAGEN 15: note = X stands for 2-(2-aminoethoxy)-acetic acid
XAWYXIXXXRXXXXX

SEQ ID NO: 312 - protein, 15 aa, synthetic construct
  MUTAGEN 1: note = X stands for 4-((carboxymethyl)amino)-butanoic acid
  MUTAGEN 5: note = X stands for (2S)-2-(methylamino)-3-phenyl-propanoic acid
  MUTAGEN 7: note = X stands for (2S)-2-(methylamino)-propanoic acid
  MUTAGEN 8: note = X stands for (S)-2-amino-3-(3-(carboxymethoxy)phenyl)-propanoic acid
  MUTAGEN 9: note = X stands for (S)-4-(2-amino-2-carboxyethyl)-benzoic acid
  MUTAGEN 11: note = X stands for (2S)-2-(methylamino)-3-phenyl-propanoic acid
  MUTAGEN 12: note = X stands for (S)-2-amino-nonanoic acid
  MUTAGEN 13: note = X stands for (2S)-2-(methylamino)-propanoic acid
  MUTAGEN 14: note = X stands for (2S)-2-(methylamino)-3-phenyl-propanoic acid
  MUTAGEN 15: note = X stands for 5-amino-pentanoic acid
XAWYXIXXXRXXXXX

SEQ ID NO: 313 - protein, 15 aa, synthetic construct
  MUTAGEN 1: note = X stands for 4-((carboxymethyl)amino)-butanoic acid
  MUTAGEN 5: note = X stands for (2S)-2-(methylamino)-3-phenyl-propanoic acid
  MUTAGEN 7: note = X stands for (2S)-2-(methylamino)-propanoic acid
  MUTAGEN 8: note = X stands for (S)-2-amino-3-(3-(carboxymethoxy)phenyl)-propanoic acid
  MUTAGEN 9: note = X stands for (S)-4-(2-amino-2-carboxyethyl)-benzoic acid
  MUTAGEN 11: note = X stands for (2S)-2-(methylamino)-3-phenyl-propanoic acid
  MUTAGEN 12: note = X stands for (S)-2-amino-nonanoic acid
  MUTAGEN 13: note = X stands for (2S)-2-(methylamino)-propanoic acid
  MUTAGEN 14: note = X stands for (2S)-2-(methylamino)-3-phenyl-propanoic acid
  MUTAGEN 15: note = X stands for 2-(2-(methylamino)ethoxy)-acetic acid
XAWYXIXXXRXXXXX

SEQ ID NO: 314 - protein, 15 aa, synthetic construct
  MUTAGEN 1: note = X stands for 4-((carboxymethyl)amino)-butanoic acid
  MUTAGEN 5: note = X stands for (2S)-2-(methylamino)-3-phenyl-propanoic acid
  MUTAGEN 7: note = X stands for (2S)-2-(methylamino)-propanoic acid
  MUTAGEN 8: note = X stands for (S)-2-amino-3-(3-(carboxymethoxy)phenyl)-propanoic acid
  MUTAGEN 9: note = X stands for (S)-4-(2-amino-2-carboxyethyl)-benzoic acid
  MUTAGEN 11: note = X stands for (2S)-2-(methylamino)-3-phenyl-propanoic acid
  MUTAGEN 12: note = X stands for (S)-2-amino-nonanoic acid
  MUTAGEN 13: note = X stands for (2S)-2-(methylamino)-propanoic acid
  MUTAGEN 14: note = X stands for (2S)-2-(methylamino)-3-phenyl-propanoic acid
  MUTAGEN 15: note = X stands for 5-(methylamino)-pentanoic acid
XAWYXIXXXRXXXXX

SEQ ID NO: 315-325 - skipped (11 entries)

SEQ ID NO: 326 - protein, 16 aa, synthetic construct
  MUTAGEN 1: note = X stands for (2S)-2-(methylamino)-pentanedioic acid
  MUTAGEN 3: note = X stands for 4-{3-[(2S)-2-amino-2-carboxyethyl]-1H-indole-1-yl}-benzoic acid
  MUTAGEN 5: note = X stands for (2S)-2-(methylamino)-3-phenyl-propanoic acid
  MUTAGEN 7: note = X stands for (2S)-2-(methylamino)-propanoic acid
  MUTAGEN 8: note = X stands for (S)-2-amino-3-(3-(carboxymethoxy)phenyl)-propanoic acid
  MUTAGEN 9: note = X stands for (S)-4-(2-amino-2-carboxyethyl)-benzoic acid
  MUTAGEN 11: note = X stands for (S)-3-(4-(aminomethyl)phenyl)-2-(methylamino)-propanoic acid
  MUTAGEN 12: note = X stands for (S)-2-amino-nonanoic acid
  MUTAGEN 13: note = X stands for (2S)-2-(methylamino)-propanoic acid
  MUTAGEN 14: note = X stands for (2S)-2-(methylamino)-3-phenyl-propanoic acid
  MUTAGEN 15: note = X stands for D-alanine
  MUTAGEN 16: note = X stands for (2S)-2-(methylamino)-propanoic acid
XAXYXIXXXRXXXXXX

SEQ ID NO: 327 - protein, 16 aa, synthetic construct
  MUTAGEN 1: note = X stands for (S)-2-(methylamino)-hexanedioic acid
  MUTAGEN 3: note = X stands for 4-{3-[(2S)-2-amino-2-carboxyethyl]-1H-indole-1-yl}-benzoic acid
  MUTAGEN 5: note = X stands for (2S)-2-(methylamino)-3-phenyl-propanoic acid
  MUTAGEN 7: note = X stands for (2S)-2-(methylamino)-propanoic acid
  MUTAGEN 8: note = X stands for (S)-2-amino-3-(3-(carboxymethoxy)phenyl)-propanoic acid
  MUTAGEN 9: note = X stands for (S)-4-(2-amino-2-carboxyethyl)-benzoic acid
  MUTAGEN 11: note = X stands for (S)-3-(4-(aminomethyl)phenyl)-2-(methylamino)-propanoic acid
  MUTAGEN 12: note = X stands for (S)-2-amino-nonanoic acid
  MUTAGEN 13: note = X stands for (2S)-2-(methylamino)-propanoic acid
  MUTAGEN 14: note = X stands for (2S)-2-(methylamino)-3-phenyl-propanoic acid
  MUTAGEN 15: note = X stands for D-alanine
  MUTAGEN 16: note = X stands for (2S)-2-(methylamino)-propanoic acid
XAXYXIXXXRXXXXXX

SEQ ID NO: 328 - protein, 16 aa, synthetic construct
  MUTAGEN 1: note = X stands for 3-((carboxymethyl)amino)-propanoic acid
  MUTAGEN 3: note = X stands for 4-{3-[(2S)-2-amino-2-carboxyethyl]-1H-indole-1-yl}-benzoic acid
  MUTAGEN 5: note = X stands for (2S)-2-(methylamino)-3-phenyl-propanoic acid
  MUTAGEN 7: note = X stands for D-proline
  MUTAGEN 8: note = X stands for (S)-2-amino-3-(3-(carboxymethoxy)phenyl)-propanoic acid
  MUTAGEN 9: note = X stands for (S)-4-(2-amino-2-carboxyethyl)-benzoic acid
  MUTAGEN 11: note = X stands for (2S)-2-(methylamino)-3-phenyl-propanoic acid
  MUTAGEN 12: note = X stands for (S)-2-amino-nonanoic acid
  MUTAGEN 13: note = X stands for (S)-3-amino-2-(methylamino)-propanoic acid
  MUTAGEN 14: note = X stands for (2S)-2-(methylamino)-3-phenyl-propanoic acid
  MUTAGEN 15: note = X stands for D-alanine
  MUTAGEN 16: note = X stands for (2S)-2-(methylamino)-propanoic acid
XAXYXIXXXRXXXXXX

SEQ ID NO: 329 - protein, 16 aa, synthetic construct
  MUTAGEN 1: note = X stands for 4-((carboxymethyl)amino)-butanoic acid
  MUTAGEN 3: note = X stands for 4-{3-[(2S)-2-amino-2-carboxyethyl]-1H-indole-1-yl}-benzoic acid
  MUTAGEN 5: note = X stands for (2S)-2-(methylamino)-3-phenyl-propanoic acid
  MUTAGEN 7: note = X stands for D-proline
  MUTAGEN 8: note = X stands for (S)-2-amino-3-(3-(carboxymethoxy)phenyl)-propanoic acid
  MUTAGEN 9: note = X stands for (S)-4-(2-amino-2-carboxyethyl)-benzoic acid
  MUTAGEN 11: note = X stands for (2S)-2-(methylamino)-3-phenyl-propanoic acid
  MUTAGEN 12: note = X stands for (S)-2-amino-nonanoic acid
  MUTAGEN 13: note = X stands for (S)-3-amino-2-(methylamino)-propanoic acid
  MUTAGEN 14: note = X stands for (2S)-2-(methylamino)-3-phenyl-propanoic acid
  MUTAGEN 15: note = X stands for D-alanine
  MUTAGEN 16: note = X stands for (2S)-2-(methylamino)-propanoic acid
XAXYXIXXXRXXXXXX

SEQ ID NO: 330 - protein, 16 aa, synthetic construct
  MUTAGEN 3: note = X stands for (S)-4-(3-(2-amino-2-carboxyethyl)-6-hydroxy-1H-indol-1-yl)-benzoic acid
  MUTAGEN 5: note = X stands for (2S)-2-(methylamino)-3-phenyl-propanoic acid
  MUTAGEN 7: note = X stands for D-proline
  MUTAGEN 8: note = X stands for (S)-2-amino-3-(3-(carboxymethoxy)phenyl)-propanoic acid
  MUTAGEN 9: note = X stands for (S)-4-(2-amino-2-carboxyethyl)-benzoic acid
  MUTAGEN 11: note = X stands for (2S)-2-(methylamino)-3-phenyl-propanoic acid
  MUTAGEN 12: note = X stands for (S)-2-amino-nonanoic acid
  MUTAGEN 13: note = X stands for (2S)-2-(methylamino)-propanoic acid
  MUTAGEN 14: note = X stands for (2S)-2-(methylamino)-3-phenyl-propanoic acid
  MUTAGEN 15: note = X stands for D-cysteine
  MUTAGEN 16: note = X stands for 3-(piperidine-4-yl)-propanoic acid
AAXYXIXXXRXXXXXX

SEQ ID NO: 331 - protein, 15 aa, synthetic construct
  MUTAGEN 3: note = X stands for (S)-2-amino-3-(6-hydroxy-1H-indol-3-yl)-propanoic acid
  MUTAGEN 5: note = X stands for (2S)-2-(methylamino)-3-phenyl-propanoic acid
  MUTAGEN 7: note = X stands for D-proline
  MUTAGEN 8: note = X stands for (S)-2-amino-3-(3-(carboxymethoxy)phenyl)-propanoic acid
  MUTAGEN 9: note = X stands for (S)-4-(2-amino-2-carboxyethyl)-benzoic acid
  MUTAGEN 11: note = X stands for (2S)-2-(methylamino)-3-phenyl-propanoic acid
  MUTAGEN 12: note = X stands for (S)-2-aminodo-decanoic acid
  MUTAGEN 13: note = X stands for (2S)-2-(methylamino)-propanoic acid
  MUTAGEN 14: note = X stands for (2S)-2-(methylamino)-3-phenyl-propanoic acid
  MUTAGEN 15: note = X stands for D-cysteine
AAXYXIXXXRXXXXX

SEQ ID NO: 332 - protein, 16 aa, synthetic construct
  MUTAGEN 1: note = X stands for 4-((carboxymethyl)amino)-butanoic acid
  MUTAGEN 3: note = X stands for (S)-2-amino-3-(6-hydroxy-1H-indol-3-yl)-propanoic acid
  MUTAGEN 5: note = X stands for (2S)-2-(methylamino)-3-phenyl-propanoic acid
  MUTAGEN 7: note = X stands for D-proline
  MUTAGEN 8: note = X stands for (S)-2-amino-3-(3-(carboxymethoxy)phenyl)-propanoic acid
  MUTAGEN 9: note = X stands for (S)-4-(2-amino-2-carboxyethyl)-benzoic acid
  MUTAGEN 11: note = X stands for (2S)-2-(methylamino)-3-phenyl-propanoic acid
  MUTAGEN 12: note = X stands for (S)-2-aminodo-decanoic acid
  MUTAGEN 13: note = X stands for (2S)-2-(methylamino)-propanoic acid
  MUTAGEN 14: note = X stands for (2S)-2-(methylamino)-3-phenyl-propanoic acid
  MUTAGEN 15: note = X stands for D-cysteine
  MUTAGEN 16: note = X stands for 3-(piperidine-4-yl)-propanoic acid
XAXYXIXXXRXXXXXX

SEQ ID NO: 333 - protein, 16 aa, synthetic construct
  MUTAGEN 1: note = X stands for 4-((carboxymethyl)amino)-butanoic acid
  MUTAGEN 3: note = X stands for (S)-2-amino-3-(6-hydroxy-1H-indol-3-yl)-propanoic acid
  MUTAGEN 5: note = X stands for (2S)-2-(methylamino)-3-phenyl-propanoic acid
  MUTAGEN 7: note = X stands for 2-(methylamino)-acetic acid
  MUTAGEN 8: note = X stands for (S)-2-amino-3-(3-(carboxymethoxy)phenyl)-propanoic acid
  MUTAGEN 9: note = X stands for (S)-4-(2-amino-2-carboxyethyl)-benzoic acid
  MUTAGEN 11: note = X stands for (2S)-2-(methylamino)-3-phenyl-propanoic acid
  MUTAGEN 12: note = X stands for (S)-2-amino-nonanoic acid
  MUTAGEN 13: note = X stands for (2S)-2-(methylamino)-propanoic acid
  MUTAGEN 14: note = X stands for (2S)-2-(methylamino)-3-phenyl-propanoic acid
  MUTAGEN 15: note = X stands for D-cysteine
  MUTAGEN 16: note = X stands for 3-(piperidine-4-yl)-propanoic acid
XAXYXIXXXRXXXXXX

SEQ ID NO: 334 - protein, 16 aa, synthetic construct
  MUTAGEN 3: note = X stands for (S)-4-(3-(2-amino-2-carboxyethyl)-6-hydroxy-1H-indol-1-yl)-benzoic acid
  MUTAGEN 5: note = X stands for (2S)-2-(methylamino)-3-phenyl-propanoic acid
  MUTAGEN 7: note = X stands for D-proline
  MUTAGEN 8: note = X stands for (S)-2-amino-3-(3-(carboxymethoxy)phenyl)-propanoic acid
  MUTAGEN 9: note = X stands for (S)-4-(2-amino-2-carboxyethyl)-benzoic acid
  MUTAGEN 11: note = X stands for (S)-3-(4-(aminomethyl)phenyl)-2-(methylamino)-propanoic acid
  MUTAGEN 12: note = X stands for (S)-2-amino-nonanoic acid
  MUTAGEN 13: note = X stands for (2S)-2-(methylamino)-propanoic acid
  MUTAGEN 14: note = X stands for (2S)-2-(methylamino)-3-phenyl-propanoic acid
  MUTAGEN 15: note = X stands for D-cysteine
  MUTAGEN 16: note = X stands for 3-(piperidine-4-yl)-propanoic acid
EAXYXIXXXRXXXXXX

SEQ ID NO: 335 - protein, 16 aa, synthetic construct
  MUTAGEN 3: note = X stands for (S)-2-amino-3-(6-hydroxy-1H-indol-3-yl)-propanoic acid
  MUTAGEN 5: note = X stands for (2S)-2-(methylamino)-3-phenyl-propanoic acid
  MUTAGEN 7: note = X stands for 2-(methylamino)-acetic acid
  MUTAGEN 8: note = X stands for (S)-2-amino-3-(3-(carboxymethoxy)phenyl)-propanoic acid
  MUTAGEN 9: note = X stands for (S)-4-(2-amino-2-carboxyethyl)-benzoic acid
  MUTAGEN 11: note = X stands for (S)-3-(4-(aminomethyl)phenyl)-2-(methylamino)-propanoic acid
  MUTAGEN 12: note = X stands for (S)-2-amino-nonanoic acid
  MUTAGEN 13: note = X stands for (2S)-2-(methylamino)-propanoic acid
  MUTAGEN 14: note = X stands for (2S)-2-(methylamino)-3-phenyl-propanoic acid
  MUTAGEN 15: note = X stands for D-cysteine
  MUTAGEN 16: note = X stands for 3-(piperidine-4-yl)-propanoic acid
EAXYXIXXXRXXXXXX

SEQ ID NO: 336 - protein, 15 aa, synthetic construct
  MUTAGEN 3: note = X stands for (S)-2-amino-3-(6-hydroxy-1H-indol-3-yl)-propanoic acid
  MUTAGEN 5: note = X stands for (2S)-2-(methylamino)-3-phenyl-propanoic acid
  MUTAGEN 7: note = X stands for D-proline
  MUTAGEN 8: note = X stands for (S)-2-amino-3-(3-(carboxymethoxy)phenyl)-propanoic acid
  MUTAGEN 9: note = X stands for (S)-4-(2-amino-2-carboxyethyl)-benzoic acid
  MUTAGEN 11: note = X stands for (S)-3-(4-(aminomethyl)phenyl)-2-(methylamino)-propanoic acid
  MUTAGEN 12: note = X stands for (S)-2-aminodo-decanoic acid
  MUTAGEN 13: note = X stands for (2S)-2-(methylamino)-propanoic acid
  MUTAGEN 14: note = X stands for (2S)-2-(methylamino)-3-phenyl-propanoic acid
  MUTAGEN 15: note = X stands for D-cysteine
EAXYXIXXXRXXXXX

SEQ ID NO: 337 - protein, 16 aa, synthetic construct
  MUTAGEN 1: note = X stands for 3-((carboxymethyl)amino)-propanoic acid
  MUTAGEN 3: note = X stands for (S)-4-(3-(2-amino-2-carboxyethyl)-6-hydroxy-1H-indol-1-yl)-benzoic acid
  MUTAGEN 5: note = X stands for (2S)-2-(methylamino)-3-phenyl-propanoic acid
  MUTAGEN 7: note = X stands for D-proline
  MUTAGEN 8: note = X stands for (S)-2-amino-3-(3-(carboxymethoxy)phenyl)-propanoic acid
  MUTAGEN 9: note = X stands for (S)-4-(2-amino-2-carboxyethyl)-benzoic acid
  MUTAGEN 11: note = X stands for (2S)-2-(methylamino)-3-phenyl-propanoic acid
  MUTAGEN 12: note = X stands for (S)-2-amino-nonanoic acid
  MUTAGEN 13: note = X stands for (S)-3-amino-2-(methylamino)-propanoic acid
  MUTAGEN 14: note = X stands for (2S)-2-(methylamino)-3-phenyl-propanoic acid
  MUTAGEN 15: note = X stands for D-cysteine
  MUTAGEN 16: note = X stands for 3-(piperidine-4-yl)-propanoic acid
XAXYXIXXXRXXXXXX

SEQ ID NO: 338 - protein, 16 aa, synthetic construct
  MUTAGEN 1: note = X stands for 3-((carboxymethyl)amino)-propanoic acid
  MUTAGEN 3: note = X stands for (S)-2-amino-3-(6-hydroxy-1H-indol-3-yl)-propanoic acid
  MUTAGEN 5: note = X stands for (2S)-2-(methylamino)-3-phenyl-propanoic acid
  MUTAGEN 7: note = X stands for 2-(methylamino)-acetic acid
  MUTAGEN 8: note = X stands for (S)-2-amino-3-(3-(carboxymethoxy)phenyl)-propanoic acid
  MUTAGEN 9: note = X stands for (S)-4-(2-amino-2-carboxyethyl)-benzoic acid
  MUTAGEN 11: note = X stands for (2S)-2-(methylamino)-3-phenyl-propanoic acid
  MUTAGEN 12: note = X stands for (S)-2-amino-nonanoic acid
  MUTAGEN 13: note = X stands for (S)-3-amino-2-(methylamino)-propanoic acid
  MUTAGEN 14: note = X stands for (2S)-2-(methylamino)-3-phenyl-propanoic acid
  MUTAGEN 15: note = X stands for D-cysteine
  MUTAGEN 16: note = X stands for 3-(piperidine-4-yl)-propanoic acid
XAXYXIXXXRXXXXXX

SEQ ID NO: 339 - protein, 16 aa, synthetic construct
  MUTAGEN 1: note = X stands for 4-((carboxymethyl)amino)-butanoic acid
  MUTAGEN 3: note = X stands for (S)-2-amino-3-(6-hydroxy-1H-indol-3-yl)-propanoic acid
  MUTAGEN 5: note = X stands for (2S)-2-(methylamino)-3-phenyl-propanoic acid
  MUTAGEN 7: note = X stands for D-proline
  MUTAGEN 8: note = X stands for (S)-2-amino-3-(3-(carboxymethoxy)phenyl)-propanoic acid
  MUTAGEN 9: note = X stands for (S)-4-(2-amino-2-carboxyethyl)-benzoic acid
  MUTAGEN 11: note = X stands for (2S)-2-(methylamino)-3-phenyl-propanoic acid
  MUTAGEN 12: note = X stands for (S)-2-aminodo-decanoic acid
  MUTAGEN 13: note = X stands for (2S)-2-(methylamino)-propanoic acid
  MUTAGEN 14: note = X stands for (2S)-2-(methylamino)-3-phenyl-propanoic acid
  MUTAGEN 15: note = X stands for D-alanine
  MUTAGEN 16: note = X stands for (2S)-2-(methylamino)-propanoic acid
XAXYXIXXXRXXXXXX

SEQ ID NO: 340 - protein, 16 aa, synthetic construct
  MUTAGEN 1: note = X stands for 4-((carboxymethyl)amino)-butanoic acid
  MUTAGEN 3: note = X stands for (S)-2-amino-3-(6-hydroxy-1H-indol-3-yl)-propanoic acid
  MUTAGEN 5: note = X stands for (2S)-2-(methylamino)-3-phenyl-propanoic acid
  MUTAGEN 7: note = X stands for 2-(methylamino)-acetic acid
  MUTAGEN 8: note = X stands for (S)-2-amino-3-(3-(carboxymethoxy)phenyl)-propanoic acid
  MUTAGEN 9: note = X stands for (S)-4-(2-amino-2-carboxyethyl)-benzoic acid
  MUTAGEN 11: note = X stands for (2S)-2-(methylamino)-3-phenyl-propanoic acid
  MUTAGEN 12: note = X stands for (S)-2-amino-nonanoic acid
  MUTAGEN 13: note = X stands for (2S)-2-(methylamino)-propanoic acid
  MUTAGEN 14: note = X stands for (2S)-2-(methylamino)-3-phenyl-propanoic acid
  MUTAGEN 15: note = X stands for D-alanine
  MUTAGEN 16: note = X stands for (2S)-2-(methylamino)-propanoic acid
XAXYXIXXXRXXXXXX

SEQ ID NO: 341 - protein, 16 aa, synthetic construct
  MUTAGEN 1: note = X stands for 4-((carboxymethyl)amino)-butanoic acid
  MUTAGEN 3: note = X stands for (S)-4-(3-(2-amino-2-carboxyethyl)-6-hydroxy-1H-indol-1-yl)-benzoic acid
  MUTAGEN 5: note = X stands for (2S)-2-(methylamino)-3-phenyl-propanoic acid
  MUTAGEN 7: note = X stands for D-proline
  MUTAGEN 8: note = X stands for (S)-2-amino-3-(3-(carboxymethoxy)phenyl)-propanoic acid
  MUTAGEN 9: note = X stands for (S)-4-(2-amino-2-carboxyethyl)-benzoic acid
  MUTAGEN 11: note = X stands for (2S)-2-(methylamino)-3-phenyl-propanoic acid
  MUTAGEN 12: note = X stands for (S)-2-amino-nonanoic acid
  MUTAGEN 13: note = X stands for (2S)-2-(methylamino)-propanoic acid
  MUTAGEN 14: note = X stands for (2S)-2-(methylamino)-3-phenyl-propanoic acid
  MUTAGEN 15: note = X stands for D-alanine
  MUTAGEN 16: note = X stands for (2S)-2-(methylamino)-propanoic acid
XAXYXIXXXRXXXXXX

SEQ ID NO: 342 - protein, 16 aa, synthetic construct
  MUTAGEN 3: note = X stands for (S)-4-(3-(2-amino-2-carboxyethyl)-6-hydroxy-1H-indol-1-yl)-benzoic acid
  MUTAGEN 5: note = X stands for (2S)-2-(methylamino)-3-phenyl-propanoic acid
  MUTAGEN 7: note = X stands for D-proline
  MUTAGEN 8: note = X stands for (S)-2-amino-3-(3-(carboxymethoxy)phenyl)-propanoic acid
  MUTAGEN 9: note = X stands for (S)-4-(2-amino-2-carboxyethyl)-benzoic acid
  MUTAGEN 11: note = X stands for (2S)-2-(methylamino)-3-phenyl-propanoic acid
  MUTAGEN 12: note = X stands for (S)-2-amino-nonanoic acid
  MUTAGEN 13: note = X stands for (2S)-2-(methylamino)-propanoic acid
  MUTAGEN 14: note = X stands for (2S)-2-(methylamino)-3-phenyl-propanoic acid
  MUTAGEN 15: note = X stands for D-alanine
  MUTAGEN 16: note = X stands for (2S)-2-(methylamino)-propanoic acid
AAXYXIXXXRXXXXXX

SEQ ID NO: 343 - protein, 16 aa, synthetic construct
  MUTAGEN 3: note = X stands for (S)-2-amino-3-(6-hydroxy-1H-indol-3-yl)-propanoic acid
  MUTAGEN 5: note = X stands for (2S)-2-(methylamino)-3-phenyl-propanoic acid
  MUTAGEN 7: note = X stands for D-proline
  MUTAGEN 8: note = X stands for (S)-2-amino-3-(3-(carboxymethoxy)phenyl)-propanoic acid
  MUTAGEN 9: note = X stands for (S)-4-(2-amino-2-carboxyethyl)-benzoic acid
  MUTAGEN 11: note = X stands for (2S)-2-(methylamino)-3-phenyl-propanoic acid
  MUTAGEN 12: note = X stands for (S)-2-aminodo-decanoic acid
  MUTAGEN 13: note = X stands for (2S)-2-(methylamino)-pentanedioic acid
  MUTAGEN 14: note = X stands for (2S)-2-(methylamino)-3-phenyl-propanoic acid
  MUTAGEN 15: note = X stands for D-alanine
  MUTAGEN 16: note = X stands for (2S)-2-(methylamino)-propanoic acid
AAXYXIXXXRXXXXXX

SEQ ID NO: 344 - protein, 16 aa, synthetic construct
  MUTAGEN 3: note = X stands for (S)-2-amino-3-(6-hydroxy-1H-indol-3-yl)-propanoic acid
  MUTAGEN 5: note = X stands for (2S)-2-(methylamino)-3-phenyl-propanoic acid
  MUTAGEN 7: note = X stands for 2-(methylamino)-acetic acid
  MUTAGEN 8: note = X stands for (S)-2-amino-3-(3-(carboxymethoxy)phenyl)-propanoic acid
  MUTAGEN 9: note = X stands for (S)-4-(2-amino-2-carboxyethyl)-benzoic acid
  MUTAGEN 11: note = X stands for (2S)-2-(methylamino)-3-phenyl-propanoic acid
  MUTAGEN 12: note = X stands for (S)-2-amino-nonanoic acid
  MUTAGEN 13: note = X stands for (2S)-2-(methylamino)-propanoic acid
  MUTAGEN 14: note = X stands for (2S)-2-(methylamino)-3-phenyl-propanoic acid
  MUTAGEN 15: note = X stands for D-alanine
  MUTAGEN 16: note = X stands for (2S)-2-(methylamino)-propanoic acid
AAXYXIXXXRXXXXXX

SEQ ID NO: 345 - protein, 16 aa, synthetic construct
  MUTAGEN 1: note = X stands for (2S)-2-(methylamino)-propanoic acid
  MUTAGEN 3: note = X stands for (S)-4-(3-(2-amino-2-carboxyethyl)-6-hydroxy-1H-indol-1-yl)-benzoic acid
  MUTAGEN 5: note = X stands for (2S)-2-(methylamino)-3-phenyl-propanoic acid
  MUTAGEN 7: note = X stands for D-proline
  MUTAGEN 8: note = X stands for (S)-2-amino-3-(3-(carboxymethoxy)phenyl)-propanoic acid
  MUTAGEN 9: note = X stands for (S)-4-(2-amino-2-carboxyethyl)-benzoic acid
  MUTAGEN 11: note = X stands for (2S)-2-(methylamino)-3-phenyl-propanoic acid
  MUTAGEN 12: note = X stands for (S)-2-amino-nonanoic acid
  MUTAGEN 13: note = X stands for (2S)-2-(methylamino)-propanoic acid
  MUTAGEN 14: note = X stands for (2S)-2-(methylamino)-3-phenyl-propanoic acid
  MUTAGEN 15: note = X stands for D-alanine
  MUTAGEN 16: note = X stands for (2S)-2-(methylamino)-propanoic acid
XAXYXIXXXRXXXXXX

SEQ ID NO: 346 - protein, 16 aa, synthetic construct
  MUTAGEN 1: note = X stands for (2S)-2-(methylamino)-propanoic acid
  MUTAGEN 3: note = X stands for (S)-2-amino-3-(6-hydroxy-1H-indol-3-yl)-propanoic acid
  MUTAGEN 5: note = X stands for (2S)-2-(methylamino)-3-phenyl-propanoic acid
  MUTAGEN 7: note = X stands for D-proline
  MUTAGEN 8: note = X stands for (S)-2-amino-3-(3-(carboxymethoxy)phenyl)-propanoic acid
  MUTAGEN 9: note = X stands for (S)-4-(2-amino-2-carboxyethyl)-benzoic acid
  MUTAGEN 11: note = X stands for (2S)-2-(methylamino)-3-phenyl-propanoic acid
  MUTAGEN 12: note = X stands for (S)-2-aminodo-decanoic acid
  MUTAGEN 13: note = X stands for (2S)-2-(methylamino)-pentanedioic acid
  MUTAGEN 14: note = X stands for (2S)-2-(methylamino)-3-phenyl-propanoic acid
  MUTAGEN 15: note = X stands for D-alanine
  MUTAGEN 16: note = X stands for (2S)-2-(methylamino)-propanoic acid
XAXYXIXXXRXXXXXX

SEQ ID NO: 347 - protein, 16 aa, synthetic construct
  MUTAGEN 1: note = X stands for 4-((carboxymethyl)amino)-butanoic acid
  MUTAGEN 3: note = X stands for (S)-4-(3-(2-amino-2-carboxyethyl)-6-hydroxy-1H-indol-1-yl)-benzoic acid
  MUTAGEN 5: note = X stands for (2S)-2-(methylamino)-3-phenyl-propanoic acid
  MUTAGEN 7: note = X stands for D-proline
  MUTAGEN 8: note = X stands for (S)-2-amino-3-(3-(carboxymethoxy)phenyl)-propanoic acid
  MUTAGEN 9: note = X stands for (S)-4-(2-amino-2-carboxyethyl)-benzoic acid
  MUTAGEN 11: note = X stands for (2S)-2-(methylamino)-3-phenyl-propanoic acid
  MUTAGEN 12: note = X stands for (S)-2-amino-nonanoic acid
  MUTAGEN 13: note = X stands for (2S)-2-(methylamino)-propanoic acid
  MUTAGEN 14: note = X stands for (2S)-2-(methylamino)-3-phenyl-propanoic acid
  MUTAGEN 15: note = X stands for D-cysteine
  MUTAGEN 16: note = X stands for 3-(piperidine-4-yl)-propanoic acid
XAXYXIXXXRXXXXXX

SEQ ID NO: 348 - protein, 16 aa, synthetic construct
  MUTAGEN 1: note = X stands for 3-((carboxymethyl)amino)-propanoic acid
  MUTAGEN 3: note = X stands for (S)-4-(3-(2-amino-2-carboxyethyl)-6-hydroxy-1H-indol-1-yl)-benzoic acid
  MUTAGEN 5: note = X stands for (2S)-2-(methylamino)-3-phenyl-propanoic acid
  MUTAGEN 7: note = X stands for D-proline
  MUTAGEN 8: note = X stands for (S)-2-amino-3-(3-(carboxymethoxy)phenyl)-propanoic acid
  MUTAGEN 9: note = X stands for (S)-4-(2-amino-2-carboxyethyl)-benzoic acid
  MUTAGEN 11: note = X stands for (2S)-2-(methylamino)-3-phenyl-propanoic acid
  MUTAGEN 12: note = X stands for (S)-2-amino-nonanoic acid
  MUTAGEN 13: note = X stands for (S)-3-amino-2-(methylamino)-propanoic acid
  MUTAGEN 14: note = X stands for (2S)-2-(methylamino)-3-phenyl-propanoic acid
  MUTAGEN 15: note = X stands for D-alanine
  MUTAGEN 16: note = X stands for (2S)-2-(methylamino)-propanoic acid
XAXYXIXXXRXXXXXX

SEQ ID NO: 349 - protein, 16 aa, synthetic construct
  MUTAGEN 1: note = X stands for (S)-2-(methylamino)-hexanedioic acid
  MUTAGEN 3: note = X stands for (S)-4-(3-(2-amino-2-carboxyethyl)-6-hydroxy-1H-indol-1-yl)-benzoic acid
  MUTAGEN 5: note = X stands for (2S)-2-(methylamino)-3-phenyl-propanoic acid
  MUTAGEN 7: note = X stands for D-proline
  MUTAGEN 9: note = X stands for (S)-4-(2-amino-2-carboxyethyl)-benzoic acid
  MUTAGEN 11: note = X stands for (S)-3-(4-(aminomethyl)phenyl)-2-(methylamino)-propanoic acid
  MUTAGEN 12: note = X stands for (S)-2-amino-nonanoic acid
  MUTAGEN 13: note = X stands for (2S)-2-(methylamino)-propanoic acid
  MUTAGEN 14: note = X stands for (2S)-2-(methylamino)-3-phenyl-propanoic acid
  MUTAGEN 15: note = X stands for D-alanine
  MUTAGEN 16: note = X stands for (2S)-2-(methylamino)-propanoic acid
  MUTAGEN 8: note = X stands for (S)-2-amino-3-(3-(carboxymethoxy)phenyl)-propanoic acid
XAXYXIXXXRXXXXXX

SEQ ID NO: 350 - protein, 16 aa, synthetic construct
  MUTAGEN 1: note = X stands for (S)-2-amino-hexanedioic acid
  MUTAGEN 3: note = X stands for (S)-4-(3-(2-amino-2-carboxyethyl)-6-hydroxy-1H-indol-1-yl)-benzoic acid
  MUTAGEN 5: note = X stands for (2S)-2-(methylamino)-3-phenyl-propanoic acid
  MUTAGEN 7: note = X stands for D-proline
  MUTAGEN 8: note = X stands for (S)-2-amino-3-(3-(carboxymethoxy)phenyl)-propanoic acid
  MUTAGEN 9: note = X stands for (S)-4-(2-amino-2-carboxyethyl)-benzoic acid
  MUTAGEN 11: note = X stands for (S)-3-(4-(aminomethyl)phenyl)-2-(methylamino)-propanoic acid
  MUTAGEN 12: note = X stands for (S)-2-amino-nonanoic acid
  MUTAGEN 13: note = X stands for (2S)-2-(methylamino)-propanoic acid
  MUTAGEN 14: note = X stands for (2S)-2-(methylamino)-3-phenyl-propanoic acid
  MUTAGEN 15: note = X stands for D-alanine
  MUTAGEN 16: note = X stands for (2S)-2-(methylamino)-propanoic acid
XAXYXIXXXRXXXXXX

SEQ ID NO: 351 - protein, 16 aa, synthetic construct
  MUTAGEN 1: note = X stands for 3-((carboxymethyl)amino)-propanoic acid
  MUTAGEN 3: note = X stands for (S)-2-amino-3-(6-hydroxy-1H-indol-3-yl)-propanoic acid
  MUTAGEN 5: note = X stands for (2S)-2-(methylamino)-3-phenyl-propanoic acid
  MUTAGEN 7: note = X stands for 2-(methylamino)-acetic acid
  MUTAGEN 8: note = X stands for (S)-2-amino-3-(3-(carboxymethoxy)phenyl)-propanoic acid
  MUTAGEN 9: note = X stands for (S)-4-(2-amino-2-carboxyethyl)-benzoic acid
  MUTAGEN 11: note = X stands for (2S)-2-(methylamino)-3-phenyl-propanoic acid
  MUTAGEN 12: note = X stands for (S)-2-amino-nonanoic acid
  MUTAGEN 13: note = X stands for (S)-3-amino-2-(methylamino)-propanoic acid
  MUTAGEN 14: note = X stands for (2S)-2-(methylamino)-3-phenyl-propanoic acid
  MUTAGEN 15: note = X stands for D-alanine
  MUTAGEN 16: note = X stands for (2S)-2-(methylamino)-propanoic acid
XAXYXIXXXRXXXXXX

SEQ ID NO: 352 - protein, 16 aa, synthetic construct
  MUTAGEN 1: note = X stands for (S)-2-(methylamino)-hexanedioic acid
  MUTAGEN 3: note = X stands for (S)-2-amino-3-(6-hydroxy-1H-indol-3-yl)-propanoic acid
  MUTAGEN 5: note = X stands for (2S)-2-(methylamino)-3-phenyl-propanoic acid
  MUTAGEN 7: note = X stands for 2-(methylamino)-acetic acid
  MUTAGEN 8: note = X stands for (S)-2-amino-3-(3-(carboxymethoxy)phenyl)-propanoic acid
  MUTAGEN 9: note = X stands for (S)-4-(2-amino-2-carboxyethyl)-benzoic acid
  MUTAGEN 11: note = X stands for (S)-3-(4-(aminomethyl)phenyl)-2-(methylamino)-propanoic acid
  MUTAGEN 12: note = X stands for (S)-2-amino-nonanoic acid
  MUTAGEN 13: note = X stands for (2S)-2-(methylamino)-propanoic acid
  MUTAGEN 14: note = X stands for (2S)-2-(methylamino)-3-phenyl-propanoic acid
  MUTAGEN 15: note = X stands for D-alanine
  MUTAGEN 16: note = X stands for (2S)-2-(methylamino)-propanoic acid
XAXYXIXXXRXXXXXX

SEQ ID NO: 353 - protein, 16 aa, synthetic construct
  MUTAGEN 1: note = X stands for (S)-2-amino-hexanedioic acid
  MUTAGEN 3: note = X stands for (S)-2-amino-3-(6-hydroxy-1H-indol-3-yl)-propanoic acid
  MUTAGEN 5: note = X stands for (2S)-2-(methylamino)-3-phenyl-propanoic acid
  MUTAGEN 7: note = X stands for 2-(methylamino)-acetic acid
  MUTAGEN 8: note = X stands for (S)-2-amino-3-(3-(carboxymethoxy)phenyl)-propanoic acid
  MUTAGEN 9: note = X stands for (S)-4-(2-amino-2-carboxyethyl)-benzoic acid
  MUTAGEN 11: note = X stands for (S)-3-(4-(aminomethyl)phenyl)-2-(methylamino)-propanoic acid
  MUTAGEN 12: note = X stands for (S)-2-amino-nonanoic acid
  MUTAGEN 13: note = X stands for (2S)-2-(methylamino)-propanoic acid
  MUTAGEN 14: note = X stands for (2S)-2-(methylamino)-3-phenyl-propanoic acid
  MUTAGEN 15: note = X stands for D-alanine
  MUTAGEN 16: note = X stands for (2S)-2-(methylamino)-propanoic acid
XAXYXIXXXRXXXXXX

SEQ ID NO: 354 - protein, 16 aa, synthetic construct
  MUTAGEN 1: note = X stands for 3-((carboxymethyl)amino)-propanoic acid
  MUTAGEN 3: note = X stands for (S)-2-amino-3-(6-hydroxy-1H-indol-3-yl)-propanoic acid
  MUTAGEN 5: note = X stands for (2S)-2-(methylamino)-3-phenyl-propanoic acid
  MUTAGEN 7: note = X stands for D-proline
  MUTAGEN 8: note = X stands for (S)-2-amino-3-(3-(carboxymethoxy)phenyl)-propanoic acid
  MUTAGEN 9: note = X stands for (S)-4-(2-amino-2-carboxyethyl)-benzoic acid
  MUTAGEN 11: note = X stands for (2S)-2-(methylamino)-3-phenyl-propanoic acid
  MUTAGEN 12: note = X stands for (S)-2-amino-nonanoic acid
  MUTAGEN 13: note = X stands for (S)-3-amino-2-(methylamino)-propanoic acid
  MUTAGEN 14: note = X stands for (2S)-2-(methylamino)-3-phenyl-propanoic acid
  MUTAGEN 15: note = X stands for D-alanine
  MUTAGEN 16: note = X stands for (2S)-2-(methylamino)-propanoic acid
XAXYXIXXXRXXXXXX

SEQ ID NO: 355 - protein, 16 aa, synthetic construct
  MUTAGEN 3: note = X stands for (S)-2-amino-3-(6-hydroxy-1H-indol-3-yl)-propanoic acid
  MUTAGEN 5: note = X stands for (2S)-2-(methylamino)-3-phenyl-propanoic acid
  MUTAGEN 7: note = X stands for D-proline
  MUTAGEN 8: note = X stands for (S)-2-amino-3-(3-(carboxymethoxy)phenyl)-propanoic acid
  MUTAGEN 9: note = X stands for (S)-4-(2-amino-2-carboxyethyl)-benzoic acid
  MUTAGEN 11: note = X stands for (2S)-2-(methylamino)-3-phenyl-propanoic acid
  MUTAGEN 12: note = X stands for (S)-2-aminodo-decanoic acid
  MUTAGEN 13: note = X stands for (2S)-2-(methylamino)-pentanedioic acid
  MUTAGEN 14: note = X stands for (2S)-2-(methylamino)-3-phenyl-propanoic acid
  MUTAGEN 15: note = X stands for D-cysteine
  MUTAGEN 16: note = X stands for 3-(piperidine-4-yl)-propanoic acid
AAXYXIXXXRXXXXXX

SEQ ID NO: 356 - protein, 16 aa, synthetic construct
  MUTAGEN 3: note = X stands for (S)-2-amino-3-(6-hydroxy-1H-indol-3-yl)-propanoic acid
  MUTAGEN 5: note = X stands for (2S)-2-(methylamino)-3-phenyl-propanoic acid
  MUTAGEN 7: note = X stands for D-proline
  MUTAGEN 8: note = X stands for (S)-2-amino-3-(3-(carboxymethoxy)phenyl)-propanoic acid
  MUTAGEN 9: note = X stands for (S)-4-(2-amino-2-carboxyethyl)-benzoic acid
  MUTAGEN 11: note = X stands for (2S)-2-(methylamino)-3-phenyl-propanoic acid
  MUTAGEN 12: note = X stands for (S)-2-aminodo-decanoic acid
  MUTAGEN 13: note = X stands for (2S)-2-(methylamino)-pentanedioic acid
  MUTAGEN 14: note = X stands for (2S)-2-(methylamino)-3-phenyl-propanoic acid
  MUTAGEN 15: note = X stands for D-cysteine
  MUTAGEN 16: note = X stands for 3-(piperidine-4-yl)-propanoic acid
AAXYXIXXXRXXXXXX

SEQ ID NO: 357 - protein, 15 aa, synthetic construct
  MUTAGEN 1: note = X stands for 4-((carboxymethyl)amino)-butanoic acid
  MUTAGEN 5: note = X stands for (2S)-2-(methylamino)-3-phenyl-propanoic acid
  MUTAGEN 7: note = X stands for (2S)-2-(methylamino)-propanoic acid
  MUTAGEN 8: note = X stands for (S)-2-amino-3-(3-(carboxymethoxy)phenyl)-propanoic acid
  MUTAGEN 9: note = X stands for (S)-4-(2-amino-2-carboxyethyl)-benzoic acid
  MUTAGEN 11: note = X stands for (2S)-2-(methylamino)-3-phenyl-propanoic acid
  MUTAGEN 12: note = X stands for (S)-2-amino-nonanoic acid
  MUTAGEN 13: note = X stands for (2S)-2-(methylamino)-propanoic acid
  MUTAGEN 14: note = X stands for (2S)-2-(methylamino)-3-phenyl-propanoic acid
  MUTAGEN 15: note = X stands for D-cysteine
XAWYXIXXXRXXXXX

SEQ ID NO: 358 - protein, 15 aa, synthetic construct
  MUTAGEN 1: note = X stands for 3-((carboxymethyl)amino)-propanoic acid
  MUTAGEN 3: note = X stands for 4-{3-[(2S)-2-amino-2-carboxyethyl]-1H-indole-1-yl}-benzoic acid
  MUTAGEN 5: note = X stands for (2S)-2-(methylamino)-3-phenyl-propanoic acid
  MUTAGEN 7: note = X stands for D-proline
  MUTAGEN 8: note = X stands for (S)-2-amino-3-(3-(carboxymethoxy)phenyl)-propanoic acid
  MUTAGEN 9: note = X stands for (S)-4-(2-amino-2-carboxyethyl)-benzoic acid
  MUTAGEN 11: note = X stands for (2S)-2-(methylamino)-3-phenyl-propanoic acid
  MUTAGEN 12: note = X stands for (S)-2-amino-nonanoic acid
  MUTAGEN 13: note = X stands for (S)-3-amino-2-(methylamino)-propanoic acid
  MUTAGEN 14: note = X stands for (2S)-2-(methylamino)-3-phenyl-propanoic acid
  MUTAGEN 15: note = X stands for D-cysteine
XAXYXIXXXRXXXXX

SEQ ID NO: 359 - protein, 15 aa, synthetic construct
  MUTAGEN 1: note = X stands for (2S)-2-(methylamino)-pentanedioic acid
  MUTAGEN 3: note = X stands for 4-{3-[(2S)-2-amino-2-carboxyethyl]-1H-indole-1-yl}-benzoic acid
  MUTAGEN 5: note = X stands for (2S)-2-(methylamino)-3-phenyl-propanoic acid
  MUTAGEN 7: note = X stands for D-proline
  MUTAGEN 8: note = X stands for (S)-2-amino-3-(3-(carboxymethoxy)phenyl)-propanoic acid
  MUTAGEN 9: note = X stands for (S)-4-(2-amino-2-carboxyethyl)-benzoic acid
  MUTAGEN 11: note = X stands for (S)-3-(4-(aminomethyl)phenyl)-2-(methylamino)-propanoic acid
  MUTAGEN 12: note = X stands for (S)-2-amino-nonanoic acid
  MUTAGEN 13: note = X stands for (2S)-2-(methylamino)-propanoic acid
  MUTAGEN 14: note = X stands for (2S)-2-(methylamino)-3-phenyl-propanoic acid
  MUTAGEN 15: note = X stands for D-cysteine
XAXYXIXXXRXXXXX

SEQ ID NO: 360 - protein, 15 aa, synthetic construct
  MUTAGEN 3: note = X stands for (S)-4-(3-(2-amino-2-carboxyethyl)-6-hydroxy-1H-indol-1-yl)-benzoic acid
  MUTAGEN 5: note = X stands for (2S)-2-(methylamino)-3-phenyl-propanoic acid
  MUTAGEN 7: note = X stands for D-proline
  MUTAGEN 8: note = X stands for (S)-2-amino-3-(3-(carboxymethoxy)phenyl)-propanoic acid
  MUTAGEN 9: note = X stands for (S)-4-(2-amino-2-carboxyethyl)-benzoic acid
  MUTAGEN 11: note = X stands for (S)-3-(4-(aminomethyl)phenyl)-2-(methylamino)-propanoic acid
  MUTAGEN 12: note = X stands for (S)-2-amino-nonanoic acid
  MUTAGEN 13: note = X stands for (2S)-2-(methylamino)-propanoic acid
  MUTAGEN 14: note = X stands for (2S)-2-(methylamino)-3-phenyl-propanoic acid
  MUTAGEN 15: note = X stands for D-cysteine
EAXYXIXXXRXXXXX

SEQ ID NO: 361 - protein, 16 aa, synthetic construct
  MUTAGEN 3: note = X stands for (S)-4-(3-(2-amino-2-carboxyethyl)-6-hydroxy-1H-indol-1-yl)-benzoic acid
  MUTAGEN 5: note = X stands for (2S)-2-(methylamino)-3-phenyl-propanoic acid
  MUTAGEN 7: note = X stands for D-proline
  MUTAGEN 8: note = X stands for (S)-2-amino-3-(3-(carboxymethoxy)phenyl)-propanoic acid
  MUTAGEN 9: note = X stands for (S)-4-(2-amino-2-carboxyethyl)-benzoic acid
  MUTAGEN 11: note = X stands for (2S)-2-(methylamino)-3-phenyl-propanoic acid
  MUTAGEN 12: note = X stands for (S)-2-amino-nonanoic acid
  MUTAGEN 13: note = X stands for (2S)-2-(methylamino)-propanoic acid
  MUTAGEN 14: note = X stands for (2S)-2-(methylamino)-3-phenyl-propanoic acid
  MUTAGEN 15: note = X stands for D-cysteine
  MUTAGEN 16: note = X stands for 3-(piperidine-4-yl)-propanoic acid
AAXYXIXXXRXXXXXX

SEQ ID NO: 362 - protein, 15 aa, synthetic construct
  MUTAGEN 3: note = X stands for (S)-2-amino-3-(6-hydroxy-1H-indol-3-yl)-propanoic acid
  MUTAGEN 5: note = X stands for (2S)-2-(methylamino)-3-phenyl-propanoic acid
  MUTAGEN 7: note = X stands for D-proline
  MUTAGEN 8: note = X stands for (S)-2-amino-3-(3-(carboxymethoxy)phenyl)-propanoic acid
  MUTAGEN 9: note = X stands for (S)-4-(2-amino-2-carboxyethyl)-benzoic acid
  MUTAGEN 11: note = X stands for (S)-3-(4-(aminomethyl)phenyl)-2-(methylamino)-propanoic acid
  MUTAGEN 12: note = X stands for (S)-2-aminodo-decanoic acid
  MUTAGEN 13: note = X stands for (2S)-2-(methylamino)-propanoic acid
  MUTAGEN 14: note = X stands for (2S)-2-(methylamino)-3-phenyl-propanoic acid
  MUTAGEN 15: note = X stands for D-cysteine
EAXYXIXXXRXXXXX

SEQ ID NO: 363 - protein, 16 aa, synthetic construct
  MUTAGEN 1: note = X stands for 3-((carboxymethyl)amino)-propanoic acid
  MUTAGEN 3: note = X stands for (S)-4-(3-(2-amino-2-carboxyethyl)-6-hydroxy-1H-indol-1-yl)-benzoic acid
  MUTAGEN 5: note = X stands for (2S)-2-(methylamino)-3-phenyl-propanoic acid
  MUTAGEN 7: note = X stands for D-proline
  MUTAGEN 8: note = X stands for (S)-2-amino-3-(3-(carboxymethoxy)phenyl)-propanoic acid
  MUTAGEN 9: note = X stands for (S)-4-(2-amino-2-carboxyethyl)-benzoic acid
  MUTAGEN 11: note = X stands for (2S)-2-(methylamino)-3-phenyl-propanoic acid
  MUTAGEN 12: note = X stands for (S)-2-amino-nonanoic acid
  MUTAGEN 13: note = X stands for (S)-3-amino-2-(methylamino)-propanoic acid
  MUTAGEN 14: note = X stands for (2S)-2-(methylamino)-3-phenyl-propanoic acid
  MUTAGEN 15: note = X stands for D-cysteine
  MUTAGEN 16: note = X stands for 3-(piperidine-4-yl)-propanoic acid
XAXYXIXXXRXXXXXX

SEQ ID NO: 364 - protein, 16 aa, synthetic construct
  MUTAGEN 1: note = X stands for 4-((carboxymethyl)amino)-butanoic acid
  MUTAGEN 3: note = X stands for (S)-4-(3-(2-amino-2-carboxyethyl)-6-hydroxy-1H-indol-1-yl)-benzoic acid
  MUTAGEN 5: note = X stands for (2S)-2-(methylamino)-3-phenyl-propanoic acid
  MUTAGEN 7: note = X stands for D-proline
  MUTAGEN 8: note = X stands for (S)-2-amino-3-(3-(carboxymethoxy)phenyl)-propanoic acid
  MUTAGEN 9: note = X stands for (S)-4-(2-amino-2-carboxyethyl)-benzoic acid
  MUTAGEN 11: note = X stands for (2S)-2-(methylamino)-3-phenyl-propanoic acid
  MUTAGEN 12: note = X stands for (S)-2-amino-nonanoic acid
  MUTAGEN 13: note = X stands for (2S)-2-(methylamino)-propanoic acid
  MUTAGEN 14: note = X stands for (2S)-2-(methylamino)-3-phenyl-propanoic acid
  MUTAGEN 15: note = X stands for D-glutamic acid
  MUTAGEN 16: note = X stands for (2S)-2-(methylamino)-propanoic acid
XAXYXIXXXRXXXXXX

SEQ ID NO: 365 - protein, 16 aa, synthetic construct
  MUTAGEN 3: note = X stands for (S)-4-(3-(2-amino-2-carboxyethyl)-6-hydroxy-1H-indol-1-yl)-benzoic acid
  MUTAGEN 5: note = X stands for (2S)-2-(methylamino)-3-phenyl-propanoic acid
  MUTAGEN 7: note = X stands for D-proline
  MUTAGEN 8: note = X stands for (S)-2-amino-3-(3-(carboxymethoxy)phenyl)-propanoic acid
  MUTAGEN 9: note = X stands for (S)-4-(2-amino-2-carboxyethyl)-benzoic acid
  MUTAGEN 11: note = X stands for (2S)-2-(methylamino)-3-phenyl-propanoic acid
  MUTAGEN 12: note = X stands for (S)-2-amino-nonanoic acid
  MUTAGEN 13: note = X stands for (2S)-2-(methylamino)-propanoic acid
  MUTAGEN 14: note = X stands for (2S)-2-(methylamino)-3-phenyl-propanoic acid
  MUTAGEN 15: note = X stands for D-glutamic acid
  MUTAGEN 16: note = X stands for (2S)-2-(methylamino)-propanoic acid
AAXYXIXXXRXXXXXX

SEQ ID NO: 366 - protein, 16 aa, synthetic construct
  MUTAGEN 1: note = X stands for (2S)-2-(methylamino)-propanoic acid
  MUTAGEN 3: note = X stands for (S)-4-(3-(2-amino-2-carboxyethyl)-6-hydroxy-1H-indol-1-yl)-benzoic acid
  MUTAGEN 5: note = X stands for (2S)-2-(methylamino)-3-phenyl-propanoic acid
  MUTAGEN 7: note = X stands for D-proline
  MUTAGEN 8: note = X stands for (S)-2-amino-3-(3-(carboxymethoxy)phenyl)-propanoic acid
  MUTAGEN 9: note = X stands for (S)-4-(2-amino-2-carboxyethyl)-benzoic acid
  MUTAGEN 11: note = X stands for (2S)-2-(methylamino)-3-phenyl-propanoic acid
  MUTAGEN 12: note = X stands for (S)-2-amino-nonanoic acid
  MUTAGEN 13: note = X stands for (2S)-2-(methylamino)-propanoic acid
  MUTAGEN 14: note = X stands for (2S)-2-(methylamino)-3-phenyl-propanoic acid
  MUTAGEN 15: note = X stands for D-glutamic acid
  MUTAGEN 16: note = X stands for (2S)-2-(methylamino)-propanoic acid
XAXYXIXXXRXXXXXX

SEQ ID NO: 367 - protein, 16 aa, synthetic construct
  MUTAGEN 1: note = X stands for 4-((carboxymethyl)amino)-butanoic acid
  MUTAGEN 3: note = X stands for (S)-4-(3-(2-amino-2-carboxyethyl)-6-hydroxy-1H-indol-1-yl)-benzoic acid
  MUTAGEN 5: note = X stands for (2S)-2-(methylamino)-3-phenyl-propanoic acid
  MUTAGEN 7: note = X stands for D-proline
  MUTAGEN 8: note = X stands for (S)-2-amino-3-(3-(carboxymethoxy)phenyl)-propanoic acid
  MUTAGEN 9: note = X stands for (S)-4-(2-amino-2-carboxyethyl)-benzoic acid
  MUTAGEN 11: note = X stands for (2S)-2-(methylamino)-3-phenyl-propanoic acid
  MUTAGEN 12: note = X stands for (S)-2-amino-nonanoic acid
  MUTAGEN 13: note = X stands for (2S)-2-(methylamino)-propanoic acid
  MUTAGEN 14: note = X stands for (2S)-2-(methylamino)-3-phenyl-propanoic acid
  MUTAGEN 15: note = X stands for D-cysteine
  MOTIF 16: note = X stands for 3-(piperidine-4-yl)-propanoic acid
XAXYXIXXXRXXXXXX

SEQ ID NO: 368 - protein, 16 aa, synthetic construct
  MUTAGEN 1: note = X stands for 3-((carboxymethyl)amino)-propanoic acid
  MUTAGEN 3: note = X stands for (S)-4-(3-(2-amino-2-carboxyethyl)-6-hydroxy-1H-indol-1-yl)-benzoic acid
  MUTAGEN 5: note = X stands for (2S)-2-(methylamino)-3-phenyl-propanoic acid
  MUTAGEN 7: note = X stands for D-proline
  MUTAGEN 8: note = X stands for (S)-2-amino-3-(3-(carboxymethoxy)phenyl)-propanoic acid
  MUTAGEN 9: note = X stands for (S)-4-(2-amino-2-carboxyethyl)-benzoic acid
  MUTAGEN 11: note = X stands for (2S)-2-(methylamino)-3-phenyl-propanoic acid
  MUTAGEN 12: note = X stands for (S)-2-amino-nonanoic acid
  MUTAGEN 13: note = X stands for (S)-3-amino-2-(methylamino)-propanoic acid
  MUTAGEN 14: note = X stands for (2S)-2-(methylamino)-3-phenyl-propanoic acid
  MUTAGEN 15: note = X stands for D-glutamic acid
  MUTAGEN 16: note = X stands for (2S)-2-(methylamino)-propanoic acid
XAXYXIXXXRXXXXXX